European Patent Application EP 4 166 660 A1, published April 19, 2023. Title: Improved methods for modification of target nucleic acids. Applicant: BASF Plant Science Company GmbH. The sequence listing filed with the application follows.

SEQUENCE LISTING (73 sequences)

SEQ ID NO: 1 - DNA, 4140 bp, synthetic construct
  misc_feature 1..4140: note = Cas9 yeast
  source 1..4140: mol_type = other DNA
atggataaaaaatattctattggtttggatattggtactaattctgttggttgggctgttattactgatgaatataaagttccatctaaaaaatttaaagttttgggtaatactgatagacattctattaaaaaaaatttgattggtgctttgttgtttgattctggtgaaactgctgaagctactagattgaaaagaactgctagaagaagatatactagaagaaaaaatagaatttgttatttgcaagaaattttttctaatgaaatggctaaagttgatgattctttttttcatagattggaagaatcttttttggttgaagaagataaaaaacatgaaagacatccaatttttggtaatattgttgatgaagttgcttatcatgaaaaatatccaactatttatcatttgagaaaaaaattggttgattctactgataaagctgatttgagattgatttatttggctttggctcatatgattaaatttagaggtcattttttgattgaaggtgatttgaatccagataattctgatgttgataaattgtttattcaattggttcaaacttataatcaattgtttgaagaaaatccaattaatgcttctggtgttgatgctaaagctattttgtctgctagattgtctaaatctagaagattggaaaatttgattgctcaattgccaggtgaaaaaaaaaatggtttgtttggtaatttgattgctttgtctttgggtttgactccaaattttaaatctaattttgatttggctgaagatgctaaattgcaattgtctaaagatacttatgatgatgatttggataatttgttggctcaaattggtgatcaatatgctgatttgtttttggctgctaaaaatttgtctgatgctattttgttgtctgatattttgagagttaatactgaaattactaaagctccattgtctgcttctatgattaaaagatatgatgaacatcatcaagatttgactttgttgaaagctttggttagacaacaattgccagaaaaatataaagaaattttttttgatcaatctaaaaatggttatgctggttatattgatggtggtgcttctcaagaagaattttataaatttattaaaccaattttggaaaaaatggatggtactgaagaattgttggttaaattgaatagagaagatttgttgagaaaacaaagaacttttgataatggttctattccacatcaaattcatttgggtgaattgcatgctattttgagaagacaagaagatttttatccatttttgaaagataatagagaaaaaattgaaaaaattttgacttttagaattccatattatgttggtccattggctagaggtaattctagatttgcttggatgactagaaaatctgaagaaactattactccatggaattttgaagaagttgttgataaaggtgcttctgctcaatcttttattgaaagaatgactaattttgataaaaatttgccaaatgaaaaagttttgccaaaacattctttgttgtatgaatattttactgtttataatgaattgactaaagttaaatatgttactgaaggtatgagaaaaccagcttttttgtctggtgaacaaaaaaaagctattgttgatttgttgtttaaaactaatagaaaagttactgttaaacaattgaaagaagattattttaaaaaaattgaatgttttgattctgttgaaatttctggtgttgaagatagatttaatgcttctttgggtacttatcatgatttgttgaaaattattaaagataaagattttttggataatgaagaaaatgaagatattttggaagatattgttttgactttgactttgtttgaagatagagaaatgattgaagaaagattgaaaacttatgctcatttgtttgatgataaagttatgaaacaattgaaaagaagaagatatactggttggggtagattgtctagaaaattgattaatggtattagagataaacaatctggtaaaactattttggattttttgaaatctgatggttttgctaatagaaattttatgcaattgattcatgatgattctttgacttttaaagaagatattcaaaaagctcaagtttctggtcaaggtgattctttgcatgaacatattgctaatttggctggttctccagctattaaaaaaggtattttgcaaactgttaaagttgttgatgaattggttaaagttatgggtagacataaaccagaaaatattgttattgaaatggctagagaaaatcaaactactcaaaaaggtcaaaaaaattctagagaaagaatgaaaagaattgaagaaggtattaaagaattgggttctcaaattttgaaagaacatccagttgaaaatactcaattgcaaaatgaaaaattgtatttgtattatttgcaaaatggtagagatatgtatgttgatcaagaattggatattaatagattgtctgattatgatgttgatcatattgttccacaatcttttttgaaagatgattctattgataataaagttttgactagatctgataaaaatagaggtaaatctgataatgttccatctgaagaagttgttaaaaaaatgaaaaattattggagacaattgttgaatgctaaattgattactcaaagaaaatttgataatttgactaaagctgaaagaggtggtttgtctgaattggataaagctggttttattaaaagacaattggttgaaactagacaaattactaaacatgttgctcaaattttggattctagaatgaatactaaatatgatgaaaatgataaattgattagagaagttaaagttattactttgaaatctaaattggtttctgattttagaaaagattttcaattttataaagttagagaaattaataattatcatcatgctcatgatgcttatttgaatgctgttgttggtactgctttgattaaaaaatatccaaaattggaatctgaatttgtttatggtgattataaagtttatgatgttagaaaaatgattgctaaatctgaacaagaaattggtaaagctactgctaaatattttttttattctaatattatgaatttttttaaaactgaaattactttggctaatggtgaaattagaaaaagaccattgattgaaactaatggtgaaactggtgaaattgtttgggataaaggtagagattttgctactgttagaaaagttttgtctatgccacaagttaatattgttaaaaaaactgaagttcaaactggtggtttttctaaagaatctattttgccaaaaagaaattctgataaattgattgctagaaaaaaagattgggatccaaaaaaatatggtggttttgattctccaactgttgcttattctgttttggttgttgctaaagttgaaaaaggtaaatctaaaaaattgaaatctgttaaagaattgttgggtattactattatggaaagatcttcttttgaaaaaaatccaattgattttttggaagctaaaggttataaagaagttaaaaaagatttgattattaaattgccaaaatattctttgtttgaattggaaaatggtagaaaaagaatgttggcttctgctggtgaattgcaaaaaggtaatgaattggctttgccatctaaatatgttaattttttgtatttggcttctcattatgaaaaattgaaaggttctccagaagataatgaacaaaaacaattgtttgttgaacaacataaacattatttggatgaaattattgaacaaatttctgaattttctaaaagagttattttggctgatgctaatttggataaagttttgtctgcttataataaacatagagataaaccaattagagaacaagctgaaaatattattcatttgtttactttgactaatttgggtgctccagctgcttttaaatattttgatactactattgatagaaaaagatatacttctactaaagaagttttggatgctactttgattcatcaatctattactggtttgtatgaaactagaattgatttgtctcaattgggtggtgattctagagctgatccaaaaaaaaaaagaaaagtttaa

SEQ ID NO: 2 - protein, 1379 aa, synthetic construct
  REGION 1..1379: note = Cas9 yeast protein
MDKKYSIGLDIGTNSVGWAVITDEYKVPSKKFKVLGNTDRHSIKKNLIGALLFDSGETAEATRLKRTARRRYTRRKNRICYLQEIFSNEMAKVDDSFFHRLEESFLVEEDKKHERHPIFGNIVDEVAYHEKYPTIYHLRKKLVDSTDKADLRLIYLALAHMIKFRGHFLIEGDLNPDNSDVDKLFIQLVQTYNQLFEENPINASGVDAKAILSARLSKSRRLENLIAQLPGEKKNGLFGNLIALSLGLTPNFKSNFDLAEDAKLQLSKDTYDDDLDNLLAQIGDQYADLFLAAKNLSDAILLSDILRVNTEITKAPLSASMIKRYDEHHQDLTLLKALVRQQLPEKYKEIFFDQSKNGYAGYIDGGASQEEFYKFIKPILEKMDGTEELLVKLNREDLLRKQRTFDNGSIPHQIHLGELHAILRRQEDFYPFLKDNREKIEKILTFRIPYYVGPLARGNSRFAWMTRKSEETITPWNFEEVVDKGASAQSFIERMTNFDKNLPNEKVLPKHSLLYEYFTVYNELTKVKYVTEGMRKPAFLSGEQKKAIVDLLFKTNRKVTVKQLKEDYFKKIECFDSVEISGVEDRFNASLGTYHDLLKIIKDKDFLDNEENEDILEDIVLTLTLFEDREMIEERLKTYAHLFDDKVMKQLKRRRYTGWGRLSRKLINGIRDKQSGKTILDFLKSDGFANRNFMQLIHDDSLTFKEDIQKAQVSGQGDSLHEHIANLAGSPAIKKGILQTVKVVDELVKVMGRHKPENIVIEMARENQTTQKGQKNSRERMKRIEEGIKELGSQILKEHPVENTQLQNEKLYLYYLQNGRDMYVDQELDINRLSDYDVDHIVPQSFLKDDSIDNKVLTRSDKNRGKSDNVPSEEVVKKMKNYWRQLLNAKLITQRKFDNLTKAERGGLSELDKAGFIKRQLVETRQITKHVAQILDSRMNTKYDENDKLIREVKVITLKSKLVSDFRKDFQFYKVREINNYHHAHDAYLNAVVGTALIKKYPKLESEFVYGDYKVYDVRKMIAKSEQEIGKATAKYFFYSNIMNFFKTEITLANGEIRKRPLIETNGETGEIVWDKGRDFATVRKVLSMPQVNIVKKTEVQTGGFSKESILPKRNSDKLIARKKDWDPKKYGGFDSPTVAYSVLVVAKVEKGKSKKLKSVKELLGITIMERSSFEKNPIDFLEAKGYKEVKKDLIIKLPKYSLFELENGRKRMLASAGELQKGNELALPSKYVNFLYLASHYEKLKGSPEDNEQKQLFVEQHKHYLDEIIEQISEFSKRVILADANLDKVLSAYNKHRDKPIREQAENIIHLFTLTNLGAPAAFKYFDTTIDRKRYTSTKEVLDATLIHQSITGLYETRIDLSQLGGDSRADPKKKRKV

SEQ ID NO: 3 - DNA, 4140 bp, synthetic construct
  misc_feature 1..4140: note = Cas9 D10A H840A inactive
  source 1..4140: mol_type = other DNA
atggataaaaaatattctattggtttggctattggtactaattctgttggttgggctgttattactgatgaatataaagttccatctaaaaaatttaaagttttgggtaatactgatagacattctattaaaaaaaatttgattggtgctttgttgtttgattctggtgaaactgctgaagctactagattgaaaagaactgctagaagaagatatactagaagaaaaaatagaatttgttatttgcaagaaattttttctaatgaaatggctaaagttgatgattctttttttcatagattggaagaatcttttttggttgaagaagataaaaaacatgaaagacatccaatttttggtaatattgttgatgaagttgcttatcatgaaaaatatccaactatttatcatttgagaaaaaaattggttgattctactgataaagctgatttgagattgatttatttggctttggctcatatgattaaatttagaggtcattttttgattgaaggtgatttgaatccagataattctgatgttgataaattgtttattcaattggttcaaacttataatcaattgtttgaagaaaatccaattaatgcttctggtgttgatgctaaagctattttgtctgctagattgtctaaatctagaagattggaaaatttgattgctcaattgccaggtgaaaaaaaaaatggtttgtttggtaatttgattgctttgtctttgggtttgactccaaattttaaatctaattttgatttggctgaagatgctaaattgcaattgtctaaagatacttatgatgatgatttggataatttgttggctcaaattggtgatcaatatgctgatttgtttttggctgctaaaaatttgtctgatgctattttgttgtctgatattttgagagttaatactgaaattactaaagctccattgtctgcttctatgattaaaagatatgatgaacatcatcaagatttgactttgttgaaagctttggttagacaacaattgccagaaaaatataaagaaattttttttgatcaatctaaaaatggttatgctggttatattgatggtggtgcttctcaagaagaattttataaatttattaaaccaattttggaaaaaatggatggtactgaagaattgttggttaaattgaatagagaagatttgttgagaaaacaaagaacttttgataatggttctattccacatcaaattcatttgggtgaattgcatgctattttgagaagacaagaagatttttatccatttttgaaagataatagagaaaaaattgaaaaaattttgacttttagaattccatattatgttggtccattggctagaggtaattctagatttgcttggatgactagaaaatctgaagaaactattactccatggaattttgaagaagttgttgataaaggtgcttctgctcaatcttttattgaaagaatgactaattttgataaaaatttgccaaatgaaaaagttttgccaaaacattctttgttgtatgaatattttactgtttataatgaattgactaaagttaaatatgttactgaaggtatgagaaaaccagcttttttgtctggtgaacaaaaaaaagctattgttgatttgttgtttaaaactaatagaaaagttactgttaaacaattgaaagaagattattttaaaaaaattgaatgttttgattctgttgaaatttctggtgttgaagatagatttaatgcttctttgggtacttatcatgatttgttgaaaattattaaagataaagattttttggataatgaagaaaatgaagatattttggaagatattgttttgactttgactttgtttgaagatagagaaatgattgaagaaagattgaaaacttatgctcatttgtttgatgataaagttatgaaacaattgaaaagaagaagatatactggttggggtagattgtctagaaaattgattaatggtattagagataaacaatctggtaaaactattttggattttttgaaatctgatggttttgctaatagaaattttatgcaattgattcatgatgattctttgacttttaaagaagatattcaaaaagctcaagtttctggtcaaggtgattctttgcatgaacatattgctaatttggctggttctccagctattaaaaaaggtattttgcaaactgttaaagttgttgatgaattggttaaagttatgggtagacataaaccagaaaatattgttattgaaatggctagagaaaatcaaactactcaaaaaggtcaaaaaaattctagagaaagaatgaaaagaattgaagaaggtattaaagaattgggttctcaaattttgaaagaacatccagttgaaaatactcaattgcaaaatgaaaaattgtatttgtattatttgcaaaatggtagagatatgtatgttgatcaagaattggatattaatagattgtctgattatgatgttgatgctattgttccacaatcttttttgaaagatgattctattgataataaagttttgactagatctgataaaaatagaggtaaatctgataatgttccatctgaagaagttgttaaaaaaatgaaaaattattggagacaattgttgaatgctaaattgattactcaaagaaaatttgataatttgactaaagctgaaagaggtggtttgtctgaattggataaagctggttttattaaaagacaattggttgaaactagacaaattactaaacatgttgctcaaattttggattctagaatgaatactaaatatgatgaaaatgataaattgattagagaagttaaagttattactttgaaatctaaattggtttctgattttagaaaagattttcaattttataaagttagagaaattaataattatcatcatgctcatgatgcttatttgaatgctgttgttggtactgctttgattaaaaaatatccaaaattggaatctgaatttgtttatggtgattataaagtttatgatgttagaaaaatgattgctaaatctgaacaagaaattggtaaagctactgctaaatattttttttattctaatattatgaatttttttaaaactgaaattactttggctaatggtgaaattagaaaaagaccattgattgaaactaatggtgaaactggtgaaattgtttgggataaaggtagagattttgctactgttagaaaagttttgtctatgccacaagttaatattgttaaaaaaactgaagttcaaactggtggtttttctaaagaatctattttgccaaaaagaaattctgataaattgattgctagaaaaaaagattgggatccaaaaaaatatggtggttttgattctccaactgttgcttattctgttttggttgttgctaaagttgaaaaaggtaaatctaaaaaattgaaatctgttaaagaattgttgggtattactattatggaaagatcttcttttgaaaaaaatccaattgattttttggaagctaaaggttataaagaagttaaaaaagatttgattattaaattgccaaaatattctttgtttgaattggaaaatggtagaaaaagaatgttggcttctgctggtgaattgcaaaaaggtaatgaattggctttgccatctaaatatgttaattttttgtatttggcttctcattatgaaaaattgaaaggttctccagaagataatgaacaaaaacaattgtttgttgaacaacataaacattatttggatgaaattattgaacaaatttctgaattttctaaaagagttattttggctgatgctaatttggataaagttttgtctgcttataataaacatagagataaaccaattagagaacaagctgaaaatattattcatttgtttactttgactaatttgggtgctccagctgcttttaaatattttgatactactattgatagaaaaagatatacttctactaaagaagttttggatgctactttgattcatcaatctattactggtttgtatgaaactagaattgatttgtctcaattgggtggtgattctagagctgatccaaaaaaaaaaagaaaagtttaa

SEQ ID NO: 4 - protein, 1379 aa, synthetic construct
  REGION 1..1379: note = Cas9 D10A H840A inactive protein
MDKKYSIGLAIGTNSVGWAVITDEYKVPSKKFKVLGNTDRHSIKKNLIGALLFDSGETAEATRLKRTARRRYTRRKNRICYLQEIFSNEMAKVDDSFFHRLEESFLVEEDKKHERHPIFGNIVDEVAYHEKYPTIYHLRKKLVDSTDKADLRLIYLALAHMIKFRGHFLIEGDLNPDNSDVDKLFIQLVQTYNQLFEENPINASGVDAKAILSARLSKSRRLENLIAQLPGEKKNGLFGNLIALSLGLTPNFKSNFDLAEDAKLQLSKDTYDDDLDNLLAQIGDQYADLFLAAKNLSDAILLSDILRVNTEITKAPLSASMIKRYDEHHQDLTLLKALVRQQLPEKYKEIFFDQSKNGYAGYIDGGASQEEFYKFIKPILEKMDGTEELLVKLNREDLLRKQRTFDNGSIPHQIHLGELHAILRRQEDFYPFLKDNREKIEKILTFRIPYYVGPLARGNSRFAWMTRKSEETITPWNFEEVVDKGASAQSFIERMTNFDKNLPNEKVLPKHSLLYEYFTVYNELTKVKYVTEGMRKPAFLSGEQKKAIVDLLFKTNRKVTVKQLKEDYFKKIECFDSVEISGVEDRFNASLGTYHDLLKIIKDKDFLDNEENEDILEDIVLTLTLFEDREMIEERLKTYAHLFDDKVMKQLKRRRYTGWGRLSRKLINGIRDKQSGKTILDFLKSDGFANRNFMQLIHDDSLTFKEDIQKAQVSGQGDSLHEHIANLAGSPAIKKGILQTVKVVDELVKVMGRHKPENIVIEMARENQTTQKGQKNSRERMKRIEEGIKELGSQILKEHPVENTQLQNEKLYLYYLQNGRDMYVDQELDINRLSDYDVDAIVPQSFLKDDSIDNKVLTRSDKNRGKSDNVPSEEVVKKMKNYWRQLLNAKLITQRKFDNLTKAERGGLSELDKAGFIKRQLVETRQITKHVAQILDSRMNTKYDENDKLIREVKVITLKSKLVSDFRKDFQFYKVREINNYHHAHDAYLNAVVGTALIKKYPKLESEFVYGDYKVYDVRKMIAKSEQEIGKATAKYFFYSNIMNFFKTEITLANGEIRKRPLIETNGETGEIVWDKGRDFATVRKVLSMPQVNIVKKTEVQTGGFSKESILPKRNSDKLIARKKDWDPKKYGGFDSPTVAYSVLVVAKVEKGKSKKLKSVKELLGITIMERSSFEKNPIDFLEAKGYKEVKKDLIIKLPKYSLFELENGRKRMLASAGELQKGNELALPSKYVNFLYLASHYEKLKGSPEDNEQKQLFVEQHKHYLDEIIEQISEFSKRVILADANLDKVLSAYNKHRDKPIREQAENIIHLFTLTNLGAPAAFKYFDTTIDRKRYTSTKEVLDATLIHQSITGLYETRIDLSQLGGDSRADPKKKRKV

SEQ ID NO: 5 - DNA, 4155 bp, synthetic construct
  misc_feature 1..4155: note = Cas9 rice
  source 1..4155: mol_type = other DNA
atggacaagaagtatagtattggtctggacattgggacgaattccgttggctgggccgtgatcaccgatgagtacaaggtcccttccaagaagtttaaggttctggggaacaccgatcggcacagcatcaagaagaatctcattggagccctcctgttcgactcaggcgagaccgccgaagcaacaaggctcaagagaaccgcaaggagacggtatacaagaaggaagaataggatctgctacctgcaggagattttcagcaacgaaatggcgaaggtggacgattcgttctttcatagattggaggagagtttcctcgtcgaggaagataagaagcacgagaggcatcctatctttggcaacattgtcgacgaggttgcctatcacgaaaagtaccccacaatctatcatctgcggaagaagcttgtggactcgactgataaggcggaccttagattgatctacctcgctctggcacacatgattaagttcaggggccattttctgatcgagggggatcttaacccggacaatagcgatgtggacaagttgttcatccagctcgtccaaacctacaatcagctctttgaggaaaacccaattaatgcttcaggcgtcgacgccaaggcgatcctgtctgcacgcctttcaaagtctcgccggcttgagaacttgatcgctcaactcccgggcgaaaagaagaacggcttgttcgggaatctcattgcactttcgttggggctcacaccaaacttcaagagtaattttgatctcgctgaggacgcaaagctgcagctttccaaggacacttatgacgatgacctggataaccttttggcccaaatcggcgatcagtacgcggacttgttcctcgccgcgaagaatttgtcggacgcgatcctcctgagtgatattctccgcgtgaacaccgagattacaaaggccccgctctcggcgagtatgatcaagcgctatgacgagcaccatcaggatctgacccttttgaaggctttggtccggcagcaactcccagagaagtacaaggaaatcttctttgatcaatccaagaacggctacgctggttatattgacggcggggcatcgcaggaggaattctacaagtttatcaagccaattctggagaagatggatggcacagaggaactcctggtgaagctcaatagggaggaccttttgcggaagcaaagaactttcgataacggcagcatccctcaccagattcatctcggggagctgcacgccatcctgagaaggcaggaagacttctacccctttcttaaggataaccgggagaagatcgaaaagattctgacgttcagaattccgtactatgtcggaccactcgcccggggtaattccagatttgcgtggatgaccagaaagagcgaggaaaccatcacaccttggaacttcgaggaagtggtcgataagggcgcttccgcacagagcttcattgagcgcatgacaaattttgacaagaacctgcctaatgagaaggtccttcccaagcattccctcctgtacgagtatttcactgtttataacgaactcacgaaggtgaagtatgtgaccgagggaatgcgcaagcccgccttcctgagcggcgagcaaaagaaggcgatcgtggaccttttgtttaagaccaatcggaaggtcacagttaagcagctcaaggaggactacttcaagaagattgaatgcttcgattccgttgagatcagcggcgtggaagacaggtttaacgcgtcactggggacttaccacgatctcctgaagatcattaaggataaggacttcttggacaacgaggaaaatgaggatatcctcgaagacattgtcctgactcttacgttgtttgaggatagggaaatgatcgaggaacgcttgaagacgtatgcccatctcttcgatgacaaggttatgaagcagctcaagagaagaagatacaccggatggggaaggctgtcccgcaagcttatcaatggcattagagacaagcaatcagggaagacaatccttgactttttgaagtctgatggcttcgcgaacaggaattttatgcagctgattcacgatgactcacttactttcaaggaggatatccagaaggctcaagtgtcgggacaaggtgacagtctgcacgagcatatcgccaaccttgcgggatctcctgcaatcaagaagggtattctgcagacagtcaaggttgtggatgagcttgtgaaggtcatgggacggcataagcccgagaacatcgttattgagatggccagagaaaatcagaccacacaaaagggtcagaagaactcgagggagcgcatgaagcgcatcgaggaaggcattaaggagctggggagtcagatccttaaggagcacccggtggaaaacacgcagttgcaaaatgagaagctctatctgtactatctgcaaaatggcagggatatgtatgtggaccaggagttggatattaaccgcctctcggattacgacgtcgatcatatcgttcctcagtccttccttaaggatgacagcattgacaataaggttctcaccaggtccgacaagaaccgcgggaagtccgataatgtgcccagcgaggaagtcgttaagaagatgaagaactactggaggcaacttttgaatgccaagttgatcacacagaggaagtttgataacctcactaaggccgagcgcggaggtctcagcgaactggacaaggcgggcttcattaagcggcaactggttgagactagacagatcacgaagcacgtggcgcagattctcgattcacgcatgaacacgaagtacgatgagaatgacaagctgatccgggaagtgaaggtcatcaccttgaagtcaaagctcgtttctgacttcaggaaggatttccaattttataaggtgcgcgagatcaacaattatcaccatgctcatgacgcatacctcaacgctgtggtcggaacagcattgattaagaagtacccgaagctcgagtccgaattcgtgtacggtgactataaggtttacgatgtgcgcaagatgatcgccaagtcagagcaggaaattggcaaggccactgcgaagtatttcttttactctaacattatgaatttctttaagactgagatcacgctggctaatggcgaaatccggaagagaccacttattgagaccaacggcgagacaggggaaatcgtgtgggacaaggggagggatttcgccacagtccgcaaggttctctctatgcctcaagtgaatattgtcaagaagactgaagtccagacgggcgggttctcaaaggaatctattctgcccaagcggaactcggataagcttatcgccagaaagaaggactgggacccgaagaagtatggaggtttcgactcaccaacggtggcttactctgtcctggttgtggcaaaggtggagaagggaaagtcaaagaagctcaagtctgtcaaggagctcctgggtatcaccattatggagaggtccagcttcgaaaagaatccgatcgattttctcgaggcgaagggatataaggaagtgaagaaggacctgatcattaagcttccaaagtacagtcttttcgagttggaaaacggcaggaagcgcatgttggcttccgcaggagagctccagaagggtaacgagcttgctttgccgtccaagtatgtgaacttcctctatctggcatcccactacgagaagctcaagggcagcccagaggataacgaacagaagcaactgtttgtggagcaacacaagcattatcttgacgagatcattgaacagatttcggagttcagtaagcgcgtcatcctcgccgacgcgaatttggataaggttctctcagcctacaacaagcaccgggacaagcctatcagagagcaggcggaaaatatcattcatctcttcaccctgacaaaccttggggctcccgctgcattcaagtattttgacactacgattgatcggaagagatacacttctacgaaggaggtgctggatgcaacccttatccaccaatcgattactggcctctacgagacgcggatcgacttgagtcagctcgggggggataagagaccagcggcaaccaagaaggcaggacaagcgaagaagaagaagtag

SEQ ID NO: 6 - DNA, 24 bp, synthetic construct
  misc_feature 1..24: note = SV40 Nuclear Localizaion Signal
  source 1..24: mol_type = other DNA
cccaagaagaagcggaaggtctcg

SEQ ID NO: 7 - DNA, 957 bp, synthetic construct
  misc_feature 1..957: note = GAL4
  source 1..957: mol_type = other DNA
atgaagctactgtcttctatcgaacaagcatgcgatatttgccgacttaaaaagctcaagtgctccaaagaaaaaccgaagtgcgccaagtgtctgaagaacaactgggagtgtcgctactctcccaaaaccaaaaggtctccgctgactagggcacatctgacagaagtggaatcaaggctagaaagactggaacagctatttctactgatttttcctcgagaagaccttgacatgattttgaaaatggattctttacaggatataaaagcattgttaacaggattatttgtacaagataatgtgaataaagatgccgtcacagatagattggcttcagtggagactgatatgcctctaacattgagacagcatagaataagtgcgacatcatcatcggaagagagtagtaacaaaggtcaaagacagttgactgtatcgccggaatttgtaatacgactcactatagggcgagccgccatcatggaggagcagaagctgatctcagaggaggacctgcatatggccatggaggccgaattcatggataaagcggaattaattcccgagcctccaaaaaagaagagaaaggtcgaattgggtaccgccgccaattttaatcaaagtgggaatattgctgatagctcattgtccttcactttcactaacagtagcaacggtccgaacctcataacaactcaaacaaattctcaagcgctttcacaaccaattgcctcctctaacgttcatgataacttcatgaataatgaaatcacggctagtaaaattgatgatggtaataattcaaaaccactgtcacctggttggacggaccaaactgcgtataacgcgtttggaatcactacagggatgtttaataccactacaatggatgatgtatataactatctattcgatgatgaagataccccaccaaacccaaaaaaagagatttaa

SEQ ID NO: 8 - protein, 318 aa, synthetic construct
  REGION 1..318: note = GAL4 protein
MKLLSSIEQACDICRLKKLKCSKEKPKCAKCLKNNWECRYSPKTKRSPLTRAHLTEVESRLERLEQLFLLIFPREDLDMILKMDSLQDIKALLTGLFVQDNVNKDAVTDRLASVETDMPLTLRQHRISATSSSEESSNKGQRQLTVSPEFVIRLTIGRAAIMEEQKLISEEDLHMAMEAEFMDKAELIPEPPKKKRKVELGTAANFNQSGNIADSSLSFTFTNSSNGPNLITTQTNSQALSQPIASSNVHDNFMNNEITASKIDDGNNSKPLSPGWTDQTAYNAFGITTGMFNTTTMDDVYNYLFDDEDTPPNPKKEI

SEQ ID NO: 9 - DNA, 958 bp, synthetic construct
  misc_feature 1..958: note = GAL4 target 1
  source 1..958: mol_type = other DNA
atgaagctactgtcttctatcgaacaagcatgcgatatttgccgacttaaaaagctcaagtgctccaaagaaaaaccgaagtgcgccaagtgtctgaagaactaactgggagtgtcgctactctcccaaaaccaaaaggtctccgctgactagggcacatctgacagaagtggaatcaaggctagaaagactggaacagctatttctactgatttttcctcgagaagaccttgacatgattttgaaaatggattctttacaggatataaaagcattgttaacaggattatttgtacaagataatgtgaataaagatgccgtcacagatagattggcttcagtggagactgatatgcctctaacattgagacagcatagaataagtgcgacatcatcatcggaagagagtagtaacaaaggtcaaagacagttgactgtatcgccggaatttgtaatacgactcactatagggcgagccgccatcatggaggagcagaagctgatctcagaggaggacctgcatatggccatggaggccgaattcatggataaagcggaattaattcccgagcctccaaaaaagaagagaaaggtcgaattgggtaccgccgccaattttaatcaaagtgggaatattgctgatagctcattgtccttcactttcactaacagtagcaacggtccgaacctcataacaactcaaacaaattctcaagcgctttcacaaccaattgcctcctctaacgttcatgataacttcatgaataatgaaatcacggctagtaaaattgatgatggtaataattcaaaaccactgtcacctggttggacggaccaaactgcgtataacgcgtttggaatcactacagggatgtttaataccactacaatggatgatgtatataactatctattcgatgatgaagataccccaccaaacccaaaaaaagagatttaa

SEQ ID NO: 10 - DNA, 938 bp, synthetic construct
  misc_feature 1..938: note = GAL4 target 2
  source 1..938: mol_type = other DNA
atgaagctactgtcttctatcgaacaagcatgcgatatttgccgacttaaaaagctcaagtgctccaaagaaaaaccgaagtgcgccaagtgtctgaagaactaactggaaccaaaaggtctccgctgactagggcacatctgacagaagtggaatcaaggctagaaagactggaacagctatttctactgatttttcctcgagaagaccttgacatgattttgaaaatggattctttacaggatataaaagcattgttaacaggattatttgtacaagataatgtgaataaagatgccgtcacagatagattggcttcagtggagactgatatgcctctaacattgagacagcatagaataagtgcgacatcatcatcggaagagagtagtaacaaaggtcaaagacagttgactgtatcgccggaatttgtaatacgactcactatagggcgagccgccatcatggaggagcagaagctgatctcagaggaggacctgcatatggccatggaggccgaattcatggataaagcggaattaattcccgagcctccaaaaaagaagagaaaggtcgaattgggtaccgccgccaattttaatcaaagtgggaatattgctgatagctcattgtccttcactttcactaacagtagcaacggtccgaacctcataacaactcaaacaaattctcaagcgctttcacaaccaattgcctcctctaacgttcatgataacttcatgaataatgaaatcacggctagtaaaattgatgatggtaataattcaaaaccactgtcacctggttggacggaccaaactgcgtataacgcgtttggaatcactacagggatgtttaataccactacaatggatgatgtatataactatctattcgatgatgaagataccccaccaaacccaaaaaaagagatttaa

SEQ ID NO: 11 - DNA, 920 bp, synthetic construct
  misc_feature 1..920: note = GAL4 target 3
  source 1..920: mol_type = other DNA
atgaagctactgtcttctatcgaacaagcatgcgatatttgccgacttaaaaagctcaagtgctccaaagaaaacaagtgtctgaagaactaactggaaggtctccgctgactagggcacatctgacagaagtggaatcaaggctagaaagactggaacagctatttctactgatttttcctcgagaagaccttgacatgattttgaaaatggattctttacaggatataaaagcattgttaacaggattatttgtacaagataatgtgaataaagatgccgtcacagatagattggcttcagtggagactgatatgcctctaacattgagacagcatagaataagtgcgacatcatcatcggaagagagtagtaacaaaggtcaaagacagttgactgtatcgccggaatttgtaatacgactcactatagggcgagccgccatcatggaggagcagaagctgatctcagaggaggacctgcatatggccatggaggccgaattcatggataaagcggaattaattcccgagcctccaaaaaagaagagaaaggtcgaattgggtaccgccgccaattttaatcaaagtgggaatattgctgatagctcattgtccttcactttcactaacagtagcaacggtccgaacctcataacaactcaaacaaattctcaagcgctttcacaaccaattgcctcctctaacgttcatgataacttcatgaataatgaaatcacggctagtaaaattgatgatggtaataattcaaaaccactgtcacctggttggacggaccaaactgcgtataacgcgtttggaatcactacagggatgtttaataccactacaatggatgatgtatataactatctattcgatgatgaagataccccaccaaacccaaaaaaagagatttaa

SEQ ID NO: 12 - DNA, 560 bp, synthetic construct
  misc_feature 1..560: note = GAL4 target 4
  source 1..560: mol_type = other DNA
atgaagctactgtcttctatcgaacaagcatgcgatatttgccgacttaaaaagctcaagtgctccaaagaaaaaccgaagtgcgccaagtgtctgaagaacaactgggagtgtcgctactctcccaaaaccaaaaggtctccgctgactagggcacatctgacagaagtggaatcaaggctagaaagactggaacagctatttctactgatttttcctcgagaagaccttgacatgattttgaaaatggattctttacaggatataaaagcattgttaacaggattatttgtacaagataatgtgaataaagatgccgtcacagatagattggcttcagtggagactgatatgcctctaacattgagacagcatagaataagtgcgacatcatcatcggaagagagtagtaacaaaggtcaaagacagttgactgtataacgccggaacgcgtttggaatcacttaacagggatgtttaataccactacaatggatgatgtatataactatctattcgatgatgaagataccccaccaaacccaaaaaaagagatttaa

SEQ ID NO: 13 - DNA, 708 bp, synthetic construct
  misc_feature 1..708: note = GAL4 target 5
  source 1..708: mol_type = other DNA
atgaagctactgtcttctatcgaacaagcatgcgatatttgccgacttaaaaagctcaagtgctccaaagaaaaaccgaagtgcgccaagtgtctgaagaacaactgggagtgtcgctactctcccaaaaccaaaaggtctccgctgactagggcacatctgacagaagtggaatcaaggctagaaagactggaacagctatttctactgatttttcctcgagaagaccttgacatgattttgaaaatggattctttacaggatataaaagcattgttaacaggattatttgtacaagataatgtgaataaagatgccgtcacagatagattggcttcagtggagactgatatgcctctaacattgagacagcatagaataagtgcgacatcatcatcggaagagagtagtaacaaaggtcaaagacagttgactgtatcgccggaatttgtaatacgactcactatagggcgagccgccatcatggaggagcagaagctgatctcagaggaggacctgcatatggccatggaggccgaattcatgtgataaagcggaattaattccccacctggttggacggaccaaactgcgtataacgcgtttggaatcactacagggatgtttaataccactacaatggatgatgtatataactatctattcgatgatgaagataccccaccaaacccaaaaaaagagatttaa

SEQ ID NO: 14 - DNA, 240 bp, synthetic construct
  misc_feature 1..240: note = GAL4 target 6
  source 1..240: mol_type = other DNA
atgaagctactgtcttctatcgaacaagcatgcgatatttgccgacttaaaaagctcaagtgctccaaagaaaaaccgaagtgcgccaagtgtctgaagaactaactggactgcgtccaaactgcgtataacgcgtttggaatcactacagggatgtttaataccactacaatggatgatgtatataactatctattcgatgatgaagataccccaccaaacccaaaaaaagagatttaa

SEQ ID NO: 15 - DNA, 356 bp, synthetic construct
  misc_feature 1..356: note = GAL4 target 7
  source 1..356: mol_type = other DNA
atgaagctactgtcttctatcgaacaagcatgcgatatttgccgacttaaaaagctcaagtgctccaaagaaaaaccgaagtgcgccaagtgtctgaagaacaactgggagtgtcgctactctcccaaaaccaaaaggtctccgctgactagggcacatctgacagaagtggaatcaaggctagaaagactggaacagctatttctactgatttttcctcgagaagaccttgactgattttgtataacgcgtttggaatcactacagggatgtttaataccactacaatggatgatgtatataactatctattcgatgatgaagataccccaccaaacccaaaaaaagagatttaa

SEQ ID NO: 16 - DNA, 268 bp, Saccharomyces cerevisiae
  misc_feature 1..268: note = SNR52 promoter
  source 1..268: mol_type = genomic DNA
ctttgaaaagataatgtatgattatgctttcactcatatttatacagaaacttgatgttttctttcgagtatatacaaggtgattacatgtacgtttgaagtacaactctagattttgtagtgccctcttgggctagcggtaaaggtgcgcattttttcacaccctacaatgttctgttcaaaagattttggtcaaacgctgtagaagtgaaagttggtgcgcatgtttcggcgttcgaaacttctccgcagtgaaagataaatgatc

SEQ ID NO: 17 - DNA, 20 bp, Saccharomyces cerevisiae
  misc_feature 1..20: note = SUP4 terminator
  source 1..20: mol_type = genomic DNA
tttttttgttttttatgtct

SEQ ID NO: 18 - DNA, 75 bp, synthetic construct
  misc_feature 1..75: note = scaffold guide RNA Cas9
  source 1..75: mol_type = other DNA
ttttagagctagaaatagcaagttaaaataaggctagtccgttatcaacttgaaaaagtggcaccgagtcggtgc

SEQ ID NO: 19 - DNA, 20 bp, synthetic construct
  misc_feature 1..20: note = spacer 1
  source 1..20: mol_type = other DNA
caagtgtctgaagaactaac

SEQ ID NO: 20 - DNA, 20 bp, synthetic construct
  misc_feature 1..20: note = spacer 2
  source 1..20: mol_type = other DNA
gacagttgactgtataacgc

SEQ ID NO: 21 - DNA, 20 bp, synthetic construct
  misc_feature 1..20: note = spacer 3
  source 1..20: mol_type = other DNA
gcgtttggaatcacttaaca

SEQ ID NO: 22 - DNA, 20 bp, synthetic construct
  misc_feature 1..20: note = spacer 4
  source 1..20: mol_type = other DNA
gcatatggccatggaggccg

SEQ ID NO: 23 - DNA, 20 bp, synthetic construct
  misc_feature 1..20: note = spacer 5
  source 1..20: mol_type = other DNA
acgcgtttggaatcactaca

SEQ ID NO: 24 - DNA, 20 bp, synthetic construct
  misc_feature 1..20: note = spacer 6
  source 1..20: mol_type = other DNA
atggtctcaaaacccttggt

SEQ ID NO: 25 - DNA, 20 bp, synthetic construct
  misc_feature 1..20: note = spacer 7
  source 1..20: mol_type = other DNA
acacgcttactgcctgacta

SEQ ID NO: 26 - DNA, 44 bp, synthetic construct
  misc_feature 1..44: note = donor 1
  source 1..44: mol_type = other DNA
cctcgagaagaccttgacatgattttgaaaatggattctttaca

SEQ ID NO: 27 - DNA, 108 bp, synthetic construct
  misc_feature 1..108: note = donor 2
  source 1..108: mol_type = other DNA
aaagactggaacagctatttctactgatttttcctcgagaagaccttgacatgattttgaaaatggattctttacaggatataaaagcattgttaacaggattatttg

SEQ ID NO: 28 - DNA, 520 bp, synthetic construct
  misc_feature 1..520: note = donor 3
  source 1..520: mol_type = other DNA
tcatcatcggaagagagtagtaacaaaggtcaaagacagttgactgtatcgccggaatttgtaatacgactcactatagggcgagccgccatcatggaggagcagaagctgatctcagaggaggacctgcatatggccatggaggccgaattcatggataaagcggaattaattcccgagcctccaaaaaagaagagaaaggtcgaattgggtaccgccgccaattttaatcaaagtgggaatattgctgatagctcattgtccttcactttcactaacagtagcaacggtccgaacctcataacaactcaaacaaattctcaagcgctttcacaaccaattgcctcctctaacgttcatgataacttcatgaataatgaaatcacggctagtaaaattgatgatggtaataattcaaaaccactgtcacctggttggacggaccaaactgcgtataacgcgtttggaatcactacagggatgtttaataccactacaatggatgatgtatataactatc

SEQ ID NO: 29 - DNA, 635 bp, synthetic construct
  misc_feature 1..635: note = donor 4
  source 1..635: mol_type = other DNA
cagatagattggcttcagtggagactgatatgcctctaacattgagacagcatagaataagtgcgacatcatcatcggaagagagtagtaacaaaggtcaaagacagttgactgtatcgccggaatttgtaatacgactcactatagggcgagccgccatcatggaggagcagaagctgatctcagaggaggacctgcatatggccatggaggccgaattcatggataaagcggaattaattcccgagcctccaaaaaagaagagaaaggtcgaattgggtaccgccgccaattttaatcaaagtgggaatattgctgatagctcattgtccttcactttcactaacagtagcaacggtccgaacctcataacaactcaaacaaattctcaagcgctttcacaaccaattgcctcctctaacgttcatgataacttcatgaataatgaaatcacggctagtaaaattgatgatggtaataattcaaaaccactgtcacctggttggacggaccaaactgcgtataacgcgtttggaatcactacagggatgtttaataccactacaatggatgatgtatataactatctattcgatgatgaagataccccaccaaacccaaaaaaagagatttaa

SEQ ID NO: 30 - DNA, 957 bp, synthetic construct; identical to SEQ ID NO: 7
  misc_feature 1..957: note = donor 5
  source 1..957: mol_type = other DNA

SEQ ID NO: 31 - DNA, 4155 bp, synthetic construct; identical to SEQ ID NO: 5
  misc_feature 1..4155: note = Cas9 rice codon-optimized
  source 1..4155: mol_type = other DNA

SEQ ID NO: 32 - DNA, 1995 bp, Zea mays
  misc_feature 1..1995: note = maize Ubi promoter containing MubG1 intron
  source 1..1995: mol_type = genomic DNA
tgcagtgcagcgtgacccggtcgtgcccctctctagagataatgagcattgcatgtctaagttataaaaaattaccacatattttttttgtcacacttgtttgaagtgcagtttatctatctttatacatatatttaaactttactctacgaataatataatctatagtactacaataatatcagtgttttagagaatcatataaatgaacagttagacatggtctaaaggacaattgagtattttgacaacaggactctacagttttatctttttagtgtgcatgtgttctcctttttttttgcaaatagcttcacctatataatacttcatccattttattagtacatccatttagggtttagggttaatggtttttatagactaatttttttagtacatctattttattctattttagcctctaaattaagaaaactaaaactctattttagtttttttatttaatagtttagatataaaatagaataaaataaagtgactaaaaattaaacaaataccctttaagaaattaaaaaaactaaggaaacatttttcttgtttcgagtagataatgccagcctgttaaacgccgtcgacgagtctaacggacaccaaccagcgaaccagcagcgtcgcgtcgggccaagcgaagcagacggcacggcatctctgtcgctgcctctggacccctctcgagagttccgctccaccgttggacttgctccgctgtcggcatccagaaattgcgtggcggagcggcagacgtgagccggcacggcaggcggcctcctcctcctctcacggcaccggcagctacgggggattcctttcccaccgctccttcgctttcccttcctcgcccgccgtaataaatagacaccccctccacaccctctttccccaacctcgtgttgttcggagcgcacacacacacaaccagatctcccccaaatccacccgtcggcacctccgcttcaaggtacgccgctcgtcctcccccccccccccccctctctaccttctctagatcggcgttccggtccatggttagggcccggtagttctacttctgttcatgtttgtgttagatccgtgtttgtgttagatccgtgctgctagcgttcgtacacggatgcgacctgtacgtcagacacgttctgattgctaacttgccagtgtttctctttggggaatcctgggatggctctagccgttccgcagacgggatcgatttcatgattttttttgtttcgttgcatagggtttggtttgcccttttcctttatttcaatatatgccgtgcacttgtttgtcgggtcatcttttcatgcttttttttgtcttggttgtgatgatgtggtctggttgggcggtcgttctagatcggagtagaattctgtttcaaactacctggtggatttattaattttggatctgtatgtgtgtgccatacatattcatagttacgaattgaagatgatggatggaaatatcgatctaggataggtatacatgttgatgcgggttttactgatgcatatacagagatgctttttgttcgcttggttgtgatgatgtggtgtggttgggcggtcgttcattcgttctagatcggagtagagtactgtttcaaactacctggtgtatttattaattttggaactgtatgtgtgtgtcatacatcttcatagttacgagtttaagatggatggaaatatcgatctaggataggtatacatgttgatgtgggttttactgatgcatatacatgatggcatatgcagcatctattcatatgctctaaccttgagtacctatctattataataaacaagtatgttttataattatttcgatcttgatatacttggatgatggcatatgcagcagctatatgtggatttttttagccctgccttcatacgctatttatttgcttggtactgtttcttttgtcgatgctcaccctgttgtttggtgttacttctgcag

SEQ ID NO: 33 - DNA, 294 bp, Agrobacterium tumefaciens
  misc_feature 1..294: note = nopaline synthase terminator (tnos)
  source 1..294: mol_type = genomic DNA
agcggccgcccggctgcagatcgttcaaacatttggcaataaagtttcttaagattgaatcctgttgccggtcttgcgatgattatcatataatttctgttgaattacgttaagcatgtaataattaacatgtaatgcatgacgttatttatgagatgggtttttatgattagagtcccgcaattatacatttaatacgcgatagaaaacaaaatatagcgcgcaaactaggataaattatcgcgcgcggtgtcatctatgttactagatccgatgataagctgtcaaacatga

SEQ ID NO: 34 - DNA, 377 bp, Oryza sativa
  misc_feature 1..377: note = RNA pol III promoter promoter from the rice U3 small nucle ar RNAgene (OsU3)
  source 1..377: mol_type = genomic DNA
aagggatctttaaacatacgaacagatcacttaaagttcttctgaagcaacttaaagttatcaggcatgcatggatcttggaggaatcagatgtgcagtcagggaccatagcacaggacaggcgtcttctactggtgctaccagcaaatgctggaagccgggaacactgggtacgttggaaaccacgtgatgtggagtaagataaactgtaggagaaaagcatttcgtagtgggccatgaagcctttcaggacatgtattgcagtatgggccggcccattacgcaattggacgacaacaaagactagtattagtaccacctcggctatccacatagatcaaagctggtttaaaagagttgtgcagatgatccgtggc

SEQ ID NO: 35 - DNA, 7787 bp, Oryza sativa
  misc_feature 1..7787: note = rice Protoporphyrinogen Oxidase (PPO2)
  source 1..7787: mol_type = genomic DNA
atgctctctcctgccaccaccttctcctcctcctcctcctcctcgtcgccgtcgcgcgcccacgctcgcgctcccacccgcttcgcggtcgcagcatccgcgcgcgccgcacggttccgccccgcgcgcgccatggccgcctccgacgacccccgcggcgggaggtccgtcgccgtcgtcggcgccggcgtcaggtgggtggggagccgcgcgcgctctccgtgggttcagttctgccctaggtttggggtgccgtgtgcgtgtgagtggggaggttgttttttttgatgattgatgaaatggttgcctctctgcagtgggctcgcggcggcgtacaggctgaggaagcgcggcgtgcaggtgacggtgttcgaggcggccgacagggcgggtgggaagatacggaccaactccgagggcgggttcatctgggacgaaggggccaacaccatggtgagcgcgctttggtgtgcctcgctgcttctgtttgatcacaatctcgggctgtgttggtctgcattgctgcaaatgctgcttctgtatgttttggattgtggcgcactggcgctgctgcggctatttgagggctggagcacactagcgagtagtgctccttggtgcgcaggctgaggaaacttgtgtttgtgaacgaaatgcaagctgctcactaatgcagacagttgttcctgcaaatggagaagtgttttcttctgcattcgtatcccacaacagacgtgaaccctttctgctatgagcatcattgaacaccgttatgtaacttatcatagcctgattcgatttcattcaccatgatctataactattatacttaccatattagttactttgtactactcttagtaaaataaataaattattttaatactccactgacaaaataggttaagattgtttcattgcttgggcacatgtgcaatactagtcgcattttttttacctgcgtgcaaatcttatcatgcctgcttgattcaatttgccgttctctctgtaatttaattattttgcctccagacagagagtgaattggaggcaagcaggcttattgacgatcttggcctacaaggcaaacagcagtatgtatgtgctaatgttatctgtgatggttaactgctttgaatgtcttctgtttcataatttacactgatatgtttaatatttcgatatcctttagcctaactcacaacacaagcgttacattgtcaaagatggagcaccaacactggtaaatagacttttcatgatatgatgcattttgttttgttcttcctatagtatgcctcacttttgaatatatttttttgtcacataagattccctcagatcccattgcgctcatgaaaagcactgttctttctacaaaatcaaaggtatgtaagttattgagtgctaattgctacaacatatcatgacctcctgacctatttgcaacaagttgcttgttgtttccacttgtcactgatggattaaaattcactagtgtagaaacaatcatattaaactgatcaccgtgacttgatttacttgttttcagttcactattacaaatttgtacatttcctgatctttcgtgttcaagctgtgtgatcgactgattgcaaccgtcatattatattactgtattgagtttagtaaaacatggtcttatctttgcagctcaagctatttctggaaccatttctctatgagaaatctagcagaaggacctcgggaaaagtgtctgatgaacatttaagtgagaggtgagccttcatactgatgttattttgagttgttgtaaacttgaaccactgataatatagttatatgtttttttcctgtgttcttccttcattctcatgcccttgtgaaatacaaatatatacttcatatcacacactccctttggtcatttttcatgtcaaacttttaaaactttgtacataaaatcagttcaatatttagattgaacgcatgagaaagtattttcataatattatgattttaccatttttttcatatacgttgcaacagaatttagtggtcaaagctacactttgaagaccttattgatgtcaaaaacagcatgttttctgaccagagagaatacatttgcagtgtgatttttctgtgtatatgtagagataatcaggtttctcttttgcagtgttgcaagtttctttgaacgccactttggaaaagaggcaagttcatttttaatgaagaaatttatggattgttaagtgaatacaatcaacactttgcaacttacatgcccattataatcagtagagggtaagaatttataactttattacaggttgttgattatcttattgatccatttgtggctggaacaagcggaggagatcctgagtcattatcagtaagttattataacatgtctcactatttgcattttccatatcagcacctttgcatttctacagtaaattgtagtcataattatttttatgtaaattgtgcgtataaacaacatatgtgcttgactttgtgatgtgttcttggggatgataactgatacggctagaacttttgggggctaatctccttgagccgtatcagtaagtcataacaattctcattcataatgatcaaaacatatcaccttcttgtgtagaactgttctggttttgagtaatattttcttctgtgcagattcgtcatgcatttccagcattatggaatttggagaataagtaagtttgtagtagtttgtttggagaataagtaagtttgtagtttgtgcattgatgttcattcaagatttaccttatcaataattcacttgtccacgtccatatgctcgtgctatatcctgtccattcaaatgtcaacaccgccatgtgaatttactgcatagtgcattttaatgatttcatttatccttgttgcttgcatctcttttttgggctcctgctgttagcttgtttttggttcctgctgttacctatttcttttctatcattttttcattggacagatggtgctctcagtccttactgcttattatttgttaacctgatatgcacctacttgaagttaatgttatgatttttagtattttatagtcatggtatcattaatacttatttttggcaatcgaaattaaaaaaacatgatgtcaaaataaaaaatcatggcagttgaatgcagtgggtatatgtatcaagaatttaagatcttgaacataagtccaattgctatatgttcaattcgttggagcataacatgatctaatttgtaagttaaatttatctgataaacgatggaaggaaattctggtaccactcatgcaactatacaagcttcaaaggcttcttacatgtggaccattggacctagaatagaatctaaatttattcataagtatataattttttttccttcatgggccatgatagttaactatatgagcttgtagagtcaaaataggcataattgcttctttgggtttccacttaatttaccctacaacacttctattgcaataaatatggtcaacaacatttctttacggtccgtttggttggagggagtttttaggagggattgggagtttagagggatggagctattaactgttttgtttggttgggagagatgggaattttggtgggatggagatggggaattgaggaaggaactccctccttttcaatacctgggtagggggtggtaattgggagggaattcctcctttactttgcctaaacaaatctcagccatccgttttcattaatgacctaatctccaactaaacttcctgtcaatttccaccacctctgccaaacaagatattgggattaaaaatcaaattcccatcttaatctcaccatcaattccctcgtgtaaactcccaatccccttccctcaagttgccaaacaagccattagtgcccagttatgttctttggtcatcttcttcataatttgttgctccatgcactttcaatgctcacaggtatggctctgtcattgctggtgccatcttgtccaaactatccactaagggtgattcagtgaagacaggaggtgcttcgccagggaaaggaaggaataaacgtgtgtcattttcatttcatggtggaatgcaggtactccacagatgtcctgtagtttcttttgtcagtgtcaaagatatcaaagacagtgataaaccctgaactttagtttgagcaattctacatgccactaaaaaatgccgaattcatatgttgtgaattgaagacctgttattttcctgcaactaggacatatgtttagtcggtgaaacttcattgctgctttaagaagtcttacaggccagagaaaactgtcttgttttttttttttttgatttgatgtcctgctttatatttatgatccagccaagcttatccatccatctgcaccctgatcctgccataatcattttttttatcagcctgacatgagcttattatgttgcataagttaggttgaagctagatcgaacaaaaaactcaaagctactgataagtacaggatatgcaacagaagtatcacacgagccaaatctgctataagaataaaacataccaagagccttagacaccactaaatagtgtgaatggtagtgatagcgaataatctcagaagatgacattttgggaaatattatcgtgtagtatactttattaattgggagttgcgatacttgccctgcacgctaaacatgctgaaaagtttcacagttatactacataacatctgggtgtgtaaaggttttatgttgttcattgcttttcagtcactaatagatgcacttcacaatgaagttggagatggtaacgtgaagcttggtacagaagtgttgtcattggcatgttgctgtgatggagtctcttcttctggtggttggtcaatttctgttgattcaaaagatgctaaagggaaagatctcagaaagaaccaatctttcgatgctgttataatgactgtaagaaaaaaattatctgtattcatctctttagaagcttgatcatttgacagccacaaattaaaatattttaccgtgtttttctttttgcccctttaggctccattgtctaatgtccagaggatgaagtttacaaaaggtggagttccctttgtgctagactttcttcctaaggtcaggttagaatcactcttttagatttaacaaatgcagtgttgcactagcatgttcttgagaaatttgtgctgggggaaattcctcttaatccttcaaattgcatttaatttcatccattaggtcgatggatccatgtcacagaaaatattttgtttatcttctagatttctattatatatgtaagactgtctcttagtttgtgaatttacaggagtcaatcatcactcccttgaatctgagcatatcagcagttcatcagcaatatggtttatttgagaaggcaacggaaactattgtttccaaaggccacttgtttgaaactttcaccactgttttgaacagtgtattaaagtaacagtcatttgtatagcagcacctggtgatttttaagtaaattttccattcccaatcaaaacaagtaacattatatgttgaacatgtactgaattgaatatggaactttatgctggagatgccagactttattttactggcatgaatacacaattattgtaacaatggtattattgcttggttacttctccgctgtgaagacatacctttcgtcaccttttcttgtttcccatattctgcaccttatgggattgtcttccacatgttaagatgccttgtagtaccagttcccctattatttgaatgtgttcttccttagatatatgtgcatttggaacgtgattggaaatacaacagcaaactggtattgttagctgcttgcctgccacagcctacatatgctgccatattacagaattatgagataggtggactttgatttctgtcataatgattaactaacttgatatactcaaactatgcagctcctagctggtatccttagaatttatcgagtatgcatagaagtctactcttaatccatatctatttgatgtactcaaacttgaaactatgcagctcctagctgggctccttagaattatcaagtatgcatagaaatcttaatccatatttatttattatatgcaggtcgattatctaccactatctctcatggtaacagcttttaagaaggaagatgtcaaaaaaccattggaaggatttggtgccttgataccctataaggaacagcaaaagcatggtctcaaaacccttggtaggttaattcagctttacacttatattttatccagcttgtagctgcttatattttgatttgcgaattaaaaattattaaaacagccttgaaagaagaaaccatgttcgctgtggagactagaaattcccacattaattggggaaagagaaatatttacaccctatgattttggcaagtgcaagttttaatggttgagattgatggattgaatatatatcatatttggactcagtatgaacaaataccagatacataaatagatagtactaattcaacatggatctgaactgttgatcagaccaattgagcacttggttgtaattgctcgcggactacacgcttactgcctgactagggttccatgatgataaggttcgattttctaaaatactattacaacaagatgactatttaataaaatttaaagagaataacgtatataaaaatttagataaatttggtgcaccgcgcaattgcgcaggtcaccctgctagctgtattgaactcaatatacaaatcaaccttgctacattgctctactttttctcaggtcttatttactctgatttctatttattctaatctatacatgtcgtcttgtacagggaccctcttctcctcgatgatgtttccagatcgagctcctaatgatcaatatctatatacatctttcattggggggagccataatagagacctcgctggggctccaacgtatacttccatattatgatcatttatgttttggttgttttttcttttcttgctagatttttctgatatatatacttatgtagggctattctgaaacaacttgtgacctctgacctaagaaagctcttgggtgttgagggacaacctacttttgtgaagtaagtgataagaaactactgccatggtttagagtatctatatgttttctcttgttgtgcttgtgttatggttttccatcactatggagttttgaggattcattcaggtttttgcactaccacttgcgaattcaatatgatgttcttttacacaggcatgtacattggagaaatgcttttcctttatatggccagaattatgatctggtactggaagctatagcaaaaatggagaacaatcttccagggttcttttacgcaggcaagtcaatgaaggcacccctattgtacaaaagaaatcttagatatttgaaacatattcctgttgattgagtacgtgaataatttgctgtttctagtaagtcaatttggtatttctcatgcaacttatggggctccttgatttgctgagaatgatgagtttcctagagcaagccaggaactgtaatcccagcatgtaatactttaccttgaaattaacttcaaaaaaataattgaagctttttctgtatctgtaggaaataacaaggatgggttggctgttggaaatgttatagcttcaggaagcaaggctgctgaccttgtgatctcttatcttgaatcttgcacagatcaggacaattag

SEQ ID NO: 36 - DNA, 20 bp, synthetic construct
  misc_feature 1..20: note = spacer 8
  source 1..20: mol_type = other DNA
atggtctcaaaacccttggt

SEQ ID NO: 37 - DNA, 20 bp, synthetic construct
  misc_feature 1..20: note = spacer 9
  source 1..20: mol_type = other DNA
acacgcttactgcctgacta

SEQ ID NO: 38 - DNA, 20 bp, synthetic construct
  misc_feature 1..20: note = spacer 10
  source 1..20: mol_type = other DNA
tatatacatctttcattggg

SEQ ID NO: 39 - DNA, 120 bp, synthetic construct
  misc_feature 1..120: note = donor 6
  source 1..120: mol_type = other DNA
gaaggatttggtgccttgataccctataaggaacagcaaaagcatggtctcaaaacctttggtagattaattcagctttacacttatattttatccagcttgtagctgcttatattttga

SEQ ID NO: 40 - DNA, 794 bp, synthetic construct
  misc_feature 1..794: note = donor 7
  source 1..794: mol_type = other DNA
gaaggatttggtgccttgataccctataaggaacagcaaaagcatggtctcaaaacctttggtaggttaattcagctttacacttatattttatccagcttgtagctgcttatattttgatttgcgaattaaaaattattaaaacagccttgaaagaagaaaccatgttcgctgtggagactagaaattcccacattaattggggaaagagaaatatttacaccctatgattttggcaagtgcaagttttaatggttgagattgatggattgaatatatatcatatttggactcagtatgaacaaataccagatacataaatagatagtactaattcaacatggatctgaactgttgatcagaccaattgagcacttggttgtaattgctcgcggactacacgcttactgcctgactagcgttccatgatgataaggttcgattttctaaaatactattacaacaagatgactatttaataaaatttaaagagaataacgtatataaaaatttagataaatttggtgcaccgcgcaattgcgcaggtcaccctgctagctgtattgaactcaatatacaaatcaaccttgctacattgctctactttttctcaggtcttatttactctgatttctatttattctaatctatacatgtcgtcttgtacagggaccctcttctcctcgatgatgtttccagatcgagctcctaatgatcaatatctatatacatctgtaattggggggagccataatagagacctcgctggggctccaacgtatacttccatatta

SEQ ID NO: 41 - DNA, 800 bp, synthetic construct
  misc_feature 1..800: note = donor 8
  source 1..800: mol_type = other DNA
atggatctgaactgttgatcagaccaattgagcacttggttgtaattgctcgcggactacacgcttactgcctgactagggttccatgatgataaggttcgattttctaaaatactattacaacaagatgactatttaataaaatttaaagagaataacgtatataaaaatttagataaatttggtgcaccgcgcaattgcgcaggtcaccctgctagctgtattgaactcaatatacaaatcaaccttgctacattgctctactttttctcaggtcttatttactctgatttctatttattctaatctatacatgtcgtcttgtacagggaccttcttctcctcgatgatgtttccagatcgagctcctaatgatcaatatctatatacatctgtaattggcggcagccataatagagacctcgctggggctccaacgtatacttccatattatgatcatttatgttttggttgttttttcttttcttgctagatttttctgatatatatacttatgtagggctattctgaaacaacttgtgacctctgacctaagaaagctcttgggtgttgagggacaacctacttttgtgaagtaagtgataagaaactactgccatggtttagagtatctatatgttttctcttgttgtgcttgtgttatggttttccatcactatggagttttgaggattcattcaggtttttgcactaccacttgcgaattcaatatgatgttcttttacacaggcatgtacattggagaaatgcttttcctttatatggccagaattatgat

SEQ ID NO: 42 - DNA, 138 bp, synthetic construct
  misc_feature 1..138: note = RecA FusionCRISPR
  source 1..138: mol_type = other DNA
gatgtggaaaccatctctacgttttagagctagaaatagcaagttaaaataaggctagtccgttatcaacttgaaaaagtggcaccgagtcggtgctttccatggatgtggaaaccatcgctttcactggatatcgcg

SEQ ID NO: 43 - DNA, 1062 bp, Escherichia coli
  misc_feature 1..1062: note = RecA
  source 1..1062: mol_type = genomic DNA
atggctatcgacgaaaacaaacagaaagcgttggcggcagcactgggccagattgagaaacaatttggtaaaggctccatcatgcgcctgggtgaagaccgttccatggatgtggaaaccatctctaccggttcgctttcactggatatcgcgcttggggcaggtggtctgccgatgggccgtatcgtcgaaatctacggaccggaatcttccggtaaaaccacgctgacgctgcaggtgatcgccgcagcgcagcgtgaaggtaaaacctgtgcgtttatcgatgctgaacacgcgctggacccaatctacgcacgtaaactgggcgtcgatatcgacaacctgctgtgctcccagccggacaccggcgagcaggcactggaaatctgtgacgccctggcgcgttctggcgcagtagacgttatcgtcgttgactccgtggcggcactgacgccgaaagcggaaatcgaaggcgaaatcggcgactctcacatgggccttgcggcacgtatgatgagccaggcgatgcgtaagctggcgggtaacctgaagcagtccaacacgctgctgatcttcatcaaccagatccgtatgaaaattggtgtgatgttcggtaacccggaaaccactaccggtggtaacgcgctgaaattctacgcctctgttcgtctcgacatccgtcgtatcggcgcggtgaaagagggcgaaaacgtggtgggtagcgaaacccgcgtgaaagtggtgaagaacaaaatcgctgcgccgtttaaacaggctgaattccagatcctctacggcgaaggtatcaacttctacggcgaactggttgacctgggcgtaaaagagaagctgatcgagaaagcaggcgcgtggtacagctacaaaggtgagaagatcggtcagggtaaagcgaatgcgactgcctggctgaaagataacccggaaaccgcgaaagagatcgagaagaaagtacgtgagttgctgctgagcaacccgaactcaacgccggatttctctgtagatgatagcgaaggcgtagcagaaactaacgaagatttttaa

SEQ ID NO: 44 - DNA, 21 bp, synthetic construct
  misc_feature 1..21: note = Primer
  source 1..21: mol_type = other DNA
atggctatcgacgaaaacaaa

SEQ ID NO: 45 - DNA, 21 bp, synthetic construct
  misc_feature 1..21: note = Primer
  source 1..21: mol_type = other DNA
cgtcagcgtggttttaccgga

SEQ ID NO: 46 - DNA, 461 bp, synthetic construct
  misc_feature 1..461: note = Expression Cassette
  source 1..461: mol_type = other DNA
tgtacaaaaaagcaggctttaaaggaaccaattcagtcgactggatccggtaccaaggtcgggcaggaagagggcctatttcccatgattccttcatatttgcatatacgatacaaggctgttagagagataattagaattaatttgactgtaaacacaaagatattagtacaaaatacgtgacgtagaaagtaataatttcttgggtagtttgcagttttaaaattatgttttaaaatggactatcatatgcttaccgtaacttgaaagtatttcgatttcttggctttatatatcttgtggaaaggacgaaacaccggcatccctcaggctgggctgttttagagctagaaatagcaagttaaaataaggctagtccgttatcaacttgaaaaagtggcaccgagtcggtgctggccatcaggcatccctcagtatggaatgaggcatctgattttttt

SEQ ID NO: 47 - DNA, 275 bp, Homo sapiens
  misc_feature 1..275: note = PRDM9 exon ENSE00001804383
  source 1..275: mol_type = genomic DNA
attgtgagatgtgtcagaacttcttcattgacagctgtgctgcccatgggccccctacatttgtaaaggacagtgcagtggacaaggggcaccccaaccgttcagccctcagtctgcccccagggctgagaattgggccatcaggcatccctcaggctgggcttggagtatggaatgaggcatctgatctgccgctgggtctgcactttggcccttatgagggccgaattacagaagacgaagaggcagccaacaatggatactcctggctgtgg

SEQ ID NO: 48 - DNA, 783 bp, synthetic construct
  misc_feature 1..783: note = Gene Fragment
  source 1..783: mol_type = other DNA
cacctaggggggaggtcgtagtacccccctatgttttctcccctaaataaccccaaaaatctaagaaaaaaagacctcaaaaaggtctttaattaacatctcaaatttcgcatttattccaatttcctttttgcgtgtgatgcgaattcttgaccgtgattagagaattgagtaaaatgtacctacgcgagacctcattcgccattcaggctacgcaactgttgggaagggcgatcggtgcgggcctcttcgctattacgccatgaggcgaaagggggatgtgctgcaaggcgattaagttgggtaacgccagggttttcccagtcacgacgttgtaaaacgacggccagactattcgtaatcatggtcatagctgtttcctgtgtgaaattgttatccgctcacaattccacacaacatacgagccggaagcataaagtgtaaagcctggggtgcctaatgagtgagctaactcacattaattgcgttgcgctcactgcccgctttccagtcgggaaacctgtcgtgccagctcgattaatgaatcggtctcagttttagagctagaaatagcaagttaaaataaggctagtccgttatcaacttgaaaaagtggcaccgagtcggtgctggccaacgaggcccgggccaataaggccttttttactccatctggatttgttcagaacgctcggttgccgccgggcgttttttatctaaagcttaggcccagtcgaaagactgggcctttttaatacgactcactatagggtcgactctaga

SEQ ID NO: 49 - DNA, 784 bp, synthetic construct
  misc_feature 1..784: note = Gene Fragment
  source 1..784: mol_type = other DNA
cacctaggggggaggtcgtagtacccccctatgttttctcccctaaataaccccaaaaatctaagaaaaaaagacctcaaaaaggtctttaattaacatctcaaatttcgcatttattccaatttcctttttgcgtgtgatgcgaattcttgaccgtgattagagaattgagtaaaatgtacctacggccaacgaggcccgggccaataaggcctacgcgagacctcattcgccattcaggctacgcaactgttgggaagggcgatcggtgcgggcctcttcgctattacgccatgaggcgaaagggggatgtgctgcaaggcgattaagttgggtaacgccagggttttcccagtcacgacgttgtaaaacgacggccagactattcgtaatcatggtcatagctgtttcctgtgtgaaattgttatccgctcacaattccacacaacatacgagccggaagcataaagtgtaaagcctggggtgcctaatgagtgagctaactcacattaattgcgttgcgctcactgcccgctttccagtcgggaaacctgtcgtgccagctcgattaatgaatcggtctcagttttagagctagaaatagcaagttaaaataaggctagtccgttatcaacttgaaaaagtggcaccgagtcggtgctttttactccatctggatttgttcagaacgctcggttgccgccgggcgttttttatctaaagcttaggcccagtcgaaagactgggcctttttaatacgactcactatagggtcgactctaga

SEQ ID NO: 50 - DNA, 24 bp, synthetic construct
  misc_feature 1..24: note = Oligonucleotide
  source 1..24: mol_type = other DNA
tacgtgaagatcaggctatcactg

SEQ ID NO: 51 - DNA, 24 bp, synthetic construct
  misc_feature 1..24: note = Oligonucleotide
  source 1..24: mol_type = other DNA
aaaccagtgatagcctgatcttca

SEQ ID NO: 52 - DNA, 52 bp, synthetic construct
  misc_feature 1..52: note = Oligonucleotide
  source 1..52: mol_type = other DNA
gatcggccaacgaggccgcggcattatgtttgaatttccgtttaaagaatgg

SEQ ID NO: 53 - DNA, 76 bp, synthetic construct
  misc_feature 1..76: note = Oligonucleotide
  source 1..76: mol_type = other DNA
gatggtttctttcggtaagtcccgtctagccttgccctcatcttgacactccttatttgattttttgaagacttac

SEQ ID NO: 54 - DNA, 40 bp, synthetic construct
  misc_feature 1..40: note = Oligonucleotide
  source 1..40: mol_type = other DNA
tgagggcaaggctagacgggacttaccgaaagaaaccatc

SEQ ID NO: 55 - DNA, 56 bp, synthetic construct
  misc_feature 1..56: note = Oligonucleotide
  source 1..56: mol_type = other DNA
gatcaggccttattggccttggcaggccgctgaatttccatgttgcgtaagtcagg

SEQ ID NO: 56 - DNA, 52 bp, synthetic construct
  misc_feature 1..52: note = Oligonucleotide
  source 1..52: mol_type = other DNA
gatcggccaacgaggccttggcaggccgctgaatttccatgttgcgtaagtc

SEQ ID NO: 57 - DNA, 76 bp, synthetic construct
  misc_feature 1..76: note = Oligonucleotide
  source 1..76: mol_type = other DNA
cgaagtaagtcttcaaaaaatcaaataaggagtgtcaagatgagggcaaggctagacgggacttaccgaaagaaac

SEQ ID NO: 58 - DNA, 40 bp, synthetic construct
  misc_feature 1..40: note = Oligonucleotide
  source 1..40: mol_type = other DNA
tcttgacactccttatttgattttttgaagacttacttcg

SEQ ID NO: 59 - DNA, 57 bp, synthetic construct
  misc_feature 1..57: note = Oligonucleotide
  source 1..57: mol_type = other DNA
gatcggccttattggccgcggcattatgtttgaatttccgtttaaagaatggtctgc

SEQ ID NO: 60 - DNA, 19 bp, synthetic construct
  misc_feature 1..19: note = Oligonucleotide
  source 1..19: mol_type = other DNA
gactttcaggcgtgaatgg

SEQ ID NO: 61 - DNA, 20 bp, synthetic construct
  misc_feature 1..20: note = Oligonucleotide
  source 1..20: mol_type = other DNA
cgtgctctccgataatatgc

SEQ ID NO: 62 - DNA, 6588 bp, synthetic construct
  misc_feature 1..6588: note = Vector RLW121
  source 1..6588: mol_type = other DNA
ccgtttaaacttagttactaatcagtgatcagattgtcgtttcccgccttcactttaaactatcagtgtttgacaggatatattggcgggtaaacctaagagaaaagagcgtttattagaataatcggatatttaaaagggcgtgaaaaggtttatccgttcgtccatttgtatgtcaatattgggggggggggaaagccacgttgtgtctcaaaatctctgatgttacattgcacaagataaaaatatatcatcatgaacaataaaactgtctgcttacataaacagtaatacaaggggtgttcgccaccatgagccatatccagcgtgaaacctcgtgctcccgcccgcgcctcaattccaatatggatgccgacctttatggctacaagtgggcgcgcgacaacgtcggccagtcgggcgcgaccatttatcggctttatggcaaacccgatgccccggaactgttcctgaagcacggcaaaggcagcgtcgcaaacgatgtcaccgatgagatggtccgcctgaactggcttaccgagttcatgccgctgccgacgattaagcatttcatccgtaccccggacgatgcctggctcttgaccacggccattccgggcaaaacggcctttcaggtccttgaagagtacccggactccggtgagaatatcgtggacgccctcgcggtcttcctccgccgtttgcatagcatccccgtgtgcaactgccccttcaactcggaccgggttttccgcctggcacaggcccagtcgcgcatgaataacggcctcgttgacgcgagcgatttcgacgatgaacggaatggctggccggtggaacaggtttggaaggaaatgcacaaactgcttccgttctcgccggattcggtggtcacgcatggtgatttttccctggataatctgatctttgacgagggcaagctgatcggctgcatcgacgtgggtcgcgtcggtatcgccgaccgctatcaggacctggcgatcttgtggaattgcctcggcgagttctcgccctcgctccagaagcgcctgttccagaagtacggcatcgacaacccggatatgaacaagctccagttccacctcatgctggacgaatttttttgaacagaattggttaattggttgtaacactggcagagcattacgctgacttgacgggacggcggctttgttgaataaatcgaacttttgctgagttgaaggatcgatgagttgaaggaccccgtagaaaagatcaaaggatcttcttgagatcctttttttctgcgcgtaatctgctgcttgcaaacaaaaaaaccaccgctaccagcggtggtttgtttgccggatcaagagctaccaactctttttccgaaggtaactggcttcagcagagcgcagataccaaatactgtccttctagtgtagccgtagttaggccaccacttcaagaactctgtagcaccgcctacatacctcgctctgctaatcctgttaccagtggctgctgccagtggcgataagtcgtgtcttaccgggttggactcaagacgatagttaccggataaggcgcagcggtcgggctgaacggggggttcgtgcacacagcccagcttggagcgaacgacctacaccgaactgagatacctacagcgtgagctatgagaaagcgccacgcttcccgaagggagaaaggcggacaggtatccggtaagcggcagggtcggaacaggagagcgcacgagggagcttccagggggaaacgcctggtatctttatagtcctgtcgggtttcgccacctctgacttgagcgtcgatttttgtgatgctcgtcaggggggcggagcctatggaaaaacgccagcaacgcggcctttttacggttcctggccttttgctggccttttgctcacatgttctttcctgcgttatcccctgattctgtggataaccgtattaccgcctttgagtgagctgataccgctcgccgcagccgaacgaccgagcgcagcgagtcagtgagcgaggaagcggaagagcgcctgatgcggtattttctccttacgcatctgtgcggtatttcacaccgcataggccgcgataggccgacgcgaagcggcggggcgtagggagcgcagcgaccgaagggtaggcgctttttgcagctcttcggctgtgcgctggccagacagttatgcacaggccaggcgggttttaagagttttaataagttttaaagagttttaggcggaaaaatcgccttttttctcttttatatcagtcacttacatgtgtgaccggttcccaatgtacggctttgggttcccaatgtacgggttccggttcccaatgtacggctttgggttcccaatgtacgtgctatccacaggaaagagaccttttcgacctttttcccctgctagggcaatttgccctagcatctgctccgtacattaggaaccggcggatgcttcgccctcgatcaggttgcggtagcgcatgactaggatcgggccagcctgccccgcctcctccttcaaatcgtactccggcaggtcatttgacccgatcagcttgcgcacggtgaaacagaacttcttgaactctccggcgctgccactgcgttcgtagatcgtcttgaacaaccatctggcttctgccttgcctgcggcgcggcgtgccaggcggtagagaaaacggccgatgccggggtcgatcaaaaagtaatcggggtgaaccgtcagcacgtccgggttcttgccttctgtgatctcgcggtacatccaatcagcaagctcgatctcgatgtactccggccgcccggtttcgctctttacgatcttgtagcggctaatcaaggcttcaccctcggataccgtcaccaggcggccgttcttggccttcttggtacgctgcatggcaacgtgcgtggtgtttaaccgaatgcaggtttctaccaggtcgtctttctgctttccgccatcggctcgccggcagaacttgagtacgtccgcaacgtgtggacggaacacgcggccgggcttgtctcccttcccttcccggtatcggttcatggattcggttagatgggaaaccgccatcagtaccaggtcgtaatcccacacactggccatgccggcggggcctgcggaaacctctacgtgcccgtctggaagctcgtagcggatcacctcgccagctcgtcggtcacgcttcgacagacggaaaacggccacgtccatgatgctgcgactatcgcgggtgcccacgtcatagagcatcggaacgaaaaaatctggttgctcgtcgcccttgggcggcttcctaatcgacggcgcaccggctgccggcggttgccgggattctttgcggattcgatcagcggccccttgccacgattcaccggggcgtgcttctgcctcgatgcgttgccgctgggcggcctgcgcggccttcaacttctccaccaggtcatcacccagcgccgcgccgatttgtaccgggccggatggtttgcgaccgctcacgccgattcctcgggcttgggggttccagtgccattgcagggccggcagacaacccagccgcttacgcctggccaaccgcccgttcctccacacatggggcattccacggcgtcggtgcctggttgttcttgattttccatgccgcctcctttagccgctaaaattcatctactcatttattcatttgctcatttactctggtagctgcgcgatgtattcagatagcagctcggtaatggtcttgccttggcgtaccgcgtacatcttcagcttggtgtgatcctccgccggcaactgaaagttgacccgcttcatggctggcgtgtctgccaggctggccaacgttgcagccttgctgctgcgtgcgctcggacggccggcacttagcgtgtttgtgcttttgctcattttctctttacctcattaactcaaatgagttttgatttaatttcagcggccagcgcctggacctcgcgggcagcgtcgccctcgggttctgattcaagaacggttgtgccggcggcggcagtgcctgggtagctcacgcgctgcgtgatacgggactcaagaatgggcagctcgtacccggccagcgcctcggcaacctcaccgccgatgcgcgtgcctttgatcgcccgcgacacgacaaaggccgcttgtagccttccatccgtgacctcaatgcgctgcttaaccagctccaccaggtcggcggtggcccaaatgtcgtaagggcttggctgcaccggaatcagcacgaagtcggctgccttgatcgcggacacagccaagtccgccgcctggggcgctccgtcgatcactacgaagtcgcgccggccgatggccttcacgtcgcggtcaatcgtcgggcggtcgatgccgacaacggttagcggttgatcttcccgcacggccgcccaatcgcgggcactgccctggggatcggaatcgactaacagaacatcggccccggcgagttgcagggcgcgggctagatgggttgcgatggtcgtcttgcctgacccgcctttctggttaagtacagcgataaccttcatgcgttccccttgcgtatttgtttatttactcatcgcatcatatacgcagcgaccgcatgacgcaagctgttttactcaaatacacatcacctttttagatgatcagtgattttgtgccgagctgccggtcggggagctgttggctggctggtggcaggatatattgtggtgtaaacaaattgacgcttagacaacttaataacacattgcggacgtctttaatgtactgaatttagttactgatcactgattaagtactgataaatttaattaacagatctcaactttgtatagaaaagttgaacgagaaacgtaaaatgatataaatatcaatatattaaattagattttgcataaaaaacagactacataatactgtaaaacacaacatatccagtcactatggtcgacctgcagactggctgtgtataagggagcctgacatttatattccccagaacatcaggttaatggcgtttttgatgtcattttcgcggtggctgagatcagccacttcttccccgataacggagaccggcacactggccatatcggtggtcatcatgcgccagctttcatccccgatatgcaccaccgggtaaagttcacgggggactttatctgacagcagacgtgcactggccagggggatcaccatccgtcgcccgggcgtgtcaataatatcactctgtacatccacaaacagacgataacggctctctcttttataggtgtaaaccttaaactgcatttcaccagcccctgttctcgtcggcaaaagagccgttcatttcaatgaaccgggcgacctcagccatcccttcctgattttccgctttccagcgttcggcacgcagacgacgggcttcattctgcatggttgtgcttaccgaaccggagatattgacatcatatatgccttgagcaactgatagctgtcgctgtcaactgtcactgtaatacgctgcttcatagcatacctctttttgacatacttcgggtatacatatcagtatatattcttataccgcaaaaatcagcgcgcaaatacgcatactgttatctggcttttagtaagccggatcctctagattacgccccgcctgccactcatcgcagtactgttgtaattcattaagcattctgccgacatggaagccatcacaaacggcatgatgaacctgaatcgccagcggcatcagcaccttgtcgccttgcgtataatatttgcccatggtgaaaacgggggcgaagaagttgtccatattggccacgtttaaatcaaaactggtgaaactcacccagggattggctgagacgaaaaacatattctcaataaaccctttagggaaataggccaggttttcaccgtaacacgccacatcttgcgaatatatgtgtagaaactgccggaaatcgtcgtggtattcactccagagcgatgaaaacgtttcagtttgctcatggaaaacggtgtaacaagggtgaacactatcccatatcaccagctcaccgtctttcattgccatacggaattccggatgagcattcatcaggcgggcaagaatgtgaataaaggccggataaaacttgtgcttatttttctttacggtctttaaaaaggccgtaatatccagctgaacggtctggttataggtacattgagcaactgactgaaatgcctcaaaatgttctttacgatgccattgggatatatcaacggtggtatatccagtgatttttttctccattttagcttccttagctcctgaaaatctcgacggatcctaactcaaaatccacatattatacgagccggaagcataaagtgtaaagcctggggtgcctaatgcggccgccatagtgactggatatgttgtgttttacagtattatgtagtctgttttttatgcaaaatctaatttaatatattgatatttatatcattttacgtttctcgttcaactttattatacatagttgataattcactgggccgg

SEQ ID NO: 63 - DNA, 7443 bp, synthetic construct
  misc_feature 1..7443: note = Vector CC003
  source 1..7443: mol_type = other DNA
ctaaattgtaagcgttaatattttgttaaaattcgcgttaaatttttgttaaatcagctcattttttaaccaataggccgaaatcggcaaaatcccttataaatcaaaagaatagaccgagatagggttgagtggccgctacagggcgctcccattcgccattcaggctgcgcaactgttgggaagggcgtttcggtgcgggcctcttcgctattacgccagctggcgaaagggggatgtgctgcaaggcgattaagttgggtaacgccagggttttcccagtcacgacgttgtaaaacgacggccagtgagcgcgacgtaatacgactcactatagggcgaattggcggaaggccgtcaaggccgcataaataatgattttattttgactgatagtgacctgttcgttgcaacaaattgataagcaatgcttttttataatgccaactttgtatagaaaagttgatttaaatgaattcaagcttttaattaacttagccactgcaacaagttcttgaaccttagcacaatcatattgtgcatgcacttgtttattgcaaagaatggtgcgtagggaacacgcatgatttttgaattgctggcacataattttatcattagaaactggaatgcaacatgtaccctttgtcatggtttctttccgagacattgcactgttttttttaatcctatcattatcataatgccaagaactggtcaccaaccagcattttgcatcatggttagttgagctgtccccatgtatcaataggtgcattgtattggtccaaaatataaatgcagtggatgcaacctatctcatggccgtcaacaaaagaaatcaaaagggaaatgcaccatcttatatctccagtttatatgaacagattggataagatcataagatcaagtggtttatattattttgaggaatataacatggattcatcctaatcactcgtctaggcagtatgtgtattcatgatggatatggtactatactacggagttttttcttcacaaaataacctgttattttgacctccaaccaaacacgaattataccaaaaattgggttatttcatctatagtacaactctattataaacatgcagtaaattatcctacacatataccaaaattcaagtgtaataatcctaatacacagacttaaaaaacaaactatttcctttttaagaaaaggaaaaccatttttttaacggaaggaaaacaaattcgggtcaaggcggaagccagcgcgccaccccacgtcagcgaatacggaggcgcggggttgacggcgtcacccggtcctaacggcgaccaacaaaccagccagaagaaattacagtaaaaaaaagtaaattgcactttgatccaccttttattacccaagtttcaatttggaccacccttaaacctatcttttcaaattgggccgggttgtggtttggactaccatgaacaacttttcgtcatgtctaacttccctttcggcaaacatatgaaccatatatagaggagatcggccgtatactagagctgatgtgtttaaggtcgttgattgcacgagaaaaaaaaaatccaaatcgcaacaatagcaaatttatctagttcaaagtgaaaagatatgtttaaaggtagtccaaagtaaaacttaggggctgtttggttcccagccatactttaccattacttgccaacaaaagttgccacaccttgtctaaggtgaggtgatcaaattgttagccacaacttactaagcctaagggaatcttgccacacttttttgagccattgacacgtgggacttaatttgttagagggaaatcttgccacaactgtggctacaaccaaacacctgtcaaatttgcctaaccttaggcgtggcaaactgtggcaaagtgtggcttacaaccaaacacacccttagataataaaatgtggtccaaagcgtaattcactaaaaaaaaatcaacgagacgtgtaccaaacggagacaaacggcatcttctcgaaatttcccaaccgctcgctcgcccgcctcgtcttcccggaaaccgcggtggtttcagcgtggcggattctccaagcagacggagacgtcacggcacgggactcctcccaccacccaaccgccataaataccagccccctcatctcctctcctcgcatcagctccacccccgaaaaatttctccccaatctcgcgaggctctcgtcgtcgaatcgaatcctctcgcgtcctcaagcttggcatccaggtacggatccgcgtcccatctccctcaccccccgtgttcttcgtgcctgcttctgggtcagatctgggtggattcgcggttgttggatgtggggggctgtgtttatttgtcggtggatctggttgtctggatctgcgttttctctgtcgtagttagcggatctgatgaaatgtttagtgttcgtgtatactggtatggtggatctggtcctaggatgcgtggaatggatatatgtaggcgaattggaggatttattttgtgaattttgctgaaatgatagttctaaacactggatctgacctcgggatgctgttaaatgtggaaatcatggtcgatgctgtcatgaacatggtgttcttatggtagatctgagcaatgtatgtttcaaaattgtttgtcacatggaaatgctatggttctagatgcaatagaatgatacatgccgagatcccctctagttgatatgatagatcatgatgttttacagctatgtcatatgaatatgttcatttgttaccgatgtatttggatctacttaacatttccaaagcacgccgcgttctaattctagatctggtagtcatgtttgtacacgtcacccacctaatacaaatacatatgtctagtgtttggtgacactgcccgtcagatctgttttttccagatctgtggaacaaatactccacgcatgtatggtagttttgaaacgatcttgtatcttccattgttgtagtaacaactaaataaagtacaattgttcaattattgggaatcgtattttctgtagtgccgatgtacagcatattcatagatgtctatttaggaactcaaattttaaattgaggactagttatttattgtgggtcagtcttttgaattgtgttatcttgctgtactggcgcgccaccatggccaccgccgccgccgcgtctaccgcgctcactggcgccactaccgctgcgcccaaggcgaggcgccgggcgcacctcctggccacccgccgcgccctcgccgcgcccatcaggtgctcagcggcgtcacccgccatgccgatggctcccccggccaccccgctccggccgtggggccccaccgatccccgcaagggcgccgacatcctcgtcgagtccctcgagcgctgcggcgtccgcgacgtcttcgcctaccccggcggcacgtccatggagatccaccaggcactcacccgctcccccgtcatcgccaaccacctcttccgccacgagcaaggggaggcctttgcggcctccggctacgcgcgctcctcgggccgcgtcggcgtctgcatcgccacctccggccccggcgccaccaaccttgtctccgcgctcgccgacgcgctgctcgattccgtccccatggtcgccatcacgggacaggtgccgcgacgcatgattggcaccgacgccttccaggagacgcccatcgtcgaggtcacccgctccatcaccaagcacaactacctggtcctcgacgtcgacgacatcccccgcgtcgtgcaggaggctttcttcctcgcctcctctggtcgaccggggccggtgcttgtcgacatccccaaggacatccagcagcagatggcggtgcctgtctgggacaagcccatgagtctgcctgggtacattgcgcgccttcccaagccccctgcgactgagttgcttgagcaggtgctgcgtcttgttggtgaatcccggcgccctgttctttatgttggcggtggctgcgcagcatctggtgaggagttgcgacgctttgtggagctgactggaatcccggtcacaactactcttatgggcctcggcaacttccccagcgacgacccactgtctctgcgcatgctaggtatgcatggcacggtgtatgcaaattatgcagtggataaggccgatctgttgcttgcacttggtgtgcggtttgatgatcgtgtgacagggaagattgaggcttttgcaagcagggctaagattgtgcacgttgatattgatccggctgagattggcaagaacaagcagccacatgtgtccatctgtgcagatgttaagcttgctttgcagggcatgaatgctcttcttgaaggaagcacatcaaagaagagctttgactttggctcatggaacgatgagttggatcagcagaagagggaattcccccttgggtataaaacatctaatgaggagatccagccacaatatgctattcaggttcttgatgagctgacgaaaggcgaggccatcatcggcacaggtgttgggcagcaccagatgtgggcggcacagtactacacttacaagcggccaaggcagtggttgtcttcagctggtcttggggctatgggatttggtttgccggctgctgctggtgcttctgtggccaacccaggtgttactgttgttgacatcgatggagatggtagctttctcatgaacgttcaggagctagctatgatccgaattgagaacctcccggtgaaggtctttgtgctaaacaaccagcacctggggatggtggtgcagtgggaggacaggttctataaggccaacagagcgcacacatacttgggaaacccagagaatgaaagtgagatatatccagatttcgtgacgatcgccaaagggttcaacattccagcggtccgtgtgacaaagaagaacgaagtccgcgcagcgataaagaagatgctcgagactccagggccgtacctcttggatataatcgtcccacaccaggagcatgtgttgcctatgatccctaatggtggggctttcaaggatatgatcctggatggtgatggcaggactgtgtactagcctgcaggcctaggatcgttcaaacatttggcaataaagtttcttaagattgaatcctgttgccggtcttgcgatgattatcatataatttctgttgaattacgttaagcatgtaataattaacatgtaatgcatgacgttatttatgagatgggtttttatgattagagtcccgcaattatacatttaatacgcgatagaaaacaaaatatagcgcgcaaactaggataaattatcgcgcgcggtgtcatctatgttactagatcggccggccgtttaaacagcctgcttttttgtacaaagttggcattataaaaaagcattgctcatcaatttgttgcaacgaacaggtcactatcagtcaaaataaaatcattatttgctgggcctcatgggccttccgctcactgcccgctttccagtcgggaaacctgtcgtgccagctgcattaacatggtcatagctgtttccttgcgtattgggcgctctccgcttcctcgctcactgactcgctgcgctcggtcgttcgggtaaagcctggggtgcctaatgagcaaaaggccagcaaaaggccaggaaccgtaaaaaggccgcgttgctggcgtttttccataggctccgcccccctgacgagcatcacaaaaatcgacgctcaagtcagaggtggcgaaacccgacaggactataaagataccaggcgtttccccctggaagctccctcgtgcgctctcctgttccgaccctgccgcttaccggatacctgtccgcctttctcccttcgggaagcgtggcgctttctcatagctcacgctgtaggtatctcagttcggtgtaggtcgttcgctccaagctgggctgtgtgcacgaaccccccgttcagcccgaccgctgcgccttatccggtaactatcgtcttgagtccaacccggtaagacacgacttatcgccactggcagcagccactggtaacaggattagcagagcgaggtatgtaggcggtgctacagagttcttgaagtggtggcctaactacggctacactagaagaacagtatttggtatctgcgctctgctgaagccagttaccttcggaaaaagagttggtagctcttgatccggcaaacaaaccaccgctggtagcggtggtttttttgtttgcaagcagcagattacgcgcagaaaaaaaggatctcaagaagatcctttgatcttttctacggggtctgacgctcagtggaacgaaaactcacgttaagggattttggtcatgagattatcaaaaaggatcttcacctagatccttttaaattaaaaatgaagttttaaatcaatctaaagtatatatgagtaaacttggtctgacagttaccaatgcttaatcagtgaggcacctatctcagcgatctgtctatttcgttcatccatagttgcctgactccccgtcgtgtagataactacgatacgggagggcttaccatctggccccagtgctgcaatgataccgcgagaaccacgctcaccggctccagatttatcagcaataaaccagccagccggaagggccgagcgcagaagtggtcctgcaactttatccgcctccatccagtctattaattgttgccgggaagctagagtaagtagttcgccagttaatagtttgcgcaacgttgttgccattgctacaggcatcgtggtgtcacgctcgtcgtttggtatggcttcattcagctccggttcccaacgatcaaggcgagttacatgatcccccatgttgtgcaaaaaagcggttagctccttcggtcctccgatcgttgtcagaagtaagttggccgcagtgttatcactcatggttatggcagcactgcataattctcttactgtcatgccatccgtaagatgcttttctgtgactggtgagtactcaaccaagtcattctgagaatagtgtatgcggcgaccgagttgctcttgcccggcgtcaatacgggataataccgcgccacatagcagaactttaaaagtgctcatcattggaaaacgttcttcggggcgaaaactctcaaggatcttaccgctgttgagatccagttcgatgtaacccactcgtgcacccaactgatcttcagcatcttttactttcaccagcgtttctgggtgagcaaaaacaggaaggcaaaatgccgcaaaaaagggaataagggcgacacggaaatgttgaatactcatactcttcctttttcaatattattgaagcatttatcagggttattgtctcatgagcggatacatatttgaatgtatttagaaaaataaacaaataggggttccgcgcacatttccccgaaaagtgccac

SEQ ID NO: 64 - DNA, 3734 bp, synthetic construct
  misc_feature 1..3734: note = Vector CC018
  source 1..3734: mol_type = other DNA
cgcggatcatgaaccaacggcctggctgtatttggtggttgtgtagggagatggggagaagaaaagcccgattctcttcgctgtgatgggctggatgcatgcgggggagcgggaggcccaagtacgtgcacggtgagcggcccacagggcgagtgtgagcgcgagaggcgggaggaacagtttagtaccacattgcccagctaactcgaacgcgaccaacttataaacccgcgcgctgtcgcttgtgtgcattgagtgctatgctgaggttttagagctagaaatagcaagttaaaataaggctagtccgttatcaacttgaaaaagtggcaccgagtcggtgctctgttcctcgtgctggacaagtgtggtttccagattctgcaaccaagactgcgcaggcattgctggacttcaaccgtgaaggattacctctgttcatcctcgctaactggagaggcttctctggtggacaaagagatctctttgaaggaattcttcaggctggctcgactattgttgagaaccttaggacatacaatcagcctgcctttgtctacattcccatggctgcagagctacgaggaggggcttgggttgtggttgatagcaagataaacccagaccgcattgagtgctatgctgagagaactgcaaaatccaatgttctggaaccgcaagggttaattgagatcaagttcaggtcagaggaactccaggattgcatgagtcggcttgacccaacattaattgatctgaaagcaaaactcgaagtagcaaataaaaatggaagtgctgacacaaaatcgcttcaagaaaatatagaagctcgaacaaaacagttgatgcctctatatactcagattgcgatacggtttgctgaattgcatgatacatccctcagaatggctgcgaaaggtgtgattaagaaagttgtggactgggaagaatcacgatctttcttttttttgcggccgccccgggcctgcaggggatcccgatcgggccggccgtttaaacccactttgtacaagaaagttgaacgagaaacgtaaaatgatataaatatcaatatattaaattagattttgcataaaaaacagactacataatactgtaaaacacaacatatgcagtcactatgaaccaactacttagatggtattagtgacctgtactgggcctcatgggccttccgctcactgcccgctttccagtcgggaaacctgtcgtgccagctgcattaacatggtcatagctgtttccttgcgtattgggcgctctccgcttcctcgctcactgactcgctgcgctcggtcgttcgggtaaagcctggggtgcctaatgagcaaaaggccagcaaaaggccaggaaccgtaaaaaggccgcgttgctggcgtttttccataggctccgcccccctgacgagcatcacaaaaatcgacgctcaagtcagaggtggcgaaacccgacaggactataaagataccaggcgtttccccctggaagctccctcgtgcgctctcctgttccgaccctgccgcttaccggatacctgtccgcctttctcccttcgggaagcgtggcgctttctcatagctcacgctgtaggtatctcagttcggtgtaggtcgttcgctccaagctgggctgtgtgcacgaaccccccgttcagcccgaccgctgcgccttatccggtaactatcgtcttgagtccaacccggtaagacacgacttatcgccactggcagcagccactggtaacaggattagcagagcgaggtatgtaggcggtgctacagagttcttgaagtggtggcctaactacggctacactagaagaacagtatttggtatctgcgctctgctgaagccagttaccttcggaaaaagagttggtagctcttgatccggcaaacaaaccaccgctggtagcggtggtttttttgtttgcaagcagcagattacgcgcagaaaaaaaggatctcaagaagatcctttgatcttttctacggggtctgacgctcagtggaacgaaaactcacgttaagggattttggtcatgagattatcaaaaaggatcttcacctagatccttttaaattaaaaatgaagttttaaatcaatctaaagtatatatgagtaaacttggtctgacagttaccaatgcttaatcagtgaggcacctatctcagcgatctgtctatttcgttcatccatagttgcctgactccccgtcgtgtagataactacgatacgggagggcttaccatctggccccagtgctgcaatgataccgcgagaaccacgctcaccggctccagatttatcagcaataaaccagccagccggaagggccgagcgcagaagtggtcctgcaactttatccgcctccatccagtctattaattgttgccgggaagctagagtaagtagttcgccagttaatagtttgcgcaacgttgttgccattgctacaggcatcgtggtgtcacgctcgtcgtttggtatggcttcattcagctccggttcccaacgatcaaggcgagttacatgatcccccatgttgtgcaaaaaagcggttagctccttcggtcctccgatcgttgtcagaagtaagttggccgcagtgttatcactcatggttatggcagcactgcataattctcttactgtcatgccatccgtaagatgcttttctgtgactggtgagtactcaaccaagtcattctgagaatagtgtatgcggcgaccgagttgctcttgcccggcgtcaatacgggataataccgcgccacatagcagaactttaaaagtgctcatcattggaaaacgttcttcggggcgaaaactctcaaggatcttaccgctgttgagatccagttcgatgtaacccactcgtgcacccaactgatcttcagcatcttttactttcaccagcgtttctgggtgagcaaaaacaggaaggcaaaatgccgcaaaaaagggaataagggcgacacggaaatgttgaatactcatactcttcctttttcaatattattgaagcatttatcagggttattgtctcatgagcggatacatatttgaatgtatttagaaaaataaacaaataggggttccgcgcacatttccccgaaaagtgccacctaaattgtaagcgttaatattttgttaaaattcgcgttaaatttttgttaaatcagctcattttttaaccaataggccgaaatcggcaaaatcccttataaatcaaaagaatagaccgagatagggttgagtggccgctacagggcgctcccattcgccattcaggctgcgcaactgttgggaagggcgtttcggtgcgggcctcttcgctattacgccagctggcgaaagggggatgtgctgcaaggcgattaagttgggtaacgccagggttttcccagtcacgacgttgtaaaacgacggccagtgagcgcgacgtaatacgactcactatagggcgaattggcggaaggccgtcaaggccgcattacaggtcactaataccatctaagtagttggttcatagtgactgcatatgttgtgttttacagtattatgtagtctgttttttatgcaaaatctaatttaatatattgatatttatatcattttacgtttctcgttcaacttttttgtacaaacttgatttaaatgaattcaagcttttaattaagcatgcgagctcggcgcgccggtaccgcgat

SEQ ID NO: 65 - DNA, 9506 bp, synthetic construct
  misc_feature 1..9506: note = Vector CC006
  source 1..9506: mol_type = other DNA
ctaaattgtaagcgttaatattttgttaaaattcgcgttaaatttttgttaaatcagctcattttttaaccaataggccgaaatcggcaaaatcccttataaatcaaaagaatagaccgagatagggttgagtggccgctacagggcgctcccattcgccattcaggctgcgcaactgttgggaagggcgtttcggtgcgggcctcttcgctattacgccagctggcgaaagggggatgtgctgcaaggcgattaagttgggtaacgccagggttttcccagtcacgacgttgtaaaacgacggccagtgagcgcgacgtaatacgactcactatagggcgaattggcggaaggccgtcaaggccgcatcaaataatgattttattttgactgatagtgacctgttcgttgcaacaaattgataagcaatgctttcttataatgccaactttgtacaagaaagctgggtatttaaatgaattcaagcttttaattaatgcagtgcagcgtgacccggtcgtgcccctctctagagataatgagcattgcatgtctaagttataaaaaattaccacatattttttttgtcacacttgtttgaagtgcagtttatctatctttatacatatatttaaactttactctacgaataatataatctatagtactacaataatatcagtgttttagagaatcatataaatgaacagttagacatggtctaaaggacaattgagtattttgacaacaggactctacagttttatctttttagtgtgcatgtgttctcctttttttttgcaaatagcttcacctatataatacttcatccattttattagtacatccatttagggtttagggttaatggtttttatagactaatttttttagtacatctattttattctattttagcctctaaattaagaaaactaaaactctattttagtttttttatttaatagtttagatataaaatagaataaaataaagtgactaaaaattaaacaaataccctttaagaaattaaaaaaactaaggaaacatttttcttgtttcgagtagataatgccagcctgttaaacgccgtcgacgagtctaacggacaccaaccagcgaaccagcagcgtcgcgtcgggccaagcgaagcagacggcacggcatctctgtcgctgcctctggacccctctcgagagttccgctccaccgttggacttgctccgctgtcggcatccagaaattgcgtggcggagcggcagacgtgagccggcacggcaggcggcctcctcctcctctcacggcaccggcagctacgggggattcctttcccaccgctccttcgctttcccttcctcgcccgccgtaataaatagacaccccctccacaccctctttccccaacctcgtgttgttcggagcgcacacacacacaaccagatctcccccaaatccacccgtcggcacctccgcttcaaggtacgccgctcgtcctccccccccccccccctctctaccttctctagatcggcgttccggtccatggttagggcccggtagttctacttctgttcatgtttgtgttagatccgtgtttgtgttagatccgtgctgctagcgttcgtacacggatgcgacctgtacgtcagacacgttctgattgctaacttgccagtgtttctctttggggaatcctgggatggctctagccgttccgcagacgggatcgatttcatgattttttttgtttcgttgcatagggtttggtttgcccttttcctttatttcaatatatgccgtgcacttgtttgtcgggtcatcttttcatgcttttttttgtcttggttgtgatgatgtggtctggttgggcggtcgttctagatcggagtagaattctgtttcaaactacctggtggatttattaattttggatctgtatgtgtgtgccatacatattcatagttacgaattgaagatgatggatggaaatatcgatctaggataggtatacatgttgatgcgggttttactgatgcatatacagagatgctttttgttcgcttggttgtgatgatgtggtgtggttgggcggtcgttcattcgttctagatcggagtagaatactgtttcaaactacctggtgtatttattaattttggaactgtatgtgtgtgtcatacatcttcatagttacgagtttaagatggatggaaatatcgatctaggataggtatacatgttgatgtgggttttactgatgcatatacatgatggcatatgcagcatctattcatatgctctaaccttgagtacctatctattataataaacaagtatgttttataattatttcgatcttgatatacttggatgatggcatatgcagcagctatatgtggatttttttagccctgccttcatacgctatttatttgcttggtactgtttcttttgtcgatgctcaccctgttgtttggtgttacttctgcagggcgcgccaccatggctcctaagaagaagcggaaggttggtattcacggggtgcctgcggctgacaagaagtactccatcggcctcgacatcggcaccaacagcgtcggctgggcggtgatcaccgacgagtacaaggtcccgtccaagaagttcaaggtcctgggcaacaccgaccgccactccatcaagaagaacctcatcggcgccctcctcttcgactccggcgagacggcggaggcgacccgcctcaagcgcaccgcccgccgccgctacacccgccgcaagaaccgcatctgctacctccaggagatcttctccaacgagatggcgaaggtcgacgactccttcttccaccgcctcgaggagtccttcctcgtggaggaggacaagaagcacgagcgccaccccatcttcggcaacatcgtcgacgaggtcgcctaccacgagaagtaccccactatctaccaccttcgtaagaagcttgttgactctactgataaggctgatcttcgtctcatctaccttgctctcgctcacatgatcaagttccgtggtcacttccttatcgagggtgaccttaaccctgataactccgacgtggacaagctcttcatccagctcgtccagacctacaaccagctcttcgaggagaaccctatcaacgcttccggtgtcgacgctaaggcgatcctttccgctaggctctccaagtccaggcgtctcgagaacctcatcgcccagctccctggtgagaagaagaacggtcttttcggtaacctcatcgctctctccctcggtctgacccctaacttcaagtccaacttcgacctcgctgaggacgctaagcttcagctctccaaggatacctacgacgatgatctcgacaacctcctcgctcagattggagatcagtacgctgatctcttccttgctgctaagaacctctccgatgctatcctcctttcggatatccttagggttaacactgagatcactaaggctcctctttctgcttccatgatcaagcgctacgacgagcaccaccaggacctcaccctcctcaaggctcttgttcgtcagcagctccccgagaagtacaaggagatcttcttcgaccagtccaagaacggctacgccggttacattgacggtggagctagccaggaggagttctacaagttcatcaagccaatccttgagaagatggatggtactgaggagcttctcgttaagcttaaccgtgaggacctccttaggaagcagaggactttcgataacggctctatccctcaccagatccaccttggtgagcttcacgccatccttcgtaggcaggaggacttctaccctttcctcaaggacaaccgtgagaagatcgagaagatccttactttccgtattccttactacgttggtcctcttgctcgtggtaactcccgtttcgcttggatgactaggaagtccgaggagactatcaccccttggaacttcgaggaggttgttgacaagggtgcttccgcccagtccttcatcgagcgcatgaccaacttcgacaagaacctccccaacgagaaggtcctccccaagcactccctcctctacgagtacttcacggtctacaacgagctcaccaaggtcaagtacgtcaccgagggtatgcgcaagcctgccttcctctccggcgagcagaagaaggctatcgttgacctcctcttcaagaccaaccgcaaggtcaccgtcaagcagctcaaggaggactacttcaagaagatcgagtgcttcgactccgtcgagatcagcggcgttgaggaccgtttcaacgcttctctcggcacctaccacgatctcctcaagatcatcaaggacaaggacttcctcgacaacgaggagaacgaggacatcctcgaggacatcgtcctcactcttactctcttcgaggatagggagatgatcgaggagaggctcaagacttacgctcatctcttcgatgacaaggttatgaagcagctcaagcgtcgccgttacaccggttggggtaggctctcccgcaagctcatcaacggtatcagggataagcagagcggcaagactatcctcgacttcctcaagtctgatggtttcgctaacaggaacttcatgcagctcatccacgatgactctcttaccttcaaggaggatattcagaaggctcaggtgtccggtcagggcgactctctccacgagcacattgctaaccttgctggttcccctgctatcaagaagggcatccttcagactgttaaggttgtcgatgagcttgtcaaggttatgggtcgtcacaagcctgagaacatcgtcatcgagatggctcgtgagaaccagactacccagaagggtcagaagaactcgagggagcgcatgaagaggattgaggagggtatcaaggagcttggttctcagatccttaaggagcaccctgtcgagaacacccagctccagaacgagaagctctacctctactacctccagaacggtagggatatgtacgttgaccaggagctcgacatcaacaggctttctgactacgacgtcgaccacattgttcctcagtctttccttaaggatgactccatcgacaacaaggtcctcacgaggtccgacaagaacaggggtaagtcggacaacgtcccttccgaggaggttgtcaagaagatgaagaactactggaggcagcttctcaacgctaagctcattacccagaggaagttcgacaacctcacgaaggctgagaggggtggcctttccgagcttgacaaggctggtttcatcaagaggcagcttgttgagacgaggcagattaccaagcacgttgctcagatcctcgattctaggatgaacaccaagtacgacgagaacgacaagctcatccgcgaggtcaaggtgatcaccctcaagtccaagctcgtctccgacttccgcaaggacttccagttctacaaggtccgcgagatcaacaactaccaccacgctcacgatgcttaccttaacgctgtcgttggcaccgctcttatcaagaagtaccctaagcttgagtccgagttcgtctacggtgactacaaggtctacgacgttcgtaagatgatcgccaagtccgagcaggagatcggcaaggccaccgccaagtacttcttctactccaacatcatgaacttcttcaagaccgagatcaccctcgccaacggcgagatccgcaagcgccctcttatcgagacgaacggtgagactggtgagatcgtttgggacaagggtcgcgacttcgctactgttcgcaaggtcctttctatgcctcaggttaacatcgtcaagaagaccgaggtccagaccggtggcttctccaaggagtctatccttccaaagagaaactcggacaagctcatcgctaggaagaaggattgggaccctaagaagtacggtggtttcgactcccctactgtcgcctactccgtcctcgtggtcgccaaggtggagaagggtaagtcgaagaagctcaagtccgtcaaggagctcctcggcatcaccatcatggagcgctcctccttcgagaagaacccgatcgacttcctcgaggccaagggctacaaggaggtcaagaaggacctcatcatcaagctccccaagtactctcttttcgagctcgagaacggtcgtaagaggatgctggcttccgctggtgagctccagaagggtaacgagcttgctcttccttccaagtacgtgaacttcctctacctcgcctcccactacgagaagctcaagggttcccctgaggataacgagcagaagcagctcttcgtggagcagcacaagcactacctcgacgagatcatcgagcagatctccgagttctccaagcgcgtcatcctcgctgacgctaacctcgacaaggtcctctccgcctacaacaagcaccgcgacaagcccatccgcgagcaggccgagaacatcatccacctcttcacgctcacgaacctcggcgcccctgctgctttcaagtacttcgacaccaccatcgacaggaagcgttacacgtccaccaaggaggttctcgacgctactctcatccaccagtccatcaccggtctttacgagactcgtatcgacctttcccagcttggtggtgataagcgtcctgctgccaccaaaaaggccggacaggctaagaaaaagaagtagcctgcaggtcctgctttaatgagatatgcgagacgcctatgatcgcatgatatttgctttcaattctgttgtgcacgttgtaaaaaacctgagcatgtgtagctcagatccttaccgccggtttcggttcattctaatgaatatatcacccgttactatcgtatttttatgaataatattctccgttcaatttactgattgtaccctactacttatatgtacaatattaaaatgaaaacaatatattgtgctgaataggtttatagcgacatctatgatagagcgccacaataacaaacaattgcgttttattattacaaatccaattttaaaaaaagcggcagaaccggtcaaacctaaaagactgattacataaatcttattcaaatttcaaaagtgccccaggggctagtatctacgacacaccgagcggcgaactaataacgctcactgaagggaactccggttccccgccggcgcgcatgggtgagattccttgaagttgagtattggccgtccgctctaccgaaagttacgggcaccattcaacccggtccagcacggcggccgggtaaccgacttgctgccccgagaattatgcagcatttttttggtgtatgtgggccccaaatgaagtgcaggtcaaaccttgacagtgacgacaaatcgttgggcgggtccagggcgaattttgcgacaacatgtcgaggctcagcaggccggccgtttaaaccaactttattatacaaagttggcattataaaaaagcattgcttatcaatttgttgcaacgaacaggtcactatcagtcaaaataaaatcattatttctgggcctcatgggccttccgctcactgcccgctttccagtcgggaaacctgtcgtgccagctgcattaacatggtcatagctgtttccttgcgtattgggcgctctccgcttcctcgctcactgactcgctgcgctcggtcgttcgggtaaagcctggggtgcctaatgagcaaaaggccagcaaaaggccaggaaccgtaaaaaggccgcgttgctggcgtttttccataggctccgcccccctgacgagcatcacaaaaatcgacgctcaagtcagaggtggcgaaacccgacaggactataaagataccaggcgtttccccctggaagctccctcgtgcgctctcctgttccgaccctgccgcttaccggatacctgtccgcctttctcccttcgggaagcgtggcgctttctcatagctcacgctgtaggtatctcagttcggtgtaggtcgttcgctccaagctgggctgtgtgcacgaaccccccgttcagcccgaccgctgcgccttatccggtaactatcgtcttgagtccaacccggtaagacacgacttatcgccactggcagcagccactggtaacaggattagcagagcgaggtatgtaggcggtgctacagagttcttgaagtggtggcctaactacggctacactagaagaacagtatttggtatctgcgctctgctgaagccagttaccttcggaaaaagagttggtagctcttgatccggcaaacaaaccaccgctggtagcggtggtttttttgtttgcaagcagcagattacgcgcagaaaaaaaggatctcaagaagatcctttgatcttttctacggggtctgacgctcagtggaacgaaaactcacgttaagggattttggtcatgagattatcaaaaaggatcttcacctagatccttttaaattaaaaatgaagttttaaatcaatctaaagtatatatgagtaaacttggtctgacagttaccaatgcttaatcagtgaggcacctatctcagcgatctgtctatttcgttcatccatagttgcctgactccccgtcgtgtagataactacgatacgggagggcttaccatctggccccagtgctgcaatgataccgcgagaaccacgctcaccggctccagatttatcagcaataaaccagccagccggaagggccgagcgcagaagtggtcctgcaactttatccgcctccatccagtctattaattgttgccgggaagctagagtaagtagttcgccagttaatagtttgcgcaacgttgttgccattgctacaggcatcgtggtgtcacgctcgtcgtttggtatggcttcattcagctccggttcccaacgatcaaggcgagttacatgatcccccatgttgtgcaaaaaagcggttagctccttcggtcctccgatcgttgtcagaagtaagttggccgcagtgttatcactcatggttatggcagcactgcataattctcttactgtcatgccatccgtaagatgcttttctgtgactggtgagtactcaaccaagtcattctgagaatagtgtatgcggcgaccgagttgctcttgcccggcgtcaatacgggataataccgcgccacatagcagaactttaaaagtgctcatcattggaaaacgttcttcggggcgaaaactctcaaggatcttaccgctgttgagatccagttcgatgtaacccactcgtgcacccaactgatcttcagcatcttttactttcaccagcgtttctgggtgagcaaaaacaggaaggcaaaatgccgcaaaaaagggaataagggcgacacggaaatgttgaatactcatactcttcctttttcaatattattgaagcatttatcagggttattgtctcatgagcggatacatatttgaatgtatttagaaaaataaacaaataggggttccgcgcacatttccccgaaaagtgccac

SEQ ID NO: 66 - DNA, 17930 bp, synthetic construct
  misc_feature 1..17930: note = Vector RLW137
  source 1..17930: mol_type = other DNA
ttatacatagttgataattcactgggccggccgtttaaacttagttactaatcagtgatcagattgtcgtttcccgccttcactttaaactatcagtgtttgacaggatatattggcgggtaaacctaagagaaaagagcgtttattagaataatcggatatttaaaagggcgtgaaaaggtttatccgttcgtccatttgtatgtcaatattgggggggggggaaagccacgttgtgtctcaaaatctctgatgttacattgcacaagataaaaatatatcatcatgaacaataaaactgtctgcttacataaacagtaatacaaggggtgttcgccaccatgagccatatccagcgtgaaacctcgtgctcccgcccgcgcctcaattccaatatggatgccgacctttatggctacaagtgggcgcgcgacaacgtcggccagtcgggcgcgaccatttatcggctttatggcaaacccgatgccccggaactgttcctgaagcacggcaaaggcagcgtcgcaaacgatgtcaccgatgagatggtccgcctgaactggcttaccgagttcatgccgctgccgacgattaagcatttcatccgtaccccggacgatgcctggctcttgaccacggccattccgggcaaaacggcctttcaggtccttgaagagtacccggactccggtgagaatatcgtggacgccctcgcggtcttcctccgccgtttgcatagcatccccgtgtgcaactgccccttcaactcggaccgggttttccgcctggcacaggcccagtcgcgcatgaataacggcctcgttgacgcgagcgatttcgacgatgaacggaatggctggccggtggaacaggtttggaaggaaatgcacaaactgcttccgttctcgccggattcggtggtcacgcatggtgatttttccctggataatctgatctttgacgagggcaagctgatcggctgcatcgacgtgggtcgcgtcggtatcgccgaccgctatcaggacctggcgatcttgtggaattgcctcggcgagttctcgccctcgctccagaagcgcctgttccagaagtacggcatcgacaacccggatatgaacaagctccagttccacctcatgctggacgaatttttttgaacagaattggttaattggttgtaacactggcagagcattacgctgacttgacgggacggcggctttgttgaataaatcgaacttttgctgagttgaaggatcgatgagttgaaggaccccgtagaaaagatcaaaggatcttcttgagatcctttttttctgcgcgtaatctgctgcttgcaaacaaaaaaaccaccgctaccagcggtggtttgtttgccggatcaagagctaccaactctttttccgaaggtaactggcttcagcagagcgcagataccaaatactgtccttctagtgtagccgtagttaggccaccacttcaagaactctgtagcaccgcctacatacctcgctctgctaatcctgttaccagtggctgctgccagtggcgataagtcgtgtcttaccgggttggactcaagacgatagttaccggataaggcgcagcggtcgggctgaacggggggttcgtgcacacagcccagcttggagcgaacgacctacaccgaactgagatacctacagcgtgagctatgagaaagcgccacgcttcccgaagggagaaaggcggacaggtatccggtaagcggcagggtcggaacaggagagcgcacgagggagcttccagggggaaacgcctggtatctttatagtcctgtcgggtttcgccacctctgacttgagcgtcgatttttgtgatgctcgtcaggggggcggagcctatggaaaaacgccagcaacgcggcctttttacggttcctggccttttgctggccttttgctcacatgttctttcctgcgttatcccctgattctgtggataaccgtattaccgcctttgagtgagctgataccgctcgccgcagccgaacgaccgagcgcagcgagtcagtgagcgaggaagcggaagagcgcctgatgcggtattttctccttacgcatctgtgcggtatttcacaccgcataggccgcgataggccgacgcgaagcggcggggcgtagggagcgcagcgaccgaagggtaggcgctttttgcagctcttcggctgtgcgctggccagacagttatgcacaggccaggcgggttttaagagttttaataagttttaaagagttttaggcggaaaaatcgccttttttctcttttatatcagtcacttacatgtgtgaccggttcccaatgtacggctttgggttcccaatgtacgggttccggttcccaatgtacggctttgggttcccaatgtacgtgctatccacaggaaagagaccttttcgacctttttcccctgctagggcaatttgccctagcatctgctccgtacattaggaaccggcggatgcttcgccctcgatcaggttgcggtagcgcatgactaggatcgggccagcctgccccgcctcctccttcaaatcgtactccggcaggtcatttgacccgatcagcttgcgcacggtgaaacagaacttcttgaactctccggcgctgccactgcgttcgtagatcgtcttgaacaaccatctggcttctgccttgcctgcggcgcggcgtgccaggcggtagagaaaacggccgatgccggggtcgatcaaaaagtaatcggggtgaaccgtcagcacgtccgggttcttgccttctgtgatctcgcggtacatccaatcagcaagctcgatctcgatgtactccggccgcccggtttcgctctttacgatcttgtagcggctaatcaaggcttcaccctcggataccgtcaccaggcggccgttcttggccttcttggtacgctgcatggcaacgtgcgtggtgtttaaccgaatgcaggtttctaccaggtcgtctttctgctttccgccatcggctcgccggcagaacttgagtacgtccgcaacgtgtggacggaacacgcggccgggcttgtctcccttcccttcccggtatcggttcatggattcggttagatgggaaaccgccatcagtaccaggtcgtaatcccacacactggccatgccggcggggcctgcggaaacctctacgtgcccgtctggaagctcgtagcggatcacctcgccagctcgtcggtcacgcttcgacagacggaaaacggccacgtccatgatgctgcgactatcgcgggtgcccacgtcatagagcatcggaacgaaaaaatctggttgctcgtcgcccttgggcggcttcctaatcgacggcgcaccggctgccggcggttgccgggattctttgcggattcgatcagcggccccttgccacgattcaccggggcgtgcttctgcctcgatgcgttgccgctgggcggcctgcgcggccttcaacttctccaccaggtcatcacccagcgccgcgccgatttgtaccgggccggatggtttgcgaccgctcacgccgattcctcgggcttgggggttccagtgccattgcagggccggcagacaacccagccgcttacgcctggccaaccgcccgttcctccacacatggggcattccacggcgtcggtgcctggttgttcttgattttccatgccgcctcctttagccgctaaaattcatctactcatttattcatttgctcatttactctggtagctgcgcgatgtattcagatagcagctcggtaatggtcttgccttggcgtaccgcgtacatcttcagcttggtgtgatcctccgccggcaactgaaagttgacccgcttcatggctggcgtgtctgccaggctggccaacgttgcagccttgctgctgcgtgcgctcggacggccggcacttagcgtgtttgtgcttttgctcattttctctttacctcattaactcaaatgagttttgatttaatttcagcggccagcgcctggacctcgcgggcagcgtcgccctcgggttctgattcaagaacggttgtgccggcggcggcagtgcctgggtagctcacgcgctgcgtgatacgggactcaagaatgggcagctcgtacccggccagcgcctcggcaacctcaccgccgatgcgcgtgcctttgatcgcccgcgacacgacaaaggccgcttgtagccttccatccgtgacctcaatgcgctgcttaaccagctccaccaggtcggcggtggcccaaatgtcgtaagggcttggctgcaccggaatcagcacgaagtcggctgccttgatcgcggacacagccaagtccgccgcctggggcgctccgtcgatcactacgaagtcgcgccggccgatggccttcacgtcgcggtcaatcgtcgggcggtcgatgccgacaacggttagcggttgatcttcccgcacggccgcccaatcgcgggcactgccctggggatcggaatcgactaacagaacatcggccccggcgagttgcagggcgcgggctagatgggttgcgatggtcgtcttgcctgacccgcctttctggttaagtacagcgataaccttcatgcgttccccttgcgtatttgtttatttactcatcgcatcatatacgcagcgaccgcatgacgcaagctgttttactcaaatacacatcacctttttagatgatcagtgattttgtgccgagctgccggtcggggagctgttggctggctggtggcaggatatattgtggtgtaaacaaattgacgcttagacaacttaataacacattgcggacgtctttaatgtactgaatttagttactgatcactgattaagtactgataaatttaattaacagatctcaactttgtatagaaaagttgatttaaatgaattcaagcttttaattaacttagccactgcaacaagttcttgaaccttagcacaatcatattgtgcatgcacttgtttattgcaaagaatggtgcgtagggaacacgcatgatttttgaattgctggcacataattttatcattagaaactggaatgcaacatgtaccctttgtcatggtttctttccgagacattgcactgttttttttaatcctatcattatcataatgccaagaactggtcaccaaccagcattttgcatcatggttagttgagctgtccccatgtatcaataggtgcattgtattggtccaaaatataaatgcagtggatgcaacctatctcatggccgtcaacaaaagaaatcaaaagggaaatgcaccatcttatatctccagtttatatgaacagattggataagatcataagatcaagtggtttatattattttgaggaatataacatggattcatcctaatcactcgtctaggcagtatgtgtattcatgatggatatggtactatactacggagttttttcttcacaaaataacctgttattttgacctccaaccaaacacgaattataccaaaaattgggttatttcatctatagtacaactctattataaacatgcagtaaattatcctacacatataccaaaattcaagtgtaataatcctaatacacagacttaaaaaacaaactatttcctttttaagaaaaggaaaaccatttttttaacggaaggaaaacaaattcgggtcaaggcggaagccagcgcgccaccccacgtcagcgaatacggaggcgcggggttgacggcgtcacccggtcctaacggcgaccaacaaaccagccagaagaaattacagtaaaaaaaagtaaattgcactttgatccaccttttattacccaagtttcaatttggaccacccttaaacctatcttttcaaattgggccgggttgtggtttggactaccatgaacaacttttcgtcatgtctaacttccctttcggcaaacatatgaaccatatatagaggagatcggccgtatactagagctgatgtgtttaaggtcgttgattgcacgagaaaaaaaaaatccaaatcgcaacaatagcaaatttatctagttcaaagtgaaaagatatgtttaaaggtagtccaaagtaaaacttaggggctgtttggttcccagccatactttaccattacttgccaacaaaagttgccacaccttgtctaaggtgaggtgatcaaattgttagccacaacttactaagcctaagggaatcttgccacacttttttgagccattgacacgtgggacttaatttgttagagggaaatcttgccacaactgtggctacaaccaaacacctgtcaaatttgcctaaccttaggcgtggcaaactgtggcaaagtgtggcttacaaccaaacacacccttagataataaaatgtggtccaaagcgtaattcactaaaaaaaaatcaacgagacgtgtaccaaacggagacaaacggcatcttctcgaaatttcccaaccgctcgctcgcccgcctcgtcttcccggaaaccgcggtggtttcagcgtggcggattctccaagcagacggagacgtcacggcacgggactcctcccaccacccaaccgccataaataccagccccctcatctcctctcctcgcatcagctccacccccgaaaaatttctccccaatctcgcgaggctctcgtcgtcgaatcgaatcctctcgcgtcctcaagcttggcatccaggtacggatccgcgtcccatctccctcaccccccgtgttcttcgtgcctgcttctgggtcagatctgggtggattcgcggttgttggatgtggggggctgtgtttatttgtcggtggatctggttgtctggatctgcgttttctctgtcgtagttagcggatctgatgaaatgtttagtgttcgtgtatactggtatggtggatctggtcctaggatgcgtggaatggatatatgtaggcgaattggaggatttattttgtgaattttgctgaaatgatagttctaaacactggatctgacctcgggatgctgttaaatgtggaaatcatggtcgatgctgtcatgaacatggtgttcttatggtagatctgagcaatgtatgtttcaaaattgtttgtcacatggaaatgctatggttctagatgcaatagaatgatacatgccgagatcccctctagttgatatgatagatcatgatgttttacagctatgtcatatgaatatgttcatttgttaccgatgtatttggatctacttaacatttccaaagcacgccgcgttctaattctagatctggtagtcatgtttgtacacgtcacccacctaatacaaatacatatgtctagtgtttggtgacactgcccgtcagatctgttttttccagatctgtggaacaaatactccacgcatgtatggtagttttgaaacgatcttgtatcttccattgttgtagtaacaactaaataaagtacaattgttcaattattgggaatcgtattttctgtagtgccgatgtacagcatattcatagatgtctatttaggaactcaaattttaaattgaggactagttatttattgtgggtcagtcttttgaattgtgttatcttgctgtactggcgcgccaccatggccaccgccgccgccgcgtctaccgcgctcactggcgccactaccgctgcgcccaaggcgaggcgccgggcgcacctcctggccacccgccgcgccctcgccgcgcccatcaggtgctcagcggcgtcacccgccatgccgatggctcccccggccaccccgctccggccgtggggccccaccgatccccgcaagggcgccgacatcctcgtcgagtccctcgagcgctgcggcgtccgcgacgtcttcgcctaccccggcggcacgtccatggagatccaccaggcactcacccgctcccccgtcatcgccaaccacctcttccgccacgagcaaggggaggcctttgcggcctccggctacgcgcgctcctcgggccgcgtcggcgtctgcatcgccacctccggccccggcgccaccaaccttgtctccgcgctcgccgacgcgctgctcgattccgtccccatggtcgccatcacgggacaggtgccgcgacgcatgattggcaccgacgccttccaggagacgcccatcgtcgaggtcacccgctccatcaccaagcacaactacctggtcctcgacgtcgacgacatcccccgcgtcgtgcaggaggctttcttcctcgcctcctctggtcgaccggggccggtgcttgtcgacatccccaaggacatccagcagcagatggcggtgcctgtctgggacaagcccatgagtctgcctgggtacattgcgcgccttcccaagccccctgcgactgagttgcttgagcaggtgctgcgtcttgttggtgaatcccggcgccctgttctttatgttggcggtggctgcgcagcatctggtgaggagttgcgacgctttgtggagctgactggaatcccggtcacaactactcttatgggcctcggcaacttccccagcgacgacccactgtctctgcgcatgctaggtatgcatggcacggtgtatgcaaattatgcagtggataaggccgatctgttgcttgcacttggtgtgcggtttgatgatcgtgtgacagggaagattgaggcttttgcaagcagggctaagattgtgcacgttgatattgatccggctgagattggcaagaacaagcagccacatgtgtccatctgtgcagatgttaagcttgctttgcagggcatgaatgctcttcttgaaggaagcacatcaaagaagagctttgactttggctcatggaacgatgagttggatcagcagaagagggaattcccccttgggtataaaacatctaatgaggagatccagccacaatatgctattcaggttcttgatgagctgacgaaaggcgaggccatcatcggcacaggtgttgggcagcaccagatgtgggcggcacagtactacacttacaagcggccaaggcagtggttgtcttcagctggtcttggggctatgggatttggtttgccggctgctgctggtgcttctgtggccaacccaggtgttactgttgttgacatcgatggagatggtagctttctcatgaacgttcaggagctagctatgatccgaattgagaacctcccggtgaaggtctttgtgctaaacaaccagcacctggggatggtggtgcagtgggaggacaggttctataaggccaacagagcgcacacatacttgggaaacccagagaatgaaagtgagatatatccagatttcgtgacgatcgccaaagggttcaacattccagcggtccgtgtgacaaagaagaacgaagtccgcgcagcgataaagaagatgctcgagactccagggccgtacctcttggatataatcgtcccacaccaggagcatgtgttgcctatgatccctaatggtggggctttcaaggatatgatcctggatggtgatggcaggactgtgtactagcctgcaggcctaggatcgttcaaacatttggcaataaagtttcttaagattgaatcctgttgccggtcttgcgatgattatcatataatttctgttgaattacgttaagcatgtaataattaacatgtaatgcatgacgttatttatgagatgggtttttatgattagagtcccgcaattatacatttaatacgcgatagaaaacaaaatatagcgcgcaaactaggataaattatcgcgcgcggtgtcatctatgttactagatcggccggccgtttaaacagcctgcttttttgtacaaacttgatttaaatgaattcaagcttttaattaagcatgcgagctcggcgcgccggtaccgcgatcgcggatcatgaaccaacggcctggctgtatttggtggttgtgtagggagatggggagaagaaaagcccgattctcttcgctgtgatgggctggatgcatgcgggggagcgggaggcccaagtacgtgcacggtgagcggcccacagggcgagtgtgagcgcgagaggcgggaggaacagtttagtaccacattgcccagctaactcgaacgcgaccaacttataaacccgcgcgctgtcgcttgtgtgcattgagtgctatgctgaggttttagagctagaaatagcaagttaaaataaggctagtccgttatcaacttgaaaaagtggcaccgagtcggtgctctgttcctcgtgctggacaagtgtggtttccagattctgcaaccaagactgcgcaggcattgctggacttcaaccgtgaaggattacctctgttcatcctcgctaactggagaggcttctctggtggacaaagagatctctttgaaggaattcttcaggctggctcgactattgttgagaaccttaggacatacaatcagcctgcctttgtctacattcccatggctgcagagctacgaggaggggcttgggttgtggttgatagcaagataaacccagaccgcattgagtgctatgctgagagaactgcaaaatccaatgttctggaaccgcaagggttaattgagatcaagttcaggtcagaggaactccaggattgcatgagtcggcttgacccaacattaattgatctgaaagcaaaactcgaagtagcaaataaaaatggaagtgctgacacaaaatcgcttcaagaaaatatagaagctcgaacaaaacagttgatgcctctatatactcagattgcgatacggtttgctgaattgcatgatacatccctcagaatggctgcgaaaggtgtgattaagaaagttgtggactgggaagaatcacgatctttcttttttttgcggccgccccgggcctgcaggggatcccgatcgggccggccgtttaaacccactttgtacaagaaagctgggtatttaaatgaattcaagcttttaattaatgcagtgcagcgtgacccggtcgtgcccctctctagagataatgagcattgcatgtctaagttataaaaaattaccacatattttttttgtcacacttgtttgaagtgcagtttatctatctttatacatatatttaaactttactctacgaataatataatctatagtactacaataatatcagtgttttagagaatcatataaatgaacagttagacatggtctaaaggacaattgagtattttgacaacaggactctacagttttatctttttagtgtgcatgtgttctcctttttttttgcaaatagcttcacctatataatacttcatccattttattagtacatccatttagggtttagggttaatggtttttatagactaatttttttagtacatctattttattctattttagcctctaaattaagaaaactaaaactctattttagtttttttatttaatagtttagatataaaatagaataaaataaagtgactaaaaattaaacaaataccctttaagaaattaaaaaaactaaggaaacatttttcttgtttcgagtagataatgccagcctgttaaacgccgtcgacgagtctaacggacaccaaccagcgaaccagcagcgtcgcgtcgggccaagcgaagcagacggcacggcatctctgtcgctgcctctggacccctctcgagagttccgctccaccgttggacttgctccgctgtcggcatccagaaattgcgtggcggagcggcagacgtgagccggcacggcaggcggcctcctcctcctctcacggcaccggcagctacgggggattcctttcccaccgctccttcgctttcccttcctcgcccgccgtaataaatagacaccccctccacaccctctttccccaacctcgtgttgttcggagcgcacacacacacaaccagatctcccccaaatccacccgtcggcacctccgcttcaaggtacgccgctcgtcctccccccccccccccctctctaccttctctagatcggcgttccggtccatggttagggcccggtagttctacttctgttcatgtttgtgttagatccgtgtttgtgttagatccgtgctgctagcgttcgtacacggatgcgacctgtacgtcagacacgttctgattgctaacttgccagtgtttctctttggggaatcctgggatggctctagccgttccgcagacgggatcgatttcatgattttttttgtttcgttgcatagggtttggtttgcccttttcctttatttcaatatatgccgtgcacttgtttgtcgggtcatcttttcatgcttttttttgtcttggttgtgatgatgtggtctggttgggcggtcgttctagatcggagtagaattctgtttcaaactacctggtggatttattaattttggatctgtatgtgtgtgccatacatattcatagttacgaattgaagatgatggatggaaatatcgatctaggataggtatacatgttgatgcgggttttactgatgcatatacagagatgctttttgttcgcttggttgtgatgatgtggtgtggttgggcggtcgttcattcgttctagatcggagtagaatactgtttcaaactacctggtgtatttattaattttggaactgtatgtgtgtgtcatacatcttcatagttacgagtttaagatggatggaaatatcgatctaggataggtatacatgttgatgtgggttttactgatgcatatacatgatggcatatgcagcatctattcatatgctctaaccttgagtacctatctattataataaacaagtatgttttataattatttcgatcttgatatacttggatgatggcatatgcagcagctatatgtggatttttttagccctgccttcatacgctatttatttgcttggtactgtttcttttgtcgatgctcaccctgttgtttggtgttacttctgcagggcgcgccaccatggctcctaagaagaagcggaaggttggtattcacggggtgcctgcggctgacaagaagtactccatcggcctcgacatcggcaccaacagcgtcggctgggcggtgatcaccgacgagtacaaggtcccgtccaagaagttcaaggtcctgggcaacaccgaccgccactccatcaagaagaacctcatcggcgccctcctcttcgactccggcgagacggcggaggcgacccgcctcaagcgcaccgcccgccgccgctacacccgccgcaagaaccgcatctgctacctccaggagatcttctccaacgagatggcgaaggtcgacgactccttcttccaccgcctcgaggagtccttcctcgtggaggaggacaagaagcacgagcgccaccccatcttcggcaacatcgtcgacgaggtcgcctaccacgagaagtaccccactatctaccaccttcgtaagaagcttgttgactctactgataaggctgatcttcgtctcatctaccttgctctcgctcacatgatcaagttccgtggtcacttccttatcgagggtgaccttaaccctgataactccgacgtggacaagctcttcatccagctcgtccagacctacaaccagctcttcgaggagaaccctatcaacgcttccggtgtcgacgctaaggcgatcctttccgctaggctctccaagtccaggcgtctcgagaacctcatcgcccagctccctggtgagaagaagaacggtcttttcggtaacctcatcgctctctccctcggtctgacccctaacttcaagtccaacttcgacctcgctgaggacgctaagcttcagctctccaaggatacctacgacgatgatctcgacaacctcctcgctcagattggagatcagtacgctgatctcttccttgctgctaagaacctctccgatgctatcctcctttcggatatccttagggttaacactgagatcactaaggctcctctttctgcttccatgatcaagcgctacgacgagcaccaccaggacctcaccctcctcaaggctcttgttcgtcagcagctccccgagaagtacaaggagatcttcttcgaccagtccaagaacggctacgccggttacattgacggtggagctagccaggaggagttctacaagttcatcaagccaatccttgagaagatggatggtactgaggagcttctcgttaagcttaaccgtgaggacctccttaggaagcagaggactttcgataacggctctatccctcaccagatccaccttggtgagcttcacgccatccttcgtaggcaggaggacttctaccctttcctcaaggacaaccgtgagaagatcgagaagatccttactttccgtattccttactacgttggtcctcttgctcgtggtaactcccgtttcgcttggatgactaggaagtccgaggagactatcaccccttggaacttcgaggaggttgttgacaagggtgcttccgcccagtccttcatcgagcgcatgaccaacttcgacaagaacctccccaacgagaaggtcctccccaagcactccctcctctacgagtacttcacggtctacaacgagctcaccaaggtcaagtacgtcaccgagggtatgcgcaagcctgccttcctctccggcgagcagaagaaggctatcgttgacctcctcttcaagaccaaccgcaaggtcaccgtcaagcagctcaaggaggactacttcaagaagatcgagtgcttcgactccgtcgagatcagcggcgttgaggaccgtttcaacgcttctctcggcacctaccacgatctcctcaagatcatcaaggacaaggacttcctcgacaacgaggagaacgaggacatcctcgaggacatcgtcctcactcttactctcttcgaggatagggagatgatcgaggagaggctcaagacttacgctcatctcttcgatgacaaggttatgaagcagctcaagcgtcgccgttacaccggttggggtaggctctcccgcaagctcatcaacggtatcagggataagcagagcggcaagactatcctcgacttcctcaagtctgatggtttcgctaacaggaacttcatgcagctcatccacgatgactctcttaccttcaaggaggatattcagaaggctcaggtgtccggtcagggcgactctctccacgagcacattgctaaccttgctggttcccctgctatcaagaagggcatccttcagactgttaaggttgtcgatgagcttgtcaaggttatgggtcgtcacaagcctgagaacatcgtcatcgagatggctcgtgagaaccagactacccagaagggtcagaagaactcgagggagcgcatgaagaggattgaggagggtatcaaggagcttggttctcagatccttaaggagcaccctgtcgagaacacccagctccagaacgagaagctctacctctactacctccagaacggtagggatatgtacgttgaccaggagctcgacatcaacaggctttctgactacgacgtcgaccacattgttcctcagtctttccttaaggatgactccatcgacaacaaggtcctcacgaggtccgacaagaacaggggtaagtcggacaacgtcccttccgaggaggttgtcaagaagatgaagaactactggaggcagcttctcaacgctaagctcattacccagaggaagttcgacaacctcacgaaggctgagaggggtggcctttccgagcttgacaaggctggtttcatcaagaggcagcttgttgagacgaggcagattaccaagcacgttgctcagatcctcgattctaggatgaacaccaagtacgacgagaacgacaagctcatccgcgaggtcaaggtgatcaccctcaagtccaagctcgtctccgacttccgcaaggacttccagttctacaaggtccgcgagatcaacaactaccaccacgctcacgatgcttaccttaacgctgtcgttggcaccgctcttatcaagaagtaccctaagcttgagtccgagttcgtctacggtgactacaaggtctacgacgttcgtaagatgatcgccaagtccgagcaggagatcggcaaggccaccgccaagtacttcttctactccaacatcatgaacttcttcaagaccgagatcaccctcgccaacggcgagatccgcaagcgccctcttatcgagacgaacggtgagactggtgagatcgtttgggacaagggtcgcgacttcgctactgttcgcaaggtcctttctatgcctcaggttaacatcgtcaagaagaccgaggtccagaccggtggcttctccaaggagtctatccttccaaagagaaactcggacaagctcatcgctaggaagaaggattgggaccctaagaagtacggtggtttcgactcccctactgtcgcctactccgtcctcgtggtcgccaaggtggagaagggtaagtcgaagaagctcaagtccgtcaaggagctcctcggcatcaccatcatggagcgctcctccttcgagaagaacccgatcgacttcctcgaggccaagggctacaaggaggtcaagaaggacctcatcatcaagctccccaagtactctcttttcgagctcgagaacggtcgtaagaggatgctggcttccgctggtgagctccagaagggtaacgagcttgctcttccttccaagtacgtgaacttcctctacctcgcctcccactacgagaagctcaagggttcccctgaggataacgagcagaagcagctcttcgtggagcagcacaagcactacctcgacgagatcatcgagcagatctccgagttctccaagcgcgtcatcctcgctgacgctaacctcgacaaggtcctctccgcctacaacaagcaccgcgacaagcccatccgcgagcaggccgagaacatcatccacctcttcacgctcacgaacctcggcgcccctgctgctttcaagtacttcgacaccaccatcgacaggaagcgttacacgtccaccaaggaggttctcgacgctactctcatccaccagtccatcaccggtctttacgagactcgtatcgacctttcccagcttggtggtgataagcgtcctgctgccaccaaaaaggccggacaggctaagaaaaagaagtagcctgcaggtcctgctttaatgagatatgcgagacgcctatgatcgcatgatatttgctttcaattctgttgtgcacgttgtaaaaaacctgagcatgtgtagctcagatccttaccgccggtttcggttcattctaatgaatatatcacccgttactatcgtatttttatgaataatattctccgttcaatttactgattgtaccctactacttatatgtacaatattaaaatgaaaacaatatattgtgctgaataggtttatagcgacatctatgatagagcgccacaataacaaacaattgcgttttattattacaaatccaattttaaaaaaagcggcagaaccggtcaaacctaaaagactgattacataaatcttattcaaatttcaaaagtgccccaggggctagtatctacgacacaccgagcggcgaactaataacgctcactgaagggaactccggttccccgccggcgcgcatgggtgagattccttgaagttgagtattggccgtccgctctaccgaaagttacgggcaccattcaacccggtccagcacggcggccgggtaaccgacttgctgccccgagaattatgcagcatttttttggtgtatgtgggccccaaatgaagtgcaggtcaaaccttgacagtgacgacaaatcgttgggcgggtccagggcgaattttgcgacaacatgtcgaggctcagcaggccggccgtttaaaccaacttta

SEQ ID NO: 67 - DNA, 3734 bp, synthetic construct
  misc_feature 1..3734: note = Vector CC019
  source 1..3734: mol_type = other DNA
cgcggatcatgaaccaacggcctggctgtatttggtggttgtgtagggagatggggagaagaaaagcccgattctcttcgctgtgatgggctggatgcatgcgggggagcgggaggcccaagtacgtgcacggtgagcggcccacagggcgagtgtgagcgcgagaggcgggaggaacagtttagtaccacattgcccagctaactcgaacgcgaccaacttataaacccgcgcgctgtcgcttgtgtgactgcaaaaggcaatgttcgttttagagctagaaatagcaagttaaaataaggctagtccgttatcaacttgaaaaagtggcaccgagtcggtgctctgttcctcgtgctggacaagtgtggtttccagattctgcaaccaagactgcgcaggcattgctggacttcaaccgtgaaggattacctctgttcatcctcgctaactggagaggcttctctggtggacaaagagatctctttgaaggaattcttcaggctggctcgactattgttgagaaccttaggacatacaatcagcctgcctttgtctacattcccatggctgcagagctacgaggaggggcttgggttgtggttgatagcaagataaacccagaccgcattgagtgctatgctgagaggactgcaaaatccaatgttctcgaaccgcaagggttaattgagatcaagttcaggtcagaggaactccaggattgcatgagtcggcttgacccaacattaattgatctgaaagcaaaactcgaagtagcaaataaaaatggaagtgctgacacaaaatcgcttcaagaaaatatagaagctcgaacaaaacagttgatgcctctatatactcagattgcgatacggtttgctgaattgcatgatacatccctcagaatggctgcgaaaggtgtgattaagaaagttgtggactgggaagaatcacgatctttcttttttttgcggccgccccgggcctgcaggggatcccgatcgggccggccgtttaaacccactttgtacaagaaagttgaacgagaaacgtaaaatgatataaatatcaatatattaaattagattttgcataaaaaacagactacataatactgtaaaacacaacatatgcagtcactatgaaccaactacttagatggtattagtgacctgtactgggcctcatgggccttccgctcactgcccgctttccagtcgggaaacctgtcgtgccagctgcattaacatggtcatagctgtttccttgcgtattgggcgctctccgcttcctcgctcactgactcgctgcgctcggtcgttcgggtaaagcctggggtgcctaatgagcaaaaggccagcaaaaggccaggaaccgtaaaaaggccgcgttgctggcgtttttccataggctccgcccccctgacgagcatcacaaaaatcgacgctcaagtcagaggtggcgaaacccgacaggactataaagataccaggcgtttccccctggaagctccctcgtgcgctctcctgttccgaccctgccgcttaccggatacctgtccgcctttctcccttcgggaagcgtggcgctttctcatagctcacgctgtaggtatctcagttcggtgtaggtcgttcgctccaagctgggctgtgtgcacgaaccccccgttcagcccgaccgctgcgccttatccggtaactatcgtcttgagtccaacccggtaagacacgacttatcgccactggcagcagccactggtaacaggattagcagagcgaggtatgtaggcggtgctacagagttcttgaagtggtggcctaactacggctacactagaagaacagtatttggtatctgcgctctgctgaagccagttaccttcggaaaaagagttggtagctcttgatccggcaaacaaaccaccgctggtagcggtggtttttttgtttgcaagcagcagattacgcgcagaaaaaaaggatctcaagaagatcctttgatcttttctacggggtctgacgctcagtggaacgaaaactcacgttaagggattttggtcatgagattatcaaaaaggatcttcacctagatccttttaaattaaaaatgaagttttaaatcaatctaaagtatatatgagtaaacttggtctgacagttaccaatgcttaatcagtgaggcacctatctcagcgatctgtctatttcgttcatccatagttgcctgactccccgtcgtgtagataactacgatacgggagggcttaccatctggccccagtgctgcaatgataccgcgagaaccacgctcaccggctccagatttatcagcaataaaccagccagccggaagggccgagcgcagaagtggtcctgcaactttatccgcctccatccagtctattaattgttgccgggaagctagagtaagtagttcgccagttaatagtttgcgcaacgttgttgccattgctacaggcatcgtggtgtcacgctcgtcgtttggtatggcttcattcagctccggttcccaacgatcaaggcgagttacatgatcccccatgttgtgcaaaaaagcggttagctccttcggtcctccgatcgttgtcagaagtaagttggccgcagtgttatcactcatggttatggcagcactgcataattctcttactgtcatgccatccgtaagatgcttttctgtgactggtgagtactcaaccaagtcattctgagaatagtgtatgcggcgaccgagttgctcttgcccggcgtcaatacgggataataccgcgccacatagcagaactttaaaagtgctcatcattggaaaacgttcttcggggcgaaaactctcaaggatcttaccgctgttgagatccagttcgatgtaacccactcgtgcacccaactgatcttcagcatcttttactttcaccagcgtttctgggtgagcaaaaacaggaaggcaaaatgccgcaaaaaagggaataagggcgacacggaaatgttgaatactcatactcttcctttttcaatattattgaagcatttatcagggttattgtctcatgagcggatacatatttgaatgtatttagaaaaataaacaaataggggttccgcgcacatttccccgaaaagtgccacctaaattgtaagcgttaatattttgttaaaattcgcgttaaatttttgttaaatcagctcattttttaaccaataggccgaaatcggcaaaatcccttataaatcaaaagaatagaccgagatagggttgagtggccgctacagggcgctcccattcgccattcaggctgcgcaactgttgggaagggcgtttcggtgcgggcctcttcgctattacgccagctggcgaaagggggatgtgctgcaaggcgattaagttgggtaacgccagggttttcccagtcacgacgttgtaaaacgacggccagtgagcgcgacgtaatacgactcactatagggcgaattggcggaaggccgtcaaggccgcattacaggtcactaataccatctaagtagttggttcatagtgactgcatatgttgtgttttacagtattatgtagtctgttttttatgcaaaatctaatttaatatattgatatttatatcattttacgtttctcgttcaacttttttgtacaaacttgatttaaatgaattcaagcttttaattaagcatgcgagctcggcgcgccggtaccgcgat

SEQ ID NO: 68 - DNA, 17930 bp, synthetic construct
  misc_feature 1..17930: note = Vector RLW138
  source 1..17930: mol_type = other DNA
ttatacatagttgataattcactgggccggccgtttaaacttagttactaatcagtgatcagattgtcgtttcccgccttcactttaaactatcagtgtttgacaggatatattggcgggtaaacctaagagaaaagagcgtttattagaataatcggatatttaaaagggcgtgaaaaggtttatccgttcgtccatttgtatgtcaatattgggggggggggaaagccacgttgtgtctcaaaatctctgatgttacattgcacaagataaaaatatatcatcatgaacaataaaactgtctgcttacataaacagtaatacaaggggtgttcgccaccatgagccatatccagcgtgaaacctcgtgctcccgcccgcgcctcaattccaatatggatgccgacctttatggctacaagtgggcgcgcgacaacgtcggccagtcgggcgcgaccatttatcggctttatggcaaacccgatgccccggaactgttcctgaagcacggcaaaggcagcgtcgcaaacgatgtcaccgatgagatggtccgcctgaactggcttaccgagttcatgccgctgccgacgattaagcatttcatccgtaccccggacgatgcctggctcttgaccacggccattccgggcaaaacggcctttcaggtccttgaagagtacccggactccggtgagaatatcgtggacgccctcgcggtcttcctccgccgtttgcatagcatccccgtgtgcaactgccccttcaactcggaccgggttttccgcctggcacaggcccagtcgcgcatgaataacggcctcgttgacgcgagcgatttcgacgatgaacggaatggctggccggtggaacaggtttggaaggaaatgcacaaactgcttccgttctcgccggattcggtggtcacgcatggtgatttttccctggataatctgatctttgacgagggcaagctgatcggctgcatcgacgtgggtcgcgtcggtatcgccgaccgctatcaggacctggcgatcttgtggaattgcctcggcgagttctcgccctcgctccagaagcgcctgttccagaagtacggcatcgacaacccggatatgaacaagctccagttccacctcatgctggacgaatttttttgaacagaattggttaattggttgtaacactggcagagcattacgctgacttgacgggacggcggctttgttgaataaatcgaacttttgctgagttgaaggatcgatgagttgaaggaccccgtagaaaagatcaaaggatcttcttgagatcctttttttctgcgcgtaatctgctgcttgcaaacaaaaaaaccaccgctaccagcggtggtttgtttgccggatcaagagctaccaactctttttccgaaggtaactggcttcagcagagcgcagataccaaatactgtccttctagtgtagccgtagttaggccaccacttcaagaactctgtagcaccgcctacatacctcgctctgctaatcctgttaccagtggctgctgccagtggcgataagtcgtgtcttaccgggttggactcaagacgatagttaccggataaggcgcagcggtcgggctgaacggggggttcgtgcacacagcccagcttggagcgaacgacctacaccgaactgagatacctacagcgtgagctatgagaaagcgccacgcttcccgaagggagaaaggcggacaggtatccggtaagcggcagggtcggaacaggagagcgcacgagggagcttccagggggaaacgcctggtatctttatagtcctgtcgggtttcgccacctctgacttgagcgtcgatttttgtgatgctcgtcaggggggcggagcctatggaaaaacgccagcaacgcggcctttttacggttcctggccttttgctggccttttgctcacatgttctttcctgcgttatcccctgattctgtggataaccgtattaccgcctttgagtgagctgataccgctcgccgcagccgaacgaccgagcgcagcgagtcagtgagcgaggaagcggaagagcgcctgatgcggtattttctccttacgcatctgtgcggtatttcacaccgcataggccgcgataggccgacgcgaagcggcggggcgtagggagcgcagcgaccgaagggtaggcgctttttgcagctcttcggctgtgcgctggccagacagttatgcacaggccaggcgggttttaagagttttaataagttttaaagagttttaggcggaaaaatcgccttttttctcttttatatcagtcacttacatgtgtgaccggttcccaatgtacggctttgggttcccaatgtacgggttccggttcccaatgtacggctttgggttcccaatgtacgtgctatccacaggaaagagaccttttcgacctttttcccctgctagggcaatttgccctagcatctgctccgtacattaggaaccggcggatgcttcgccctcgatcaggttgcggtagcgcatgactaggatcgggccagcctgccccgcctcctccttcaaatcgtactccggcaggtcatttgacccgatcagcttgcgcacggtgaaacagaacttcttgaactctccggcgctgccactgcgttcgtagatcgtcttgaacaaccatctggcttctgccttgcctgcggcgcggcgtgccaggcggtagagaaaacggccgatgccggggtcgatcaaaaagtaatcggggtgaaccgtcagcacgtccgggttcttgccttctgtgatctcgcggtacatccaatcagcaagctcgatctcgatgtactccggccgcccggtttcgctctttacgatcttgtagcggctaatcaaggcttcaccctcggataccgtcaccaggcggccgttcttggccttcttggtacgctgcatggcaacgtgcgtggtgtttaaccgaatgcaggtttctaccaggtcgtctttctgctttccgccatcggctcgccggcagaacttgagtacgtccgcaacgtgtggacggaacacgcggccgggcttgtctcccttcccttcccggtatcggttcatggattcggttagatgggaaaccgccatcagtaccaggtcgtaatcccacacactggccatgccggcggggcctgcggaaacctctacgtgcccgtctggaagctcgtagcggatcacctcgccagctcgtcggtcacgcttcgacagacggaaaacggccacgtccatgatgctgcgactatcgcgggtgcccacgtcatagagcatcggaacgaaaaaatctggttgctcgtcgcccttgggcggcttcctaatcgacggcgcaccggctgccggcggttgccgggattctttgcggattcgatcagcggccccttgccacgattcaccggggcgtgcttctgcctcgatgcgttgccgctgggcggcctgcgcggccttcaacttctccaccaggtcatcacccagcgccgcgccgatttgtaccgggccggatggtttgcgaccgctcacgccgattcctcgggcttgggggttccagtgccattgcagggccggcagacaacccagccgcttacgcctggccaaccgcccgttcctccacacatggggcattccacggcgtcggtgcctggttgttcttgattttccatgccgcctcctttagccgctaaaattcatctactcatttattcatttgctcatttactctggtagctgcgcgatgtattcagatagcagctcggtaatggtcttgccttggcgtaccgcgtacatcttcagcttggtgtgatcctccgccggcaactgaaagttgacccgcttcatggctggcgtgtctgccaggctggccaacgttgcagccttgctgctgcgtgcgctcggacggccggcacttagcgtgtttgtgcttttgctcattttctctttacctcattaactcaaatgagttttgatttaatttcagcggccagcgcctggacctcgcgggcagcgtcgccctcgggttctgattcaagaacggttgtgccggcggcggcagtgcctgggtagctcacgcgctgcgtgatacgggactcaagaatgggcagctcgtacccggccagcgcctcggcaacctcaccgccgatgcgcgtgcctttgatcgcccgcgacacgacaaaggccgcttgtagccttccatccgtgacctcaatgcgctgcttaaccagctccaccaggtcggcggtggcccaaatgtcgtaagggcttggctgcaccggaatcagcacgaagtcggctgccttgatcgcggacacagccaagtccgccgcctggggcgctccgtcgatcactacgaagtcgcgccggccgatggccttcacgtcgcggtcaatcgtcgggcggtcgatgccgacaacggttagcggttgatcttcccgcacggccgcccaatcgcgggcactgccctggggatcggaatcgactaacagaacatcggccccggcgagttgcagggcgcgggctagatgggttgcgatggtcgtcttgcctgacccgcctttctggttaagtacagcgataaccttcatgcgttccccttgcgtatttgtttatttactcatcgcatcatatacgcagcgaccgcatgacgcaagctgttttactcaaatacacatcacctttttagatgatcagtgattttgtgccgagctgccggtcggggagctgttggctggctggtggcaggatatattgtggtgtaaacaaattgacgcttagacaacttaataacacattgcggacgtctttaatgtactgaatttagttactgatcactgattaagtactgataaatttaattaacagatctcaactttgtatagaaaagttgatttaaatgaattcaagcttttaattaacttagccactgcaacaagttcttgaaccttagcacaatcatattgtgcatgcacttgtttattgcaaagaatggtgcgtagggaacacgcatgatttttgaattgctggcacataattttatcattagaaactggaatgcaacatgtaccctttgtcatggtttctttccgagacattgcactgttttttttaatcctatcattatcataatgccaagaactggtcaccaaccagcattttgcatcatggttagttgagctgtccccatgtatcaataggtgcattgtattggtccaaaatataaatgcagtggatgcaacctatctcatggccgtcaacaaaagaaatcaaaagggaaatgcaccatcttatatctccagtttatatgaacagattggataagatcataagatcaagtggtttatattattttgaggaatataacatggattcatcctaatcactcgtctaggcagtatgtgtattcatgatggatatggtactatactacggagttttttcttcacaaaataacctgttattttgacctccaaccaaacacgaattataccaaaaattgggttatttcatctatagtacaactctattataaacatgcagtaaattatcctacacatataccaaaattcaagtgtaataatcctaatacacagacttaaaaaacaaactatttcctttttaagaaaaggaaaaccatttttttaacggaaggaaaacaaattcgggtcaaggcggaagccagcgcgccaccccacgtcagcgaatacggaggcgcggggttgacggcgtcacccggtcctaacggcgaccaacaaaccagccagaagaaattacagtaaaaaaaagtaaattgcactttgatccaccttttattacccaagtttcaatttggaccacccttaaacctatcttttcaaattgggccgggttgtggtttggactaccatgaacaacttttcgtcatgtctaacttccctttcggcaaacatatgaaccatatatagaggagatcggccgtatactagagctgatgtgtttaaggtcgttgattgcacgagaaaaaaaaaatccaaatcgcaacaatagcaaatttatctagttcaaagtgaaaagatatgtttaaaggtagtccaaagtaaaacttaggggctgtttggttcccagccatactttaccattacttgccaacaaaagttgccacaccttgtctaaggtgaggtgatcaaattgttagccacaacttactaagcctaagggaatcttgccacacttttttgagccattgacacgtgggacttaatttgttagagggaaatcttgccacaactgtggctacaaccaaacacctgtcaaatttgcctaaccttaggcgtggcaaactgtggcaaagtgtggcttacaaccaaacacacccttagataataaaatgtggtccaaagcgtaattcactaaaaaaaaatcaacgagacgtgtaccaaacggagacaaacggcatcttctcgaaatttcccaaccgctcgctcgcccgcctcgtcttcccggaaaccgcggtggtttcagcgtggcggattctccaagcagacggagacgtcacggcacgggactcctcccaccacccaaccgccataaataccagccccctcatctcctctcctcgcatcagctccacccccgaaaaatttctccccaatctcgcgaggctctcgtcgtcgaatcgaatcctctcgcgtcctcaagcttggcatccaggtacggatccgcgtcccatctccctcaccccccgtgttcttcgtgcctgcttctgggtcagatctgggtggattcgcggttgttggatgtggggggctgtgtttatttgtcggtggatctggttgtctggatctgcgttttctctgtcgtagttagcggatctgatgaaatgtttagtgttcgtgtatactggtatggtggatctggtcctaggatgcgtggaatggatatatgtaggcgaattggaggatttattttgtgaattttgctgaaatgatagttctaaacactggatctgacctcgggatgctgttaaatgtggaaatcatggtcgatgctgtcatgaacatggtgttcttatggtagatctgagcaatgtatgtttcaaaattgtttgtcacatggaaatgctatggttctagatgcaatagaatgatacatgccgagatcccctctagttgatatgatagatcatgatgttttacagctatgtcatatgaatatgttcatttgttaccgatgtatttggatctacttaacatttccaaagcacgccgcgttctaattctagatctggtagtcatgtttgtacacgtcacccacctaatacaaatacatatgtctagtgtttggtgacactgcccgtcagatctgttttttccagatctgtggaacaaatactccacgcatgtatggtagttttgaaacgatcttgtatcttccattgttgtagtaacaactaaataaagtacaattgttcaattattgggaatcgtattttctgtagtgccgatgtacagcatattcatagatgtctatttaggaactcaaattttaaattgaggactagttatttattgtgggtcagtcttttgaattgtgttatcttgctgtactggcgcgccaccatggccaccgccgccgccgcgtctaccgcgctcactggcgccactaccgctgcgcccaaggcgaggcgccgggcgcacctcctggccacccgccgcgccctcgccgcgcccatcaggtgctcagcggcgtcacccgccatgccgatggctcccccggccaccccgctccggccgtggggccccaccgatccccgcaagggcgccgacatcctcgtcgagtccctcgagcgctgcggcgtccgcgacgtcttcgcctaccccggcggcacgtccatggagatccaccaggcactcacccgctcccccgtcatcgccaaccacctcttccgccacgagcaaggggaggcctttgcggcctccggctacgcgcgctcctcgggccgcgtcggcgtctgcatcgccacctccggccccggcgccaccaaccttgtctccgcgctcgccgacgcgctgctcgattccgtccccatggtcgccatcacgggacaggtgccgcgacgcatgattggcaccgacgccttccaggagacgcccatcgtcgaggtcacccgctccatcaccaagcacaactacctggtcctcgacgtcgacgacatcccccgcgtcgtgcaggaggctttcttcctcgcctcctctggtcgaccggggccggtgcttgtcgacatccccaaggacatccagcagcagatggcggtgcctgtctgggacaagcccatgagtctgcctgggtacattgcgcgccttcccaagccccctgcgactgagttgcttgagcaggtgctgcgtcttgttggtgaatcccggcgccctgttctttatgttggcggtggctgcgcagcatctggtgaggagttgcgacgctttgtggagctgactggaatcccggtcacaactactcttatgggcctcggcaacttccccagcgacgacccactgtctctgcgcatgctaggtatgcatggcacggtgtatgcaaattatgcagtggataaggccgatctgttgcttgcacttggtgtgcggtttgatgatcgtgtgacagggaagattgaggcttttgcaagcagggctaagattgtgcacgttgatattgatccggctgagattggcaagaacaagcagccacatgtgtccatctgtgcagatgttaagcttgctttgcagggcatgaatgctcttcttgaaggaagcacatcaaagaagagctttgactttggctcatggaacgatgagttggatcagcagaagagggaattcccccttgggtataaaacatctaatgaggagatccagccacaatatgctattcaggttcttgatgagctgacgaaaggcgaggccatcatcggcacaggtgttgggcagcaccagatgtgggcggcacagtactacacttacaagcggccaaggcagtggttgtcttcagctggtcttggggctatgggatttggtttgccggctgctgctggtgcttctgtggccaacccaggtgttactgttgttgacatcgatggagatggtagctttctcatgaacgttcaggagctagctatgatccgaattgagaacctcccggtgaaggtctttgtgctaaacaaccagcacctggggatggtggtgcagtgggaggacaggttctataaggccaacagagcgcacacatacttgggaaacccagagaatgaaagtgagatatatccagatttcgtgacgatcgccaaagggttcaacattccagcggtccgtgtgacaaagaagaacgaagtccgcgcagcgataaagaagatgctcgagactccagggccgtacctcttggatataatcgtcccacaccaggagcatgtgttgcctatgatccctaatggtggggctttcaaggatatgatcctggatggtgatggcaggactgtgtactagcctgcaggcctaggatcgttcaaacatttggcaataaagtttcttaagattgaatcctgttgccggtcttgcgatgattatcatataatttctgttgaattacgttaagcatgtaataattaacatgtaatgcatgacgttatttatgagatgggtttttatgattagagtcccgcaattatacatttaatacgcgatagaaaacaaaatatagcgcgcaaactaggataaattatcgcgcgcggtgtcatctatgttactagatcggccggccgtttaaacagcctgcttttttgtacaaacttgatttaaatgaattcaagcttttaattaagcatgcgagctcggcgcgccggtaccgcgatcgcggatcatgaaccaacggcctggctgtatttggtggttgtgtagggagatggggagaagaaaagcccgattctcttcgctgtgatgggctggatgcatgcgggggagcgggaggcccaagtacgtgcacggtgagcggcccacagggcgagtgtgagcgcgagaggcgggaggaacagtttagtaccacattgcccagctaactcgaacgcgaccaacttataaacccgcgcgctgtcgcttgtgtgactgcaaaaggcaatgttcgttttagagctagaaatagcaagttaaaataaggctagtccgttatcaacttgaaaaagtggcaccgagtcggtgctctgttcctcgtgctggacaagtgtggtttccagattctgcaaccaagactgcgcaggcattgctggacttcaaccgtgaaggattacctctgttcatcctcgctaactggagaggcttctctggtggacaaagagatctctttgaaggaattcttcaggctggctcgactattgttgagaaccttaggacatacaatcagcctgcctttgtctacattcccatggctgcagagctacgaggaggggcttgggttgtggttgatagcaagataaacccagaccgcattgagtgctatgctgagaggactgcaaaatccaatgttctcgaaccgcaagggttaattgagatcaagttcaggtcagaggaactccaggattgcatgagtcggcttgacccaacattaattgatctgaaagcaaaactcgaagtagcaaataaaaatggaagtgctgacacaaaatcgcttcaagaaaatatagaagctcgaacaaaacagttgatgcctctatatactcagattgcgatacggtttgctgaattgcatgatacatccctcagaatggctgcgaaaggtgtgattaagaaagttgtggactgggaagaatcacgatctttcttttttttgcggccgccccgggcctgcaggggatcccgatcgggccggccgtttaaacccactttgtacaagaaagctgggtatttaaatgaattcaagcttttaattaatgcagtgcagcgtgacccggtcgtgcccctctctagagataatgagcattgcatgtctaagttataaaaaattaccacatattttttttgtcacacttgtttgaagtgcagtttatctatctttatacatatatttaaactttactctacgaataatataatctatagtactacaataatatcagtgttttagagaatcatataaatgaacagttagacatggtctaaaggacaattgagtattttgacaacaggactctacagttttatctttttagtgtgcatgtgttctcctttttttttgcaaatagcttcacctatataatacttcatccattttattagtacatccatttagggtttagggttaatggtttttatagactaatttttttagtacatctattttattctattttagcctctaaattaagaaaactaaaactctattttagtttttttatttaatagtttagatataaaatagaataaaataaagtgactaaaaattaaacaaataccctttaagaaattaaaaaaactaaggaaacatttttcttgtttcgagtagataatgccagcctgttaaacgccgtcgacgagtctaacggacaccaaccagcgaaccagcagcgtcgcgtcgggccaagcgaagcagacggcacggcatctctgtcgctgcctctggacccctctcgagagttccgctccaccgttggacttgctccgctgtcggcatccagaaattgcgtggcggagcggcagacgtgagccggcacggcaggcggcctcctcctcctctcacggcaccggcagctacgggggattcctttcccaccgctccttcgctttcccttcctcgcccgccgtaataaatagacaccccctccacaccctctttccccaacctcgtgttgttcggagcgcacacacacacaaccagatctcccccaaatccacccgtcggcacctccgcttcaaggtacgccgctcgtcctccccccccccccccctctctaccttctctagatcggcgttccggtccatggttagggcccggtagttctacttctgttcatgtttgtgttagatccgtgtttgtgttagatccgtgctgctagcgttcgtacacggatgcgacctgtacgtcagacacgttctgattgctaacttgccagtgtttctctttggggaatcctgggatggctctagccgttccgcagacgggatcgatttcatgattttttttgtttcgttgcatagggtttggtttgcccttttcctttatttcaatatatgccgtgcacttgtttgtcgggtcatcttttcatgcttttttttgtcttggttgtgatgatgtggtctggttgggcggtcgttctagatcggagtagaattctgtttcaaactacctggtggatttattaattttggatctgtatgtgtgtgccatacatattcatagttacgaattgaagatgatggatggaaatatcgatctaggataggtatacatgttgatgcgggttttactgatgcatatacagagatgctttttgttcgcttggttgtgatgatgtggtgtggttgggcggtcgttcattcgttctagatcggagtagaatactgtttcaaactacctggtgtatttattaattttggaactgtatgtgtgtgtcatacatcttcatagttacgagtttaagatggatggaaatatcgatctaggataggtatacatgttgatgtgggttttactgatgcatatacatgatggcatatgcagcatctattcatatgctctaaccttgagtacctatctattataataaacaagtatgttttataattatttcgatcttgatatacttggatgatggcatatgcagcagctatatgtggatttttttagccctgccttcatacgctatttatttgcttggtactgtttcttttgtcgatgctcaccctgttgtttggtgttacttctgcagggcgcgccaccatggctcctaagaagaagcggaaggttggtattcacggggtgcctgcggctgacaagaagtactccatcggcctcgacatcggcaccaacagcgtcggctgggcggtgatcaccgacgagtacaaggtcccgtccaagaagttcaaggtcctgggcaacaccgaccgccactccatcaagaagaacctcatcggcgccctcctcttcgactccggcgagacggcggaggcgacccgcctcaagcgcaccgcccgccgccgctacacccgccgcaagaaccgcatctgctacctccaggagatcttctccaacgagatggcgaaggtcgacgactccttcttccaccgcctcgaggagtccttcctcgtggaggaggacaagaagcacgagcgccaccccatcttcggcaacatcgtcgacgaggtcgcctaccacgagaagtaccccactatctaccaccttcgtaagaagcttgttgactctactgataaggctgatcttcgtctcatctaccttgctctcgctcacatgatcaagttccgtggtcacttccttatcgagggtgaccttaaccctgataactccgacgtggacaagctcttcatccagctcgtccagacctacaaccagctcttcgaggagaaccctatcaacgcttccggtgtcgacgctaaggcgatcctttccgctaggctctccaagtccaggcgtctcgagaacctcatcgcccagctccctggtgagaagaagaacggtcttttcggtaacctcatcgctctctccctcggtctgacccctaacttcaagtccaacttcgacctcgctgaggacgctaagcttcagctctccaaggatacctacgacgatgatctcgacaacctcctcgctcagattggagatcagtacgctgatctcttccttgctgctaagaacctctccgatgctatcctcctttcggatatccttagggttaacactgagatcactaaggctcctctttctgcttccatgatcaagcgctacgacgagcaccaccaggacctcaccctcctcaaggctcttgttcgtcagcagctccccgagaagtacaaggagatcttcttcgaccagtccaagaacggctacgccggttacattgacggtggagctagccaggaggagttctacaagttcatcaagccaatccttgagaagatggatggtactgaggagcttctcgttaagcttaaccgtgaggacctccttaggaagcagaggactttcgataacggctctatccctcaccagatccaccttggtgagcttcacgccatccttcgtaggcaggaggacttctaccctttcctcaaggacaaccgtgagaagatcgagaagatccttactttccgtattccttactacgttggtcctcttgctcgtggtaactcccgtttcgcttggatgactaggaagtccgaggagactatcaccccttggaacttcgaggaggttgttgacaagggtgcttccgcccagtccttcatcgagcgcatgaccaacttcgacaagaacctccccaacgagaaggtcctccccaagcactccctcctctacgagtacttcacggtctacaacgagctcaccaaggtcaagtacgtcaccgagggtatgcgcaagcctgccttcctctccggcgagcagaagaaggctatcgttgacctcctcttcaagaccaaccgcaaggtcaccgtcaagcagctcaaggaggactacttcaagaagatcgagtgcttcgactccgtcgagatcagcggcgttgaggaccgtttcaacgcttctctcggcacctaccacgatctcctcaagatcatcaaggacaaggacttcctcgacaacgaggagaacgaggacatcctcgaggacatcgtcctcactcttactctcttcgaggatagggagatgatcgaggagaggctcaagacttacgctcatctcttcgatgacaaggttatgaagcagctcaagcgtcgccgttacaccggttggggtaggctctcccgcaagctcatcaacggtatcagggataagcagagcggcaagactatcctcgacttcctcaagtctgatggtttcgctaacaggaacttcatgcagctcatccacgatgactctcttaccttcaaggaggatattcagaaggctcaggtgtccggtcagggcgactctctccacgagcacattgctaaccttgctggttcccctgctatcaagaagggcatccttcagactgttaaggttgtcgatgagcttgtcaaggttatgggtcgtcacaagcctgagaacatcgtcatcgagatggctcgtgagaaccagactacccagaagggtcagaagaactcgagggagcgcatgaagaggattgaggagggtatcaaggagcttggttctcagatccttaaggagcaccctgtcgagaacacccagctccagaacgagaagctctacctctactacctccagaacggtagggatatgtacgttgaccaggagctcgacatcaacaggctttctgactacgacgtcgaccacattgttcctcagtctttccttaaggatgactccatcgacaacaaggtcctcacgaggtccgacaagaacaggggtaagtcggacaacgtcccttccgaggaggttgtcaagaagatgaagaactactggaggcagcttctcaacgctaagctcattacccagaggaagttcgacaacctcacgaaggctgagaggggtggcctttccgagcttgacaaggctggtttcatcaagaggcagcttgttgagacgaggcagattaccaagcacgttgctcagatcctcgattctaggatgaacaccaagtacgacgagaacgacaagctcatccgcgaggtcaaggtgatcaccctcaagtccaagctcgtctccgacttccgcaaggacttccagttctacaaggtccgcgagatcaacaactaccaccacgctcacgatgcttaccttaacgctgtcgttggcaccgctcttatcaagaagtaccctaagcttgagtccgagttcgtctacggtgactacaaggtctacgacgttcgtaagatgatcgccaagtccgagcaggagatcggcaaggccaccgccaagtacttcttctactccaacatcatgaacttcttcaagaccgagatcaccctcgccaacggcgagatccgcaagcgccctcttatcgagacgaacggtgagactggtgagatcgtttgggacaagggtcgcgacttcgctactgttcgcaaggtcctttctatgcctcaggttaacatcgtcaagaagaccgaggtccagaccggtggcttctccaaggagtctatccttccaaagagaaactcggacaagctcatcgctaggaagaaggattgggaccctaagaagtacggtggtttcgactcccctactgtcgcctactccgtcctcgtggtcgccaaggtggagaagggtaagtcgaagaagctcaagtccgtcaaggagctcctcggcatcaccatcatggagcgctcctccttcgagaagaacccgatcgacttcctcgaggccaagggctacaaggaggtcaagaaggacctcatcatcaagctccccaagtactctcttttcgagctcgagaacggtcgtaagaggatgctggcttccgctggtgagctccagaagggtaacgagcttgctcttccttccaagtacgtgaacttcctctacctcgcctcccactacgagaagctcaagggttcccctgaggataacgagcagaagcagctcttcgtggagcagcacaagcactacctcgacgagatcatcgagcagatctccgagttctccaagcgcgtcatcctcgctgacgctaacctcgacaaggtcctctccgcctacaacaagcaccgcgacaagcccatccgcgagcaggccgagaacatcatccacctcttcacgctcacgaacctcggcgcccctgctgctttcaagtacttcgacaccaccatcgacaggaagcgttacacgtccaccaaggaggttctcgacgctactctcatccaccagtccatcaccggtctttacgagactcgtatcgacctttcccagcttggtggtgataagcgtcctgctgccaccaaaaaggccggacaggctaagaaaaagaagtagcctgcaggtcctgctttaatgagatatgcgagacgcctatgatcgcatgatatttgctttcaattctgttgtgcacgttgtaaaaaacctgagcatgtgtagctcagatccttaccgccggtttcggttcattctaatgaatatatcacccgttactatcgtatttttatgaataatattctccgttcaatttactgattgtaccctactacttatatgtacaatattaaaatgaaaacaatatattgtgctgaataggtttatagcgacatctatgatagagcgccacaataacaaacaattgcgttttattattacaaatccaattttaaaaaaagcggcagaaccggtcaaacctaaaagactgattacataaatcttattcaaatttcaaaagtgccccaggggctagtatctacgacacaccgagcggcgaactaataacgctcactgaagggaactccggttccccgccggcgcgcatgggtgagattccttgaagttgagtattggccgtccgctctaccgaaagttacgggcaccattcaacccggtccagcacggcggccgggtaaccgacttgctgccccgagaattatgcagcatttttttggtgtatgtgggccccaaatgaagtgcaggtcaaaccttgacagtgacgacaaatcgttgggcgggtccagggcgaattttgcgacaacatgtcgaggctcagcaggccggccgtttaaaccaacttta

SEQ ID NO: 69 - DNA, 3755 bp, synthetic construct
  misc_feature 1..3755: note = Vector CC020
  source 1..3755: mol_type = other DNA
cgcggatcatgaaccaacggcctggctgtatttggtggttgtgtagggagatggggagaagaaaagcccgattctcttcgctgtgatgggctggatgcatgcgggggagcgggaggcccaagtacgtgcacggtgagcggcccacagggcgagtgtgagcgcgagaggcgggaggaacagtttagtaccacattgcccagctaactcgaacgcgaccaacttataaacccgcgcgctgtcgcttgtgtgtgggttattgattctgttggttttagagctagaaatagcaagttaaaataaggctagtccgttatcaacttgaaaaagtggcaccgagtcggtgcattacgttcagagctggatcatttggcccaagggaagatgcattctttgaagctgttaccaacctagcctgtgagaagaaacttcctcttatttatttggcagcaaattctggtgctcgaattggcatagcagatgaagtgaaatcttgcttccgtgttgggtggtctgatgatggcagccctgaacgtgggtttcagtacatttatctaagcgaagaagactatgctcgtattggcacttctgtcatagcacataagatgcagctagacagtggtgaaattaggtgggttattgattctgttgtcggcaaggaagatggacttggtgtggagaatctccatggaagtgctgctattgccagtgcttattctagggcatataaggagacatttacacttacatttgtgactggaagaactgttggaataggagcttatcttgctcgacttggcatccggtgcatacagcgtcttgaccagcctattattcttacaggctattctgcactgaacaagcttcttgggcgggaagtgtacagctcccacatgcagttgggtggtcccaaaatcatggcaactaatggtgttgtccatcttactgtttcagatgaccttgaaggcgtttctaatatattgaggttttttttgcggccgccccgggcctgcaggggatcccgatcgggccggccgtttaaacccactttgtacaagaaagttgaacgagaaacgtaaaatgatataaatatcaatatattaaattagattttgcataaaaaacagactacataatactgtaaaacacaacatatgcagtcactatgaaccaactacttagatggtattagtgacctgtactgggcctcatgggccttccgctcactgcccgctttccagtcgggaaacctgtcgtgccagctgcattaacatggtcatagctgtttccttgcgtattgggcgctctccgcttcctcgctcactgactcgctgcgctcggtcgttcgggtaaagcctggggtgcctaatgagcaaaaggccagcaaaaggccaggaaccgtaaaaaggccgcgttgctggcgtttttccataggctccgcccccctgacgagcatcacaaaaatcgacgctcaagtcagaggtggcgaaacccgacaggactataaagataccaggcgtttccccctggaagctccctcgtgcgctctcctgttccgaccctgccgcttaccggatacctgtccgcctttctcccttcgggaagcgtggcgctttctcatagctcacgctgtaggtatctcagttcggtgtaggtcgttcgctccaagctgggctgtgtgcacgaaccccccgttcagcccgaccgctgcgccttatccggtaactatcgtcttgagtccaacccggtaagacacgacttatcgccactggcagcagccactggtaacaggattagcagagcgaggtatgtaggcggtgctacagagttcttgaagtggtggcctaactacggctacactagaagaacagtatttggtatctgcgctctgctgaagccagttaccttcggaaaaagagttggtagctcttgatccggcaaacaaaccaccgctggtagcggtggtttttttgtttgcaagcagcagattacgcgcagaaaaaaaggatctcaagaagatcctttgatcttttctacggggtctgacgctcagtggaacgaaaactcacgttaagggattttggtcatgagattatcaaaaaggatcttcacctagatccttttaaattaaaaatgaagttttaaatcaatctaaagtatatatgagtaaacttggtctgacagttaccaatgcttaatcagtgaggcacctatctcagcgatctgtctatttcgttcatccatagttgcctgactccccgtcgtgtagataactacgatacgggagggcttaccatctggccccagtgctgcaatgataccgcgagaaccacgctcaccggctccagatttatcagcaataaaccagccagccggaagggccgagcgcagaagtggtcctgcaactttatccgcctccatccagtctattaattgttgccgggaagctagagtaagtagttcgccagttaatagtttgcgcaacgttgttgccattgctacaggcatcgtggtgtcacgctcgtcgtttggtatggcttcattcagctccggttcccaacgatcaaggcgagttacatgatcccccatgttgtgcaaaaaagcggttagctccttcggtcctccgatcgttgtcagaagtaagttggccgcagtgttatcactcatggttatggcagcactgcataattctcttactgtcatgccatccgtaagatgcttttctgtgactggtgagtactcaaccaagtcattctgagaatagtgtatgcggcgaccgagttgctcttgcccggcgtcaatacgggataataccgcgccacatagcagaactttaaaagtgctcatcattggaaaacgttcttcggggcgaaaactctcaaggatcttaccgctgttgagatccagttcgatgtaacccactcgtgcacccaactgatcttcagcatcttttactttcaccagcgtttctgggtgagcaaaaacaggaaggcaaaatgccgcaaaaaagggaataagggcgacacggaaatgttgaatactcatactcttcctttttcaatattattgaagcatttatcagggttattgtctcatgagcggatacatatttgaatgtatttagaaaaataaacaaataggggttccgcgcacatttccccgaaaagtgccacctaaattgtaagcgttaatattttgttaaaattcgcgttaaatttttgttaaatcagctcattttttaaccaataggccgaaatcggcaaaatcccttataaatcaaaagaatagaccgagatagggttgagtggccgctacagggcgctcccattcgccattcaggctgcgcaactgttgggaagggcgtttcggtgcgggcctcttcgctattacgccagctggcgaaagggggatgtgctgcaaggcgattaagttgggtaacgccagggttttcccagtcacgacgttgtaaaacgacggccagtgagcgcgacgtaatacgactcactatagggcgaattggcggaaggccgtcaaggccgcattacaggtcactaataccatctaagtagttggttcatagtgactgcatatgttgtgttttacagtattatgtagtctgttttttatgcaaaatctaatttaatatattgatatttatatcattttacgtttctcgttcaacttttttgtacaaacttgatttaaatgaattcaagcttttaattaagcatgcgagctcggcgcgccggtaccgcgat

SEQ ID NO: 70 - DNA, 17951 bp, synthetic construct
  misc_feature 1..17951: note = Vector RLW139
  source 1..17951: mol_type = other DNA
ttatacatagttgataattcactgggccggccgtttaaacttagttactaatcagtgatcagattgtcgtttcccgccttcactttaaactatcagtgtttgacaggatatattggcgggtaaacctaagagaaaagagcgtttattagaataatcggatatttaaaagggcgtgaaaaggtttatccgttcgtccatttgtatgtcaatattgggggggggggaaagccacgttgtgtctcaaaatctctgatgttacattgcacaagataaaaatatatcatcatgaacaataaaactgtctgcttacataaacagtaatacaaggggtgttcgccaccatgagccatatccagcgtgaaacctcgtgctcccgcccgcgcctcaattccaatatggatgccgacctttatggctacaagtgggcgcgcgacaacgtcggccagtcgggcgcgaccatttatcggctttatggcaaacccgatgccccggaactgttcctgaagcacggcaaaggcagcgtcgcaaacgatgtcaccgatgagatggtccgcctgaactggcttaccgagttcatgccgctgccgacgattaagcatttcatccgtaccccggacgatgcctggctcttgaccacggccattccgggcaaaacggcctttcaggtccttgaagagtacccggactccggtgagaatatcgtggacgccctcgcggtcttcctccgccgtttgcatagcatccccgtgtgcaactgccccttcaactcggaccgggttttccgcctggcacaggcccagtcgcgcatgaataacggcctcgttgacgcgagcgatttcgacgatgaacggaatggctggccggtggaacaggtttggaaggaaatgcacaaactgcttccgttctcgccggattcggtggtcacgcatggtgatttttccctggataatctgatctttgacgagggcaagctgatcggctgcatcgacgtgggtcgcgtcggtatcgccgaccgctatcaggacctggcgatcttgtggaattgcctcggcgagttctcgccctcgctccagaagcgcctgttccagaagtacggcatcgacaacccggatatgaacaagctccagttccacctcatgctggacgaatttttttgaacagaattggttaattggttgtaacactggcagagcattacgctgacttgacgggacggcggctttgttgaataaatcgaacttttgctgagttgaaggatcgatgagttgaaggaccccgtagaaaagatcaaaggatcttcttgagatcctttttttctgcgcgtaatctgctgcttgcaaacaaaaaaaccaccgctaccagcggtggtttgtttgccggatcaagagctaccaactctttttccgaaggtaactggcttcagcagagcgcagataccaaatactgtccttctagtgtagccgtagttaggccaccacttcaagaactctgtagcaccgcctacatacctcgctctgctaatcctgttaccagtggctgctgccagtggcgataagtcgtgtcttaccgggttggactcaagacgatagttaccggataaggcgcagcggtcgggctgaacggggggttcgtgcacacagcccagcttggagcgaacgacctacaccgaactgagatacctacagcgtgagctatgagaaagcgccacgcttcccgaagggagaaaggcggacaggtatccggtaagcggcagggtcggaacaggagagcgcacgagggagcttccagggggaaacgcctggtatctttatagtcctgtcgggtttcgccacctctgacttgagcgtcgatttttgtgatgctcgtcaggggggcggagcctatggaaaaacgccagcaacgcggcctttttacggttcctggccttttgctggccttttgctcacatgttctttcctgcgttatcccctgattctgtggataaccgtattaccgcctttgagtgagctgataccgctcgccgcagccgaacgaccgagcgcagcgagtcagtgagcgaggaagcggaagagcgcctgatgcggtattttctccttacgcatctgtgcggtatttcacaccgcataggccgcgataggccgacgcgaagcggcggggcgtagggagcgcagcgaccgaagggtaggcgctttttgcagctcttcggctgtgcgctggccagacagttatgcacaggccaggcgggttttaagagttttaataagttttaaagagttttaggcggaaaaatcgccttttttctcttttatatcagtcacttacatgtgtgaccggttcccaatgtacggctttgggttcccaatgtacgggttccggttcccaatgtacggctttgggttcccaatgtacgtgctatccacaggaaagagaccttttcgacctttttcccctgctagggcaatttgccctagcatctgctccgtacattaggaaccggcggatgcttcgccctcgatcaggttgcggtagcgcatgactaggatcgggccagcctgccccgcctcctccttcaaatcgtactccggcaggtcatttgacccgatcagcttgcgcacggtgaaacagaacttcttgaactctccggcgctgccactgcgttcgtagatcgtcttgaacaaccatctggcttctgccttgcctgcggcgcggcgtgccaggcggtagagaaaacggccgatgccggggtcgatcaaaaagtaatcggggtgaaccgtcagcacgtccgggttcttgccttctgtgatctcgcggtacatccaatcagcaagctcgatctcgatgtactccggccgcccggtttcgctctttacgatcttgtagcggctaatcaaggcttcaccctcggataccgtcaccaggcggccgttcttggccttcttggtacgctgcatggcaacgtgcgtggtgtttaaccgaatgcaggtttctaccaggtcgtctttctgctttccgccatcggctcgccggcagaacttgagtacgtccgcaacgtgtggacggaacacgcggccgggcttgtctcccttcccttcccggtatcggttcatggattcggttagatgggaaaccgccatcagtaccaggtcgtaatcccacacactggccatgccggcggggcctgcggaaacctctacgtgcccgtctggaagctcgtagcggatcacctcgccagctcgtcggtcacgcttcgacagacggaaaacggccacgtccatgatgctgcgactatcgcgggtgcccacgtcatagagcatcggaacgaaaaaatctggttgctcgtcgcccttgggcggcttcctaatcgacggcgcaccggctgccggcggttgccgggattctttgcggattcgatcagcggccccttgccacgattcaccggggcgtgcttctgcctcgatgcgttgccgctgggcggcctgcgcggccttcaacttctccaccaggtcatcacccagcgccgcgccgatttgtaccgggccggatggtttgcgaccgctcacgccgattcctcgggcttgggggttccagtgccattgcagggccggcagacaacccagccgcttacgcctggccaaccgcccgttcctccacacatggggcattccacggcgtcggtgcctggttgttcttgattttccatgccgcctcctttagccgctaaaattcatctactcatttattcatttgctcatttactctggtagctgcgcgatgtattcagatagcagctcggtaatggtcttgccttggcgtaccgcgtacatcttcagcttggtgtgatcctccgccggcaactgaaagttgacccgcttcatggctggcgtgtctgccaggctggccaacgttgcagccttgctgctgcgtgcgctcggacggccggcacttagcgtgtttgtgcttttgctcattttctctttacctcattaactcaaatgagttttgatttaatttcagcggccagcgcctggacctcgcgggcagcgtcgccctcgggttctgattcaagaacggttgtgccggcggcggcagtgcctgggtagctcacgcgctgcgtgatacgggactcaagaatgggcagctcgtacccggccagcgcctcggcaacctcaccgccgatgcgcgtgcctttgatcgcccgcgacacgacaaaggccgcttgtagccttccatccgtgacctcaatgcgctgcttaaccagctccaccaggtcggcggtggcccaaatgtcgtaagggcttggctgcaccggaatcagcacgaagtcggctgccttgatcgcggacacagccaagtccgccgcctggggcgctccgtcgatcactacgaagtcgcgccggccgatggccttcacgtcgcggtcaatcgtcgggcggtcgatgccgacaacggttagcggttgatcttcccgcacggccgcccaatcgcgggcactgccctggggatcggaatcgactaacagaacatcggccccggcgagttgcagggcgcgggctagatgggttgcgatggtcgtcttgcctgacccgcctttctggttaagtacagcgataaccttcatgcgttccccttgcgtatttgtttatttactcatcgcatcatatacgcagcgaccgcatgacgcaagctgttttactcaaatacacatcacctttttagatgatcagtgattttgtgccgagctgccggtcggggagctgttggctggctggtggcaggatatattgtggtgtaaacaaattgacgcttagacaacttaataacacattgcggacgtctttaatgtactgaatttagttactgatcactgattaagtactgataaatttaattaacagatctcaactttgtatagaaaagttgatttaaatgaattcaagcttttaattaacttagccactgcaacaagttcttgaaccttagcacaatcatattgtgcatgcacttgtttattgcaaagaatggtgcgtagggaacacgcatgatttttgaattgctggcacataattttatcattagaaactggaatgcaacatgtaccctttgtcatggtttctttccgagacattgcactgttttttttaatcctatcattatcataatgccaagaactggtcaccaaccagcattttgcatcatggttagttgagctgtccccatgtatcaataggtgcattgtattggtccaaaatataaatgcagtggatgcaacctatctcatggccgtcaacaaaagaaatcaaaagggaaatgcaccatcttatatctccagtttatatgaacagattggataagatcataagatcaagtggtttatattattttgaggaatataacatggattcatcctaatcactcgtctaggcagtatgtgtattcatgatggatatggtactatactacggagttttttcttcacaaaataacctgttattttgacctccaaccaaacacgaattataccaaaaattgggttatttcatctatagtacaactctattataaacatgcagtaaattatcctacacatataccaaaattcaagtgtaataatcctaatacacagacttaaaaaacaaactatttcctttttaagaaaaggaaaaccatttttttaacggaaggaaaacaaattcgggtcaaggcggaagccagcgcgccaccccacgtcagcgaatacggaggcgcggggttgacggcgtcacccggtcctaacggcgaccaacaaaccagccagaagaaattacagtaaaaaaaagtaaattgcactttgatccaccttttattacccaagtttcaatttggaccacccttaaacctatcttttcaaattgggccgggttgtggtttggactaccatgaacaacttttcgtcatgtctaacttccctttcggcaaacatatgaaccatatatagaggagatcggccgtatactagagctgatgtgtttaaggtcgttgattgcacgagaaaaaaaaaatccaaatcgcaacaatagcaaatttatctagttcaaagtgaaaagatatgtttaaaggtagtccaaagtaaaacttaggggctgtttggttcccagccatactttaccattacttgccaacaaaagttgccacaccttgtctaaggtgaggtgatcaaattgttagccacaacttactaagcctaagggaatcttgccacacttttttgagccattgacacgtgggacttaatttgttagagggaaatcttgccacaactgtggctacaaccaaacacctgtcaaatttgcctaaccttaggcgtggcaaactgtggcaaagtgtggcttacaaccaaacacacccttagataataaaatgtggtccaaagcgtaattcactaaaaaaaaatcaacgagacgtgtaccaaacggagacaaacggcatcttctcgaaatttcccaaccgctcgctcgcccgcctcgtcttcccggaaaccgcggtggtttcagcgtggcggattctccaagcagacggagacgtcacggcacgggactcctcccaccacccaaccgccataaataccagccccctcatctcctctcctcgcatcagctccacccccgaaaaatttctccccaatctcgcgaggctctcgtcgtcgaatcgaatcctctcgcgtcctcaagcttggcatccaggtacggatccgcgtcccatctccctcaccccccgtgttcttcgtgcctgcttctgggtcagatctgggtggattcgcggttgttggatgtggggggctgtgtttatttgtcggtggatctggttgtctggatctgcgttttctctgtcgtagttagcggatctgatgaaatgtttagtgttcgtgtatactggtatggtggatctggtcctaggatgcgtggaatggatatatgtaggcgaattggaggatttattttgtgaattttgctgaaatgatagttctaaacactggatctgacctcgggatgctgttaaatgtggaaatcatggtcgatgctgtcatgaacatggtgttcttatggtagatctgagcaatgtatgtttcaaaattgtttgtcacatggaaatgctatggttctagatgcaatagaatgatacatgccgagatcccctctagttgatatgatagatcatgatgttttacagctatgtcatatgaatatgttcatttgttaccgatgtatttggatctacttaacatttccaaagcacgccgcgttctaattctagatctggtagtcatgtttgtacacgtcacccacctaatacaaatacatatgtctagtgtttggtgacactgcccgtcagatctgttttttccagatctgtggaacaaatactccacgcatgtatggtagttttgaaacgatcttgtatcttccattgttgtagtaacaactaaataaagtacaattgttcaattattgggaatcgtattttctgtagtgccgatgtacagcatattcatagatgtctatttaggaactcaaattttaaattgaggactagttatttattgtgggtcagtcttttgaattgtgttatcttgctgtactggcgcgccaccatggccaccgccgccgccgcgtctaccgcgctcactggcgccactaccgctgcgcccaaggcgaggcgccgggcgcacctcctggccacccgccgcgccctcgccgcgcccatcaggtgctcagcggcgtcacccgccatgccgatggctcccccggccaccccgctccggccgtggggccccaccgatccccgcaagggcgccgacatcctcgtcgagtccctcgagcgctgcggcgtccgcgacgtcttcgcctaccccggcggcacgtccatggagatccaccaggcactcacccgctcccccgtcatcgccaaccacctcttccgccacgagcaaggggaggcctttgcggcctccggctacgcgcgctcctcgggccgcgtcggcgtctgcatcgccacctccggccccggcgccaccaaccttgtctccgcgctcgccgacgcgctgctcgattccgtccccatggtcgccatcacgggacaggtgccgcgacgcatgattggcaccgacgccttccaggagacgcccatcgtcgaggtcacccgctccatcaccaagcacaactacctggtcctcgacgtcgacgacatcccccgcgtcgtgcaggaggctttcttcctcgcctcctctggtcgaccggggccggtgcttgtcgacatccccaaggacatccagcagcagatggcggtgcctgtctgggacaagcccatgagtctgcctgggtacattgcgcgccttcccaagccccctgcgactgagttgcttgagcaggtgctgcgtcttgttggtgaatcccggcgccctgttctttatgttggcggtggctgcgcagcatctggtgaggagttgcgacgctttgtggagctgactggaatcccggtcacaactactcttatgggcctcggcaacttccccagcgacgacccactgtctctgcgcatgctaggtatgcatggcacggtgtatgcaaattatgcagtggataaggccgatctgttgcttgcacttggtgtgcggtttgatgatcgtgtgacagggaagattgaggcttttgcaagcagggctaagattgtgcacgttgatattgatccggctgagattggcaagaacaagcagccacatgtgtccatctgtgcagatgttaagcttgctttgcagggcatgaatgctcttcttgaaggaagcacatcaaagaagagctttgactttggctcatggaacgatgagttggatcagcagaagagggaattcccccttgggtataaaacatctaatgaggagatccagccacaatatgctattcaggttcttgatgagctgacgaaaggcgaggccatcatcggcacaggtgttgggcagcaccagatgtgggcggcacagtactacacttacaagcggccaaggcagtggttgtcttcagctggtcttggggctatgggatttggtttgccggctgctgctggtgcttctgtggccaacccaggtgttactgttgttgacatcgatggagatggtagctttctcatgaacgttcaggagctagctatgatccgaattgagaacctcccggtgaaggtctttgtgctaaacaaccagcacctggggatggtggtgcagtgggaggacaggttctataaggccaacagagcgcacacatacttgggaaacccagagaatgaaagtgagatatatccagatttcgtgacgatcgccaaagggttcaacattccagcggtccgtgtgacaaagaagaacgaagtccgcgcagcgataaagaagatgctcgagactccagggccgtacctcttggatataatcgtcccacaccaggagcatgtgttgcctatgatccctaatggtggggctttcaaggatatgatcctggatggtgatggcaggactgtgtactagcctgcaggcctaggatcgttcaaacatttggcaataaagtttcttaagattgaatcctgttgccggtcttgcgatgattatcatataatttctgttgaattacgttaagcatgtaataattaacatgtaatgcatgacgttatttatgagatgggtttttatgattagagtcccgcaattatacatttaatacgcgatagaaaacaaaatatagcgcgcaaactaggataaattatcgcgcgcggtgtcatctatgttactagatcggccggccgtttaaacagcctgcttttttgtacaaacttgatttaaatgaattcaagcttttaattaagcatgcgagctcggcgcgccggtaccgcgatcgcggatcatgaaccaacggcctggctgtatttggtggttgtgtagggagatggggagaagaaaagcccgattctcttcgctgtgatgggctggatgcatgcgggggagcgggaggcccaagtacgtgcacggtgagcggcccacagggcgagtgtgagcgcgagaggcgggaggaacagtttagtaccacattgcccagctaactcgaacgcgaccaacttataaacccgcgcgctgtcgcttgtgtgtgggttattgattctgttggttttagagctagaaatagcaagttaaaataaggctagtccgttatcaacttgaaaaagtggcaccgagtcggtgcattacgttcagagctggatcatttggcccaagggaagatgcattctttgaagctgttaccaacctagcctgtgagaagaaacttcctcttatttatttggcagcaaattctggtgctcgaattggcatagcagatgaagtgaaatcttgcttccgtgttgggtggtctgatgatggcagccctgaacgtgggtttcagtacatttatctaagcgaagaagactatgctcgtattggcacttctgtcatagcacataagatgcagctagacagtggtgaaattaggtgggttattgattctgttgtcggcaaggaagatggacttggtgtggagaatctccatggaagtgctgctattgccagtgcttattctagggcatataaggagacatttacacttacatttgtgactggaagaactgttggaataggagcttatcttgctcgacttggcatccggtgcatacagcgtcttgaccagcctattattcttacaggctattctgcactgaacaagcttcttgggcgggaagtgtacagctcccacatgcagttgggtggtcccaaaatcatggcaactaatggtgttgtccatcttactgtttcagatgaccttgaaggcgtttctaatatattgaggttttttttgcggccgccccgggcctgcaggggatcccgatcgggccggccgtttaaacccactttgtacaagaaagctgggtatttaaatgaattcaagcttttaattaatgcagtgcagcgtgacccggtcgtgcccctctctagagataatgagcattgcatgtctaagttataaaaaattaccacatattttttttgtcacacttgtttgaagtgcagtttatctatctttatacatatatttaaactttactctacgaataatataatctatagtactacaataatatcagtgttttagagaatcatataaatgaacagttagacatggtctaaaggacaattgagtattttgacaacaggactctacagttttatctttttagtgtgcatgtgttctcctttttttttgcaaatagcttcacctatataatacttcatccattttattagtacatccatttagggtttagggttaatggtttttatagactaatttttttagtacatctattttattctattttagcctctaaattaagaaaactaaaactctattttagtttttttatttaatagtttagatataaaatagaataaaataaagtgactaaaaattaaacaaataccctttaagaaattaaaaaaactaaggaaacatttttcttgtttcgagtagataatgccagcctgttaaacgccgtcgacgagtctaacggacaccaaccagcgaaccagcagcgtcgcgtcgggccaagcgaagcagacggcacggcatctctgtcgctgcctctggacccctctcgagagttccgctccaccgttggacttgctccgctgtcggcatccagaaattgcgtggcggagcggcagacgtgagccggcacggcaggcggcctcctcctcctctcacggcaccggcagctacgggggattcctttcccaccgctccttcgctttcccttcctcgcccgccgtaataaatagacaccccctccacaccctctttccccaacctcgtgttgttcggagcgcacacacacacaaccagatctcccccaaatccacccgtcggcacctccgcttcaaggtacgccgctcgtcctccccccccccccccctctctaccttctctagatcggcgttccggtccatggttagggcccggtagttctacttctgttcatgtttgtgttagatccgtgtttgtgttagatccgtgctgctagcgttcgtacacggatgcgacctgtacgtcagacacgttctgattgctaacttgccagtgtttctctttggggaatcctgggatggctctagccgttccgcagacgggatcgatttcatgattttttttgtttcgttgcatagggtttggtttgcccttttcctttatttcaatatatgccgtgcacttgtttgtcgggtcatcttttcatgcttttttttgtcttggttgtgatgatgtggtctggttgggcggtcgttctagatcggagtagaattctgtttcaaactacctggtggatttattaattttggatctgtatgtgtgtgccatacatattcatagttacgaattgaagatgatggatggaaatatcgatctaggataggtatacatgttgatgcgggttttactgatgcatatacagagatgctttttgttcgcttggttgtgatgatgtggtgtggttgggcggtcgttcattcgttctagatcggagtagaatactgtttcaaactacctggtgtatttattaattttggaactgtatgtgtgtgtcatacatcttcatagttacgagtttaagatggatggaaatatcgatctaggataggtatacatgttgatgtgggttttactgatgcatatacatgatggcatatgcagcatctattcatatgctctaaccttgagtacctatctattataataaacaagtatgttttataattatttcgatcttgatatacttggatgatggcatatgcagcagctatatgtggatttttttagccctgccttcatacgctatttatttgcttggtactgtttcttttgtcgatgctcaccctgttgtttggtgttacttctgcagggcgcgccaccatggctcctaagaagaagcggaaggttggtattcacggggtgcctgcggctgacaagaagtactccatcggcctcgacatcggcaccaacagcgtcggctgggcggtgatcaccgacgagtacaaggtcccgtccaagaagttcaaggtcctgggcaacaccgaccgccactccatcaagaagaacctcatcggcgccctcctcttcgactccggcgagacggcggaggcgacccgcctcaagcgcaccgcccgccgccgctacacccgccgcaagaaccgcatctgctacctccaggagatcttctccaacgagatggcgaaggtcgacgactccttcttccaccgcctcgaggagtccttcctcgtggaggaggacaagaagcacgagcgccaccccatcttcggcaacatcgtcgacgaggtcgcctaccacgagaagtaccccactatctaccaccttcgtaagaagcttgttgactctactgataaggctgatcttcgtctcatctaccttgctctcgctcacatgatcaagttccgtggtcacttccttatcgagggtgaccttaaccctgataactccgacgtggacaagctcttcatccagctcgtccagacctacaaccagctcttcgaggagaaccctatcaacgcttccggtgtcgacgctaaggcgatcctttccgctaggctctccaagtccaggcgtctcgagaacctcatcgcccagctccctggtgagaagaagaacggtcttttcggtaacctcatcgctctctccctcggtctgacccctaacttcaagtccaacttcgacctcgctgaggacgctaagcttcagctctccaaggatacctacgacgatgatctcgacaacctcctcgctcagattggagatcagtacgctgatctcttccttgctgctaagaacctctccgatgctatcctcctttcggatatccttagggttaacactgagatcactaaggctcctctttctgcttccatgatcaagcgctacgacgagcaccaccaggacctcaccctcctcaaggctcttgttcgtcagcagctccccgagaagtacaaggagatcttcttcgaccagtccaagaacggctacgccggttacattgacggtggagctagccaggaggagttctacaagttcatcaagccaatccttgagaagatggatggtactgaggagcttctcgttaagcttaaccgtgaggacctccttaggaagcagaggactttcgataacggctctatccctcaccagatccaccttggtgagcttcacgccatccttcgtaggcaggaggacttctaccctttcctcaaggacaaccgtgagaagatcgagaagatccttactttccgtattccttactacgttggtcctcttgctcgtggtaactcccgtttcgcttggatgactaggaagtccgaggagactatcaccccttggaacttcgaggaggttgttgacaagggtgcttccgcccagtccttcatcgagcgcatgaccaacttcgacaagaacctccccaacgagaaggtcctccccaagcactccctcctctacgagtacttcacggtctacaacgagctcaccaaggtcaagtacgtcaccgagggtatgcgcaagcctgccttcctctccggcgagcagaagaaggctatcgttgacctcctcttcaagaccaaccgcaaggtcaccgtcaagcagctcaaggaggactacttcaagaagatcgagtgcttcgactccgtcgagatcagcggcgttgaggaccgtttcaacgcttctctcggcacctaccacgatctcctcaagatcatcaaggacaaggacttcctcgacaacgaggagaacgaggacatcctcgaggacatcgtcctcactcttactctcttcgaggatagggagatgatcgaggagaggctcaagacttacgctcatctcttcgatgacaaggttatgaagcagctcaagcgtcgccgttacaccggttggggtaggctctcccgcaagctcatcaacggtatcagggataagcagagcggcaagactatcctcgacttcctcaagtctgatggtttcgctaacaggaacttcatgcagctcatccacgatgactctcttaccttcaaggaggatattcagaaggctcaggtgtccggtcagggcgactctctccacgagcacattgctaaccttgctggttcccctgctatcaagaagggcatccttcagactgttaaggttgtcgatgagcttgtcaaggttatgggtcgtcacaagcctgagaacatcgtcatcgagatggctcgtgagaaccagactacccagaagggtcagaagaactcgagggagcgcatgaagaggattgaggagggtatcaaggagcttggttctcagatccttaaggagcaccctgtcgagaacacccagctccagaacgagaagctctacctctactacctccagaacggtagggatatgtacgttgaccaggagctcgacatcaacaggctttctgactacgacgtcgaccacattgttcctcagtctttccttaaggatgactccatcgacaacaaggtcctcacgaggtccgacaagaacaggggtaagtcggacaacgtcccttccgaggaggttgtcaagaagatgaagaactactggaggcagcttctcaacgctaagctcattacccagaggaagttcgacaacctcacgaaggctgagaggggtggcctttccgagcttgacaaggctggtttcatcaagaggcagcttgttgagacgaggcagattaccaagcacgttgctcagatcctcgattctaggatgaacaccaagtacgacgagaacgacaagctcatccgcgaggtcaaggtgatcaccctcaagtccaagctcgtctccgacttccgcaaggacttccagttctacaaggtccgcgagatcaacaactaccaccacgctcacgatgcttaccttaacgctgtcgttggcaccgctcttatcaagaagtaccctaagcttgagtccgagttcgtctacggtgactacaaggtctacgacgttcgtaagatgatcgccaagtccgagcaggagatcggcaaggccaccgccaagtacttcttctactccaacatcatgaacttcttcaagaccgagatcaccctcgccaacggcgagatccgcaagcgccctcttatcgagacgaacggtgagactggtgagatcgtttgggacaagggtcgcgacttcgctactgttcgcaaggtcctttctatgcctcaggttaacatcgtcaagaagaccgaggtccagaccggtggcttctccaaggagtctatccttccaaagagaaactcggacaagctcatcgctaggaagaaggattgggaccctaagaagtacggtggtttcgactcccctactgtcgcctactccgtcctcgtggtcgccaaggtggagaagggtaagtcgaagaagctcaagtccgtcaaggagctcctcggcatcaccatcatggagcgctcctccttcgagaagaacccgatcgacttcctcgaggccaagggctacaaggaggtcaagaaggacctcatcatcaagctccccaagtactctcttttcgagctcgagaacggtcgtaagaggatgctggcttccgctggtgagctccagaagggtaacgagcttgctcttccttccaagtacgtgaacttcctctacctcgcctcccactacgagaagctcaagggttcccctgaggataacgagcagaagcagctcttcgtggagcagcacaagcactacctcgacgagatcatcgagcagatctccgagttctccaagcgcgtcatcctcgctgacgctaacctcgacaaggtcctctccgcctacaacaagcaccgcgacaagcccatccgcgagcaggccgagaacatcatccacctcttcacgctcacgaacctcggcgcccctgctgctttcaagtacttcgacaccaccatcgacaggaagcgttacacgtccaccaaggaggttctcgacgctactctcatccaccagtccatcaccggtctttacgagactcgtatcgacctttcccagcttggtggtgataagcgtcctgctgccaccaaaaaggccggacaggctaagaaaaagaagtagcctgcaggtcctgctttaatgagatatgcgagacgcctatgatcgcatgatatttgctttcaattctgttgtgcacgttgtaaaaaacctgagcatgtgtagctcagatccttaccgccggtttcggttcattctaatgaatatatcacccgttactatcgtatttttatgaataatattctccgttcaatttactgattgtaccctactacttatatgtacaatattaaaatgaaaacaatatattgtgctgaataggtttatagcgacatctatgatagagcgccacaataacaaacaattgcgttttattattacaaatccaattttaaaaaaagcggcagaaccggtcaaacctaaaagactgattacataaatcttattcaaatttcaaaagtgccccaggggctagtatctacgacacaccgagcggcgaactaataacgctcactgaagggaactccggttccccgccggcgcgcatgggtgagattccttgaagttgagtattggccgtccgctctaccgaaagttacgggcaccattcaacccggtccagcacggcggccgggtaaccgacttgctgccccgagaattatgcagcatttttttggtgtatgtgggccccaaatgaagtgcaggtcaaaccttgacagtgacgacaaatcgttgggcgggtccagggcgaattttgcgacaacatgtcgaggctcagcaggccggccgtttaaaccaacttta

SEQ ID NO: 71 - protein, 10 aa, synthetic construct
  REGION 1..10: note = Nuclear Localization Signal
MSERKRREKL

SEQ ID NO: 72 - protein, 16 aa, synthetic construct
  REGION 1..16: note = Nuclear Localization Signal
KRPAATKKAGQAKKKK

SEQ ID NO: 73 - DNA, 377 bp, Oryza sativa; identical to SEQ ID NO: 34
  misc_feature 1..377: note = U3 snRNA promoter
  source 1..377: mol_type = genomic DNA